European Patent Specification EP 3 905 880 B1, published June 12, 2024. Title: SUPPLEMENTED SERUM-CONTAINING CULTURE MEDIUM FOR ENHANCED ARPE-19 GROWTH AND HUMAN CYTOMEGALOVIRUS VACCINE PRODUCTION. Applicant: Merck Sharp & Dohme Corp. Christanti, Sianny Esther Wei Yee Lim Rodriguez, Jason Daniels, Christopher L. The sequence listing filed with the application follows.

SEQUENCE LISTING (1 sequence)

SEQ ID NO: 1 - DNA, 230966 bp, Artificial Sequence
  rdCMV - Destabilized IE 1/2 and UL51
gggccgcgtggtgggtcctcgaggggcgggggggtgtttttagcgggggggtgaaacttggagttgcgtgtgtggacggcgactagttgcgtgtggtgcggaggacggcgacggcgaataaaagcgacgtgcggcgcgcacggcgaaaagaagacgcgtgtctgtgtctgtgtgattccccggggaaaagaggaagttcccgggggacggcagcatgggtccctggggacacacgaaaagcaacgcccgggggcgagggacgacggccctggggaccgcgggggaaataacggccgcgaggccacacactcgttcctgcgaagccgcacaccccgaggccgcgcacaccgccgacacaccccgccaccacaccccgccggcacacccgccacacgcccgcgacacacccggcacgacacacccggcacacgcccgcgacacaccctgacacaccctgccaacacacccccgacacacccaacacacgcccgcgacacacccggcacacacccacccggccgcgccccgacacacccaaaacaccgccggtgcggggccgcgtggtgggtcctcgagggagtgttgagggccgtaagcgtgttgtgtccgacgctgcctgcgcactgccggtgcgtgtcgtcccacggtatttgttgtcggcaccgggcttcgggacggtgtttcggcgcgctgccggtgcgttccacggtccttgcctgtgtcgtttcggcgctgcgcttgtcgggggttttcgagcgttctggccgccggcgatgccggggtgttgcggagacggggggtgtgcgggacggtgttggggccggggacgggggttgcgctggggccggggctgttcgcgccgcgtaggggaggttacgttggggacggggacagtttgcggcgcggaccagggaacccacctcacctatttaacctccacccactacaacacacacatgccgcacaatcatgccagccacagacacaaacagcacccacaccacgccgcttcacccagacgcccaacacacgttacccttacaccacagcaacacacaaccgcatgtccaaacctcggacaaacacgccgacgaagaacaccgcacacagatggagctcgacgccgcagactacgctgcttgcgcacaggcccgccaacacctctacgatcaaacacaacccctactactcgcataccccaacaccaacccacaggacagcgctcattttcccacagagaatcaacatcaactcacgcatccacttcacaacattggcgagggcgcagcactcggctaccccgtcccccgcgcggaaatccgccgcggcggtggcgactgggccgacagcgcaagcgactttgacgccgactgctggtgcatgtggggacgcttcggaaccatgggccgccaacctgtcgtcaccttactgttggcgcgccaacgcgacggcctcgctgactggaacgtcgtacgctgccgcggcacaggctttcgcgcacacgattccgaggacggcgtctctgtctggcgtcagcacctggtttttttactcggaggccacggccgccgtgtacagttagaacgtccatccgcgggagaagcccaagctcgaggcctcttgccacgcatccggatcacccccatctccacatctccacgtcggaaaccgccgcaccccgccacatccaccgcatcgcaccacccacatgcttcgcctcggtcagatcacacgctttttcctgtcccatctacaccctcagccacggttcacaatccccgaaactacgccgtccaacttcacgccgaaacgacccgcacatggcgctgggcacaacgcggtgaacgtggcgcgtggatgccggccgagacatttacgtgtccaaaggataaacgtccctggtagacggggtagggggatctaccagcccagggatcgcgtctttcgccgccacgctgcttcaccgatatccaataaacccatcccctcgccacgacgtctccgcgtatctttgtagcctcaagaatccgtccccacgtccacccatcccgagcactccacacgccataacaaaccacggacacgacaaatgcatgcaaacttctcatttattgtgtctactactctgtgttgctacagggagtgaagagggtgaaggcaaagaaaaaaaaaaggaacaaaataatagattagcagaaggaataatccgtgcgaccgagcttgtgcttcttttcttataaggaggcaaatatactagggaaaacataagaataggaagaaaccgaggtttgggagaaaagctgagataaaatagcgcattttccatacagaggttgttgtttttgtggatcctaagaggtttcaagtgcgaatctcaaagttctcacgagaatattgtcttcaagtatcgacaactgtggtccaagatttttttttggtctttttaggttctgcgagggacatcacgatggatcgttgcgatgaagtcacgcgtacgcctctggtgtggcgcggtgtcgtgacaggagagtgtgttttcagtgcagagctgtcttgattcctatatccgagtatctgttttctcgtaaggacggtaatcttctttggtgtaagtacatctaaaagctgcaaactatattttaagggctgtctctaggtgtactttgatgctggagtttttcgctgtgttgatgtgaataaatctactactactattatatgcagaaagagtgattatgccgagacaagattgcattggctgaactgtttcaaaaacgcctacactctacttatccgtaaacctaaggtaatactatgtgtaagttgtttttttttctttttgtagtaaaatggtgatacgtgcaattaaaactgtattccatgtttccatcctttcatttcaactttaaaggcggctttgagagcgaagaagtgcgaggataaaaatggatgactccttcgtgtccagggagtcgactactgcaacgctgattgattaaaagatggtctccgatgatgatgttgttattgatcgaatcatggtgcagaacggcgacggagaggagcgtgtccgccgccgggaaggtggtctctttctcttttcttttttcaagaaatcttccatgtgtttatcgtagtgatcgaaatcgactgatctcgggttctttttgttggtttcttttcggttaatcatgtattgttttctttttttacagaaagatactttttttcatgagcaattcctcgcccggcgccggcatgccgaggtggggccactgcgatcagcggcatgccgacgccgacccggggatcttggattcaccgttttctctcttctctctctacatacagaccgggtggcaggagcggtaaggaatcatcgtcgtctttcattcttcgatgattatggtaatactaaatcttatctaggagcatatacatctaagattggagtactagtagtcgtttgtggtttctatttttttttatatttatctatgacagtttttctgtttttcgttttgataataatataataaaaactcatggacgtgaaatctggcttggttgtggtgatttcattctcattattgttgttttctttccgtcttgcggatgaagatgttgcgatgcggttgttgttggtgttgctatacaccgagagagatgatctttttgttcttctggttcatttcctatgattgtttggctgctgaccgacgcgtcaggatgtgcagggcatgcggggaatcaggaccggacacgggataatttcatctacctatacggagatcgcggtcctcgccatgaggatcgcgacaggcgcgtcgagggggcaggaacacccttgcggattgacattcttggtggtgtttcgttgttgtcggtagttgttgttgacgatgaggataaataaaaatgaccttgtttttgttctgttttctcttgttgggaatcgtcgactttgaattcttcgagttatcggaaagctgaggtacccaaatgtctgtagcttttttctttttaccctcttgtttatcatctgcgattcgtggtaggtaggagagggaaatgataatccgagattaaggaaaggagaagataaaaaataaaaaaaaataataaaacagaagccgaccggccgccgacccgttccccaggaccagcctacgaggaacggataacgcggtggcgacggcagcggtggtggcgctgggggtggcggcagtggtactgctgatggtagtcgggacggaggagaggcgatgcatacatacacgcgtgcatgctgcatgggtggatggtacggccgggagacgcggaagagaaactcacataaaaaggtgacaaaaagagcggttgaaaaaagaaaacaagattcgaccagacagaagagaaggaccggggcttggcgacccttccacgactgctgttgtcatctcggctcctccgtcttctcccggccacgggcggctaagtcaccgccgttctccccatccgtccgagcgccgaccgaccagccggccgattcgcccgccggggcttctggagaacgccggggcagcagcgatctggggaagctgctaaacccctgcgtttttatatggtagctctgccgagcgcgggctgacgcgttgggtaagcggaaagacgtgtgtgacgaaaaggggtcccatggtatttcacgtgacgatgaggagatacggtttggagcacatacggtttagaaaaagggagttgtcgtgacaagggctgagggacctctgtctccatgtgtgtataaaaagcaaggcacgttcataatgtaaaaaagaacacgttgtaaacaagctattgctgtatcattcggctgactatgcttcattcggactgattttcttttcctaacggcgtaacttaaagtgattaacgtatgatatttgttccccagagttatactatagtcatcatcctaaaattcagatataaatgaacacatgtcgtatgggattattaagaaaccgaaactctccacagttcaccatcttcttcgtcattcaaccgatgacccactccgtacaacgaatcagtctgctgcgtcatattgcaaagcacaagcgacgtatgcgaacaacttgaaacacaggctgttgtattgacgaccgttgtaccattattagtcaccaccgttatcccatgtttcccacccgatggaaaaccgtcttctatcatcaactgtggtaagatttcgaccctgcgaggtattcagtttcctcatatccataacctggattttatcattaaaccccaatattaaacacttttttagtaccccccacccaccaaaaaatgtgactggaccggttcctagcagctctgggagccatgttcaggttgaaccacagctacagcgaaaccgagtccagtgaccggtaaccacgtccagcccctgcgtatgtaccagtccaagcacgtccggtcattgttctacacaggaaatctaactaggtcaacgcaattttattccaccgttacgcagaatactaacaaaaaaacacacaaatttaacgaattacacgtagtttattacatgaaaactgtaagaacaccaattcactaagcgatacaacatttagctgacttccaagtgccacacatcaccactgtattcatccatgttttcaccgaaccaacgagacagatcgaagaagccagaatctcccgactttaaattacataaatccaacgtattatgaccacagctcgacacacaaatagttgcgttactattcacagtagcattacctatacccgtaacgttgcacaaccactgatcaccattgttaccaaaaacggttttccacttagttgtcaacggatctttcctatgcgtaatggtaaaattactaccagtcgtcgcttttagctcattacgagtattatccgcatccacatatatcaacgtcatagctaggcacgctataagtaccccccccccacaatggaatgttgccaaaccggttctttcccgttatagccatagcgttcccaggcaaaagcaaacgccaaacctaatgcagtgaaaagcgcttgcagccagaaccagcttatgtaccagccacaatcacatccggttattgtttccacaggaaatcctaccaggcaaagccccgcttgttttgttcctatcttgtttagcaattcgtaaactgtcagcctagcgacgtccgtttagatcaaaagtcacgtatatagcgacgctgtttccatccgtttccccgtcccgccgtttccgaacaacccacccgggttcagacaaccgaccaccaacagaaatatacacacagaccactgggagttcagttaaagatttcatcaggtttattttggctgctgctagtcttttgcttcttagaaaaaaaatacccatatagagaaataatgatagtttgacaacacatatggcagggatttcttcttcatcaataagatatgcaattcccccagggagagactttcaacaattgaatttacaaaaacaaaattacatcaggagaaagagaggatacattaataaatatattatatctggtgtatatactgaatgctgctggttcataaggtaacgatgctactttttttaattccaagatggtttttctttgttagtcttttgttgacttgctggttcctaaaagttcgcaaaaacgattgtgtgaagattttatgacgttggttgactagttcatgagattctgctgtacgtgtgatggttattcgctggttcgttctaagatgagtatcgtactgtgtctgcgatggtcgtctcttactggcattctctcggctgcctcttgctttcatgattgaaaaggaaaaaaggactccgagggcgcggtcatcttttacttttcggttttctcgttggcgggtcagaggtagtcagatcatgagactgtcgtggtcgatgaaactgtgtctgctcaagtgacgtccatttcttgtacggagaaaaaagtcatcgggataaataaggctatacaaggcgttgtcaagcgtgcggctctaaacaaattaagcgatacaaaattacagtaatacgaataataaattacccccctccccctgtggtcccccgagacgagagccacccatcgtgtactctcgcaccacccacgaccacagagggagacgggacgaagagacgacgcacagcgccatctcctcctggaggccggcgacgttaactgctacagctgcggcggcgaagacagctgcgatttgtcggccgacatgccgatggtatgggcggcggcggcaatggccgcggcagcggggaggagaggagagagaagaggagcggggcgtccgaaggcgaggatggcatggtctcgccggagcgcccggcttttatggaacactcgcgtccggttgggtatcacccacaggaagatgagtcacaacttccaaaccatcttgagacccgagtaacggtttacaggtcgcacgccagtcagctaaaaacagcggacagtcccacgctgtttctgttgtggctctctccagtttcctcatcaccgtcccggtctccgtcgtcatcggaagaataccacccgctctcatgcggcagtcgatcggcctcgacgaacgagacgcggcgacgcctctccacggccgactggttgtggtggtgaaagaagagcaccagcaatcccaggaggagcaacaagccctcacatgtccaggaggtcggggagagggcctgtcggagatggccgtgaggcatcacgtacggcagctgaggagaaacggagaagaaaggaaaattaccgtcaggggccggggttcttattagagaaacagcacgtaggtcaggatccagatgctaatggcaatcatgatgacgatgatcatgcaggccaagacgcggcgcaccaatgccgaatccaatagccgccgtgcctccggttggtggccggcggcatctagagacatgatttgggggggaccggcggcgcaaaaagacagggagatggacagtgtcacggtgttttgttataattaggacatggggaccggaagccgagacagagtactacagggtgttgaagggtaacgtgagggagatcatgtcatgggcgggctgaagaccgtgcggggaggattgacgtgtgcggtgcttgtggaacacggtgttttaatatgtatccgcgtgtaatgcacgcggtgtgctttctggcactcagcttggtaagctatgtggccgtctgcgccgaaaccaaagtcgccaccaactgtctcgtgaaatcagaagatacccatttgacgtgcaagtgcagtccgaataacacatcatctaataccggcaatggcagcaagtgccacgcgatgtgcaaatgccggatcacagaacccattaccatgctaggcgcatactcggcctggggcgcgggctcgttcgtggctacgctgatagtcctgctggtggtcttctttgtaatttacgcgcgcgaggaggagaaaaacaacacgggcaccgaggtagatcaatgtctggcctatcggagcctgacacgcaaaaagctggaacaacacgcggctaaaaagcagaacatctacgaacggattccataccgaccctccagacagaaagataactccccgttgatcgaaccgacgggcacagacgacgaagaggacgaggacgacaacgtctgataaggaaggcgagaacgtgttttgcaccatgcagacctacagcacccccctcacgcttgtcatagtcacgtcgctgtttttgttcacaactcagggaagttcatcgaacgccgtcgaaccaaccaaaaaacccctaaagctcgccaactaccgtgccacctgcgaggaccgtacacgcacgctggttaccaggcttaacactagccatcacagcgtagtctggcagcgttatgatatctacagcagatacatgcgtcgtatgccgccactttgtatcattacagacgcctataaagaaaccacgcgtcagggcggtgcggcgttcgcgtgcacgcgccaaaatctgacgctgtacaatctcacggttaaagatacgggagtctacctcctgcaggatcagtataccggcgatgtcgaggctttctacctcatcatccacccacgtagcttctgccgagccttggaaacgcgtcgatgcttttatccgggaccagggagagttgtggttacggattcccaagaggcagaccgggcaattatctcggatttaaaacgccagtggtccggcctctcactccattgcgcctgggtttcgggaatgatgatctttgttggcgcgctggtcatctgcttcctgcgatcgcaacgaatcggggaacaggacgctgaacatctgcggacggacctagatacggaacctttgttgttgacggtggacggggatttacagtaaaagatgcgtgtcgcctgccgaagacctcaccatctcacgtacaggcatacggcgtatacaatcataatattctatattctgcatagagttacatgcaacagtactactaccaatactgcatccatcacatcacccaacactgcttctaccacctttgtgaccagcgtattttctactccgaataacaacacatcaacgacgccacacacatctgtcacctcacaagcgtcaaccattggcaacatcaccaacgttacctccgacttgagtactttcacaaccgtatattctacattcaatacatcatatgctaatatatccaatacggctgccactacagaattgatttcaacaaataccaacactatattatcttttaccaacgtaacagcaaacgctacatcatcttataacacaacaatcaccgtaactatcacgtcagatgaaacttcgcacaacgtatccactaatactgcacttataagcacgccatggcttacaaattgcagcgccacaacgtacaccacgtacaaccgtactaactcttccaacgcttgtcacacagagacaacaatcatacgtttcaaagaaactaatacaacaggaatagaagggagtaatgtcaccataaaaggtaattctacgtgggattgtctttcagtcgcctggatacgacattacaatcgatccacacacggacatcatctaggtcatcgtaagaacgcacatacccaatcttggtattggttacgcatccttacctctcatactgtatgtcattctcaacatgaaagaccttcactgtaccatgacttatgtcgttcgtgcaacaacacagaactacatctgtacgatctaaatatcaccaattccggcaggtacagcagacgttgttttaaagaaaattacttcacaggacatcacgaagatgaaaatttctacctattagtaacaccaaaaaatcatactgaagctattaatgctactttcgtttgccctagatacaacaccgatatcgaaaatgaagatagagagaaaggaagtcaacatactaacaatacacatcaccacaaacgtaatctctatcatagctcgcaaagaagccgcaccgtatggaccatcgtgttggtttgtatggcctgcatagttctgttttttgcacgacgagcctttaacaaaaagtaccatatgttgcaagacaccgtcagtgaatcagaattcattgttcgatatcacacagaacatgaagattgagctacgtttccgggcagacatcttatgaagctgaacaataaactaaaacattctgtaaggctcagcgttcaaaggaatattaatgcccattgagcgagaactaatattgcaatggactggcgatttacggttatgtggacgatactaatatccgcgttatcagaaagctgcaatcaaacctgttcctgtcaatgtccctgtagtactaccgttaactattccactagtactgagacagccacatcaacatacagtacaacagttatcagcaataaaagcacttcagaatctataaattgctctactgcaactgcaccagcaaccaccgtttctacaaaaccgtcgaaaacaaccacacagatatccacaacgacaaatacaaacgttgagactaccacatgtaccaacaccaccacgaccgttacttgtgatggtttcaattatacagtccataaaagatgcgaccgcagttacgaggtaatcaacgtaacaggatacgttggtggcaacataactctaaaaaatgcaatcagactgagaaatggcacaatgtagactggattcattatgagtaccccacgcataaaatgtgcgaattaggcaactatcaccaaacaacaccacggcacgacatatgttttgactgcaacgacacctccctaactatctacaacttaaccacaagaaacgctggaaaatataccaggcatcaccgtgataacggtcaagaagaaaattactacgtaacggtgttaattggagacacaacgttatccactcttggcacatgccctgtaagatataaagaatctaggaacactgaaaacaccattggaagtaacatcataaaaaccattgagaaagctaacattcccctgggaattcatgctgtatgggcaggcgtagtggtatcagtggcgcttatagcgttgtacatgggtagccatcgcattcccaaaaaaccgcattacaccaaacttcccaaatatgatccagatgaattttggactaaggcttaacatgcacatcaataaactttttttaaccaataacatgtctctgtttttttttgttaacaacctatgatataaagcggtatattcaatcattactaaacaaaaaaacatgggcatgcaatgcaacactaaattgttattgccagtcgcactaataccggttgtaatcatcctaattggtactctagtgcccatacttttacatgaacaaaaaaaggcgttttactggcgactttttctgcaaagtcaacatgtagaagcacccattacagtaacgcagggagacacagtctacctagatgctagcaataatccctgtaattattccagcttttggtaccacggtaattgcgaactttgtggatggaacggatatctacgcaatgttacacattactacacaaacacatcgtgttccccgcaattcatgtgcataaacgaaactaaaggtctgcagttatataatgtaacattaaacgattcaggtgcttatactgaacacgtttacgaatgtgatctttcatgtaacattactacttataacgaatatgaaatactcaattacttcgataactgtaactacaccataaatagcaccaagcatattatcaccgtggtgtcttcacgtcattctaaacaaacaaattcccacgtatccactcacgctggttgggcagccgccgtggtgacggtaattatgatctacgttttgatccactttaacgttccggcaactctgagacacaaactacgaactagaaacaacgtaaatcgcatagcgtgattacaaagtatcgacactaatttatccaagataaaatttgattactccgtgcggttctcaaaaactgtaaggtcccgcttttctactccatcatgaaggatcgcaatagaatactgctatgtatcatctttatttgcatcatgtgcctcatttgtatttactttaaacgtcgttgtgttcttactccgtctccagacaaagcggatctgcgagtggaatttccctcgttacccccgtgtatcggcatacaatgtgctgcatgagaacacgcgtgacacatagcgtacccctggacggtacagtttatgataacgtcattcaggggaagtatacattactatcgacgtgttatcacagaacacacagattttctgcgtgttttataaaagagcgtctcgaagcagcttgagccacactacggtccagatgacgagcgtaatcaaaaatatgccgcgcagtagtcgaaagccgtactgagcgtgcgaggcgggtagggtgccgaacgacggatatgcgtcgttgtcatcttcgactataaggatcgcgaccgagtcttcggccatggtaaacgtcaccctgtgtggctggtatgtagcgtatccggtttggaattgttctgctccagctcgggggatagtgaggaattctcaagggatacgggacccaatgactggataagagaagggtttttccccgtaagatgatcctcgtatcacatgaggtctggatatgtataaatgaagagtgaaataggcacagggaatcagatgccagcctcgtgatgcagccgctggttctctcggcgaagaaattgtcgtctctgttggcttgcaaatacatcccaccttaagcgatgagtccataaagcaccgttgtccgggtacggtgaaagtgactcggattgtagcacgtcccttttttttgtttttgtatcgcttatcgccactgacagtgcaatattttgatcgtgaggctgagtatggttatgatgcttagaacgtggagattattaccaatggtactacttgccgcgtactgttattgtgtttttgggacttgttcaatcggcacgacgactgctcccgtggaatggaagtctcccgaccgtcagattcctaagaatattacttgcgctaactactcagggaccatcaacggcaacgttacatttcgaggtcttcagaacaaaacggaagactttttgcactggttgttagggtggggtcataagtccatctgttcgttcttcccgaaactccagggcaactataacgaacaacattacagatatgaagtagcgaacctgacgtataactgcacctataaccgcttgacgttgctaaatctgacgacggaaaacagcggaaagtactattttaaaagggaagatgcgaatttcaccttttattactcttgttacaacctgaccgtgtcctaaagaacgcacgtgaagttccacagagccgcgtggctgtagctattgtgtttacgttgcttttgaaatgttaagcgtccctacggcgctaacatgtttctaggctactctgactgtgtagatcccggccttgctgtgtatcgtgtatctagatcacgcttaaagctcgtgttgtcttttgtgtggttggtcggtttgcgtctccatgattgtgccgcgttcgagtcctgctgttacgacatcaccgaggcggagagtaacaaggctatatcaagggacaaagcagcattcacctccagcgtgagcacccgtacaccgtccctggcgatcgcgcctcctcctgatcgatcgatgctgttgtcgcgggaggaagaactcgttccgtggagtcgtctcatcatcactaagcagttctacggaggcctgattttccacaccacctgggtcaccggcttcgtcttactaggacttttgacgcttttcgccagcctgtttcgcgtaccgcaatccatctgtcgtttctgcatagaccgtctccgggacatcgcccgtcctctgaaataccgctatcaacgtctcgtcgctaccgtgtagctagttagccagctgtgtatagtttgttgtgttttgcttttgcatatttgttttcagtcagagagtctgaaacggggtgggagggacttttacgggtaatgcatgctaagatgaacgggtgggctggggtgcgcttggtaactcactgtttgaatacgcgctcacgcacatatgtagcactcaacatgttagcttttgcccgcacgccccggggcgtgccgagctgcctttttaataaagtctgggtttccagatacgcgctggttctgattttgatggtttgtgcctctgaaagctctacgagctgggccgtgacatccaatcgactgcctaactgtagcacgataactacaacagcgggtcaagacgctgaattgcacggtccggcaccgttaagctgtaatgtgacccagtggggacgttacgagaatggaagcacacccgtattatggtgcactttatggggatcacgcacgcgagtctcattaggacaccgtgtagcgtttggctgttcttggaaaacattttttatttataacgtttctgaaagtagtggtggcacttattatcaaaaaggttacaactgcaccgacaaacatataacactatcttgtttcaacctaacggtggttcctcgagcggttcaaagcacaaccaccgtaatgacacccacggtggttacaaactccacattcagtgtgtcacttgttgcgtcgagactgacgacaaattccagcgcgtttagacacgctagttatcaacggcaacagcgtgtcggaaacgggacgttatccaagaacataactaacttggcattcacctacggcagctggggcgtcgcgatgctgctgttcgccgccgtgatggtgctcgttgatttgggtttgcctcaatcggcttggcgacgctggcgaagccacgtggacgatgaagaacgtggtttgttaatgtaggaaataaaaggcactgtttgagcatgactgtttccaaaccgtaacgtggtaaataaatcatggcttccgacgtgagctcccatcttctaacggttacacaatcccgttggacaatacatcatatgtacaataaactgttgattttggcgttgtttacccccgtgattctggaatccatcatctacgtgtctgggccacagggagggaacgttaccctggtatccaacttcacttcaaacatcagcgcacggtggtttcgctgggacggcaacgatagtcatctcatttgcttttacaaacgtggagagggtctttctacgccctatgtgggtttaagcctaagttgtgcggctaaccagatcactatcttcaacctcacgttaaacgactccggtcgttacggagcagaaggttttacgagaagcggcgaaaatgaaacgttcctgtggtataatttgaccgtgaaaccgaaacctttggaaactactacagctagtaacgtaacaaccatcgtcacgacgacaccaacggtgatcggcacgaaaagtaacgttacggggaacgccagtttagcaccacaactacgtgccgtcgctggattcttaaatcagacgcctcgggaaaacaacacgcacctggccttggtaggtgttatcgtatttatagctctaatagttgtttgtattatgggatggtggaagttgttatgtagtaaaccaaagttatagtgatgtgctttttatcagggagaaggttttgtgccaacaatgactaaccctgggctatatgcatcggaaaattataacggaaattatgaacttacggaagccgccaatacagcacgtacaaatagcagtgactgggtaacgttaggaaccagtgcgtcgctgttgagaagcacggagactgcggttaaccctagcaacgcgactacggttactccacaacctgtggaatacccagctggggaagtacaatatcaaagaacgaaaacacattattcttggatgctaattattgccataattctcatcatttttattatcatctgtctgcgagcacctcaaaaagtctacgatcgctggaaagacaataaacagtacggacaagtatttatgacggacacggagctgtgatgaactacaatgtatagatacacgtggctgctttggtggataacaatattgcttcgtatacaacagttctatcaatggtggaaaccagatacaacgtcatgcattcagaaaacgggatatgaaggtcaaaacctcagtctgcctcctagtaatgcattatcatctaaagactatactttttcatggtataaagattcacttaaagcccttaacatgttatgttattatactgaaaaacttgaagaaatagatagcaagccagatactatacgacgatgttttttgaatcatacattgtttcttattaatttaacaagtcactatagcgggatttactacttcgattctctatacacatatggttgggtattacggacacctctatgttacaatgtcactgtatattccatatatcaaacacacatccacacaactatattgctctatccgcctacgtccacatataattcattaactatatcatcatttacctcaaccaacttaacacataccgcggtccactatgccgccggtaacgttgaagcacaacacgatactgccaccccacatacaatgtggatcatacccttagttatcgttacaacaattatcgttttaatttgtttcaaatttccccagaaagcttggaataaattcacacaataccgatacaacagtatgctcaccgccgcttaaagaatcaccgtcgagaaaactaaaacgtaaaaagaatggccatgtacgtttatttttcagctcactgtttgaataccgtaaacataatgacgtacatatacgtgattatacaacaggtgtttgtgttatgcggcgactgattaaccatatcgtgaaccatgatcttttccgatggtccgtcatgaccgcaatgatattttacaggtattccgaaacctgtatggaggtcactgtcagagtaggtgatccagttaccctcggtagtggacatggttatcatccaggacaaaaagtacactggtataaccagtcatgcgtcggcattagcaacggcgaaaatacgcatcctatctgcacctacgaccctcctaaacctggtagacgaaagacaatgaaaaccactccgttaccatcaccactgttgtacgagtgtcacaattccacattaagcattcttcatgtaaacgtctcagatcccaaaaactattgcaggcgaaaatgtccaccaaacggtaactgtgaatttcccacatgttttacgttatcactgatttccagaacgacaaccaccagaaaacccggacaaaaaactacgttgtcgcgattaaaaaccacgccaaataaacatacgcagcacaaaagatccacgcgaagaacgtcacctagagattacaatgtaacgggtctgccgaaaggctttgcggactcgtttaccggtaacgtagaggcacatagagccaaagatgccgcacacagcgcatggatcctcattgtcatcatcattatcatagtcgtcattttatttttcttcaagattcctcaaagactcagagagaaatgggacaccagaggatacctttacaaaggaaccgacggcctgcccactacggactacttatcgtgagcggacggatatctccggtttcaaacccactgtttgaatatagggacagtccctacggaacctgagaacatgtggaaatcacctgtggtagaatgctgctcaggtacattacctttcatcgtgaaaaggtactttacctagcgatcgcatgcttctttggtatctacatcagtttccacgacgcatgcattctggtacctgctaaagtaggtactaacgtcacattgaacgcggtacatgtgcatgacggtgactatgtgtactggtcttttggtggaggtggagctaatagattaatgtgtcgctatacaccaaggctagacgaaattcacaaaaacaccaatcgaagtttttcatgtcttacaaatcacagtctccttctcatcaatgtaacggaagaatatactgattactatcgcaccatgaccacattcgtacatcagtcccataattggcacaaccacggcaacaaatggactttagacacatgttattatgtatacgttacccaaaacggaacacttcccactaccaccaccaaaaaacccactacgaccacgagaacgacaactaccaccacaacaaagaaaacaaccaccacgagcacgacaacgaccaccactaccaccaagaagacgacgacaagcactacccatcatcgacactccaatcccaaagaatccaccacccctaaaacccacgtagaacttcacgtcggtttaggagccacagcagcggaaacaccgttacaaccaagcccacagtaccaacacgtggctacacacgccctctgggttttagcggtcgtaatcgttattatcatcattatcattttctactttcgaataccgcaaaagctgtggctgctctggcagcatgacaagcacggcatcgtgctcatccctcaaaccgatctgtgagcaagtcgcgtaggaaatgattgcatgaaatcactgtgaaacgccaactccgtgccagctggcgcggcggacaggcctttgacgtatttgaagccaggcgcgctctcgataccgaaaggatccgagggggctttccaaagccgacgtccctgattcccttcataaagctgttgaccggccctagaaagaccaagagcatgctgtgggcccactgcggtcgcttcttgcgttatcatctgctcccgctgctgctgtgtagactgccattcttactccttttccagcggccgcagtgggcccacggcttggacattgtcgaggaggacgagtggctacgggagatacaaggagcgacgtaccagctgtccatagtgcgccaagccatgcagcacgccggattccaagtcagagcagcgtcggtcatgacgcggcgaaacgccgttgacctggaccgaccgccgctttggtcgggatcgctcccgcatttgcccgtctacgatgtgcgttccccgcggccgttgagaccgccgtcatcacagcatcacgccgtatcacccgaactgccgtcgcgagacgggatacgttggcagtaccaagagctgcagtatctggtggaagaacaacggcggcgaaatcagtcgcgcaatgcgattccgagaccctcgttcccccctccggatccaccatcgcagccggcagaggatgcacgagacgcggacgcagaacgtaccgaatcaccacatagtgcagaaagcaccgtcaggcacgacgcgagtgagaacgcagtgcggcgacggcacgaaagacggcgctataacgctctgacggtccgcagccgggactcgctgctcctgacgcgaatacgcttctccaaccaacggtgtttcggacgcgggcgtctgagacatcccgcgggaagcggtcccaacaccggcggaccgcgacccggcggtgcgggactccgtcaactacgccaacaactgacggtccgctggcagctgttccgcctacggtgccacggttggacacagcaggtctctagccagatcagaacccgctgggaggaaagcaacgtcgtgagccagacggccacgcgagtacgtacgtggttcgtggaaagaaccacgttttggcgtcgcacgtgggttccgagacagaacccggcggccgaagcgcaagaactggccgtcataccgccggcacccacggtgctccggcagaacgaggaaccacgtcaacagcttacgggagaggagacaagaaattcaacgcacactcaacgtgaagaagtggaggacgtttcgagagagggcgcgagagaagggaatgatgggagccgagcaagtggaaacgacgagagaaggaataatgcgggaagatatgatgatgatcatgaggttcaagagccgcaggtcacttatccagcgggacaaggagaactgaataggaggtcacaggaggagaacgaggaaggtggaccgtgtgaatcgccgccaatgacgacaaatacgctgaccgtggcctgtccgccccgagaacccccgcatcgtgccctgtttcgtctatgcttaggactgtgggtctcgagctacctggttcgacggcccatgacgatttagaatacaccgagccattcctttatttccccccatccccggtcgcttatgcgtgttaaacactaccaataaagataatctgccaatcgcaccttatatataatatgtggtcgcgtgtggtctttttaaggagctctgaaacacagacaggtatgggcggtggtcggctgccgccgctgtggctgccgctactgatcgcctggagcgagtggggcaactgctgcctcgatgcgcctccggtggtgcgttcgccctgtctgcagccggtgcgcgaccgcaaccgcgagcggaacccgggctcaccgcagttgctgccttacggcgaccgtctggaggtggcctgcatcttccccgcgcacgactggccagaggtctctatccgagtccacctctgctactggcccgagatcgtgcgttcgctggtggtggacgcacgcagcggtcaggtgttacacaacgacgccagctgttacatcgccggcgggcgctggcgcttcgaggacggcggcgcggcgcagcggctgagcctctcgtttcggctcatcaccgagaccgcgggcacctacacctgcgtgctgggcaacgagacccacagcctggcgaccgagaccacggcgctggtggccgacgtgcacgacctgcgccactcggaccgctcctgcgacctggctttcggatcgcgctcacagacgcggtacctgtggacgcccgatccctccaggttgcgcagtataaactgcggttgggagggtgaacggcaccgcgtagtccactacatccccggcacctcgggtttgctgccctcgtgcgaggaggacgagcgcgaactgtgcgtgcccttcatcagccagagcattgcggacaacaactgcagccgccggcatcgagttgacggcgctaggcggcgctatcatctacggagggattactggctgacggatccgaagatcgggttgctggccgcgggatcggtggccctgacctccctctgccacctgctgtgctactggtgttccgaatcgtaccggcgtctgaacaccgaggaggaaagcgaggcggcggaggaaactgccgcgggagaagcctctgcggtagcggcggcggccgtctctgaggaagagcagcggcgggagtaaacgaggagagccatgaagcggatgattcgcagtcacggcaggaaaacggaatgtcagatgacgagcgccggcgagcgacgcggctccgccgtcggtgcgcccatctgcggcagcggtacccgacgcggcagcggcgccaacgaacgccgcgactccgacgtcggtcccatcgcccacagtagcggtaccagacgcggttcggcgaatgaaacgtccgcctgtacgcggaccgatcaccagaaggcggacattgggctgtggttcatgtttctggtttttggactgtgttcgtggttggcgatgcggtatcgcgcacaataaattttgaatcgatgtcaaggaacgcgtgttttgtattttattgggaatattggcggggataaacctgtttcggatgtttacccttaatcttaccggggacctcgttgtcctctcctccttcttcctcggacaccgggctccatgctgacgtaggtaccgactggggtcaaaagcctgggtacttatgaggagcgcgcacaaaggaccgttaggcgccggcatggagcgtcgccgaggtacggtaccgctgggatgggtgttttttgttctttgcttatctgcctcttcctcgtgtgctgttgacctgggtagcaagtcctccaactcgacctgccgcttgaatgtgacggagttggcctcgatccatcctggggaaacgtggacgttacacgggatgtgtatttctatctgctactacgagaatgtgaccgaggacgagatcatcggcgtggcttttacttggcagcataacgagtctgtggttgacctgtggttgtaccagaacgacacggtgatccgcaatttcagcgacatcaccactaacatcttgcaagacggactgaaaatgcgaaccgtccctgtgactaaactgtacaccagccgcatggtcactaatcttaccgtgggccgctatgactgtttacgctgcgagaacggtacgacgaaaataatcgagcgcctctacgtccgattgggctcgctatatccgagaccgcccggatccgggctcgccaaacacccctccgtaagcgccgacgaggaactgtccgcgaccttggcgagagacatcgtgttggtctcagccatcactctgttcttcttcttgttggccctacggatcccccagcgactgtgtcagcggctgcgcattcgcctgccgcatcgataccagcggttacgcaccgaggactgaacggataaccgcaaaggccacgtgcaacgttcacgctgctataagaaggccatgtcccccgtggacgggtctctttgacacgagcgcggcacgccgttgccacgagcatggatcacgcgctcttcacacacttcgtcggccgaccccgtcactgtcggttggaaatgttgattctggacgaacaggtgtctaagagatcctgggacaccacggtttaccacaggcgccgcaaacatctacctcgacgtcgcgctccgtgcggcccccagaggcccgccgagattcccaaaagaagaaaaaaggcggccgtccttctattttggcacgatttgtgctggctgtttcgacgacttttctttcctcgggaggactcagagccactgatgtcggatccggcacggtctcccgaagaggaggagtaaacaacacacggctaagaggatacatcatcaaagaagataggaggggtcaaaacgcggactgaaagtatataacgccgatcatgtccgaggaactgttaataaaacgccatgatgacaatgtggtgtctgacgttgtttgtgctgtggatgttgagagtggtgggaatgcacgtgttgcgttacgggtacacggggattttcgatgatacatcgcatatgacgttgaccgttgtggggatttttgacgggcaacacttttttacctatcacgttaattccagcgataaagcgtcaagtcgggccaacggtaccatttcttggatggctaacgtctcggcggcctaccccacctacctggacggggaaagagccaaaggtgaccttatttttaaccaaaccgagcaaaacctgttagagctggaaattgcgttgggttaccggtcacagagcgtgctgacgtggacgcacgagtgtaataccacggaaaacggtagttttgtagccggttacgagggatttgggtgggacggggaaactttaatggagctcaaggataacctgacactatggacgggccccaattacgaaattagttggttgaagcaaaacaaaacgtacatcgacggtaaaattaaaaacatcagcgagggggatactacaatacaaaggaactatctcaagggtaattgcactcaatggtccgtcatttatagcgggtttcaaccccccgtcacccacccagtggtaaagggcggtgtccgaaaccagaatgacaacagagctgaagcattctgtacatcttacgggttctttccaggggaaattaatattacttttattcattacggtgataaggtgcccgaggatagcgagcctcaatgcaatccgctacttcccaccttggatgggactttccatcagggatgttacgtagccatcttttgcaatcaaaactacacctgccgcgttacacacggtaattggacggtggaaatccccatcagcgttacctcacctgacgacagttcctcgggggaggtccctgatcacccgacagctaacaaacgctataacaccatgaccatcagcagtgtcctcctagccctgcttttatgcgctttgctattcgcgttcctgcactactttaccaccttgaaacaatacctacgtaacctggcctttgcgtggcgctatcgcaaggtccggtcgtcatgaccagcaacgccctgtatgagctgtttcgacgtaggttaccgcgtgcccccgtcaacacggtcatgtttctcacgcgacgcactcgtgatgggttctgcggtcggttgacgtccatcgccacgaattcccactacactatgttcgtgttagatcacgggtccgtgcgcatcgagcgaccgagtcagtcagaagtggattgcgccagtttaatggaaacgctgaagcggattcggttacgaaattcgtgggtagcgtcagaagacgagctagatgtgagtcgcggggacgcgtgacacaaaacgcgttcaggattaacgtaggttttcgaaataacctacgtccgtgagtgacgcggtttcgtgttgaaacccgcgccggttctcacggtggtttatgatgaaaccggcgttggggatctacgcgggttcctcattcaacctgcgaaaagaggaagttgcggtaaaaccacgtcaataaagacgtcaatgacacctcaatgttgcgttggaacggtctttatatatacaaacgccgttatgttcagtgtccggcaagatgctcgggatacgggctatgctggtgatgctggattactactggatacagttgataacaaacaatgacactcgaagcaacaataccgataccatctttgtatctctccttaccggggccaacggagttactcgcacagccatcgggggtctgcattcaaactacaccaacttaaccgaggcattcagattcactccagcaaacacaacaactaactcttccacggagggtaattggagcgtgactaacctaacggagagttgcatcaaccgcggtgagtcctatctaactaccatctggcttctgaactgcgctgacaacaatacttattggtactctggaaatgcctataaccatacaattgacacttgtaaaaatacagtttcgggatatctcttcttcggcatgtgccagctatggaaagattgggttactaatgcttctcacgacactgtcagaattcagtcgttgggaaatgaaatacgctgcatgctgctccctagacagtataccctcaacgccacggtggaatggtacaacaaatctgaaggtgacgtaccagaagaatttatggactatgttatcctgacccccttggcagtgcttacatgcggactgcaggaagcttatatactcgacaagggtcgtagatacatgtatttgttttccgtgtcctgcgcgggaatcacaggtaccgtatctattatactcgtctccctatcgctgctcatcctcatctgttactatcgctgtggccggcttctgatatgcccacgcggctttgaactcttgccagaattcactgaggaagaggaggaaaaagaaaaattgttaacgtacaaggacattgaagtccaggtgcctatccgcacgcggcggctgctcgtcccttggatccgggagagcaaaatgtgggtactaccacccccgctgcctccacgacctccccacttaatagaattcccgccgtctcctccgccgtcgcctgggcccatgcacatggtggtctgcatgccagcatgacggactttgaactttgagccccaagcggtacggactacatattttccataaatctacactgaacttgagcacaaaaatactgacaatggactgaatatacagacttttatatgatccttgtacagatgtaaataaaatgtttttatttaaaactggtcccaatgttcttcgggaatcatggggtggggacgggggacgcggtaaggagcaaaaccgggtacatgggggggaacatcgtccagcagtagcaccagcggattgggtaggggttgctgcggaggtcggtcgatgacgatgtcgatctccatcggcagatccggcaacatctcttcgtctccctcaccgaccagcactcggcgctgttctggatgtatatgattttggaaaagcctccgacgagctcgcggcgcgtagaaagccaagcggcgcaagggccggcgagcccgaaagtccatgcgcacagatggcatgagtccttgagtgacggtggtgagctggggaacagggctacctcccatcgcgacggtgacagtggatccatgagagaggcgccgcacgctgcatggctaaataccgtgaatcccctgacgtcgtctttcgtcccgaacgcgtcatgttgggggcgaggcgtaaaccgtcgaggttgaaaaaccgcgtatctgcgacccgtccggactacgttgtttttcagaagcggccacatgacctcgagatgtcgtcacccaaggtatttaacggcacacagccagacgcgttcgtcagcagcgacgccgacaagacctcagcatggctcggaggctatggatcttgagcttactagccgtgaccttgacggtggctttggcggcaccttctcagaaatcgaagcgcaggtaaacggaatctggggaattcaacacaggtaagaaatacaaaaaataacgtgattgtgaacgcggttatcgtgtttttgcagcgtgacggtggaacaacccagtaccagcgctgatggtagtaataccacccccagcaagaacgtaactctcagtcagggggggtccaccaccgacggagacgaagattactccggggagtatgacgttttgattacagacggagatggcagcgaacatcagcaaccacaaaagactgatgaacacaaagaaaatcaagccaaagaaaatgaaaagaagattcagtaacagcagaccccaagggttaacgattatgttgactaccttgttttttattaaaaagctgtaaggttttgctctaaaaacaccccgcctccggtcttttttcttttgtattcggcacgcgaaacacggtttcttcccatagcctgtctaactagccttcccgtgagagtttatgaacatgtatctcaccagaatgctagtttgtagaggctatgcgggatgctgcggcggcgcgaccttccctctccacccagccccgtcaaaacacacgcgactcgagcggttcgtatgaaaaataaaaaacagctttttatttacaggaacggggaaaaaaaaggcacacggtccgtgggagacgcgggttcacgcgtcgtcaaaaagttggtggtccactccgtaaggacaggtaggcttatttagcttccgcatgctcctggttccgtaataaatgccgttttcgtggcagcgtgtcatgccgcgagtcacaaactccatcaaactgtcggccacgatgcaaacgtgctgattgttggcagcaaagacgcgcatacagtcgtccacgaagaggttgatcacgtcgtaggggctcaccaaccagcctaaaggttccacgtggttactgccgaccatgaccctccagtcgttaatctcgctccagtcgtacagccgaatcgtggagacgcgaatgacgctgtaatcacccatgaccatgagtcggccgcgatacgtagcacgccactgcgcgaacgcgtggatgtgcatgcagccggccagcgctctaagcgaggcggtgtgcggcagctcctctgggacggtgatgaagttgcagcgtcgcaaaccgatgttgagaaattcagtgatgctctcggccacaaaggtcaacgagtcagagtagatgtggtcggtccacaggtacatggcgcccgaggcgcccaggtacagttcagacggcacgttgtgatcgcccttgtgtttaagaaagttgtaggtgcagatgctgccgacgaaacgcagcggctcggggcagcagaggtagctggccagacgctgtgcatcccgtccttcgtcgcgcaccaagcgccagcgacgccggataacgaggcagcggtctttgggccagaccagggccacgcgttgcccgggtttccacggtcgcgacgtcttaggaggcctccagcggtcgagcagattgagaaaacagtccttgattaccgacatcgcggtcgcgcgtcggtggacaaaaagaaatcgggccgatccggaaaaaaaaaacgacggcaaaacaccgccgtgctcgagcgaagggtggcggagggccagaagaggcggccttgacggcgttggcagcgaaaaaattggcacgcgagtcaaacgggaagtagcgtcggtgttttatgccccaagcagcgtcgtcgtcactcgtggcgtcacagtcaacggtgctgacgtcctttggggcagtcgggcacgcgatcgtagatgccgttgtggccgctgaaacgtcggttttcaaacagcaggttaagtcccagacacatgaacgtgttgagattatctcccacccggatgtagcggtcgtcgcgcacgtcgcaggcgtagacggccccggtataggcgacgacgatggggataaggtcgacgggccagcgcaagtgaggaaagggcgcgttctcgcccttgaggctgacggttcccaggccgagaacgcgcattccgaaagcggttttgatgttgcgcagcaagtgaccgccttccacgctgttttcgaaacacctgaggttgcatagacgcagttccgttcccggcgggtacgtcaacggcatgaactgcccgtggtggcggatgatgaatcgcgccatggtatccaaaccgaggctccaggcgcgcaacagcgggcgaaagtagcgcttaaccaacgacgaggtcaggtagcgcatgcagtgcagggtctcgacggcgcgcagcccgacgcgcgcaaactccatgaggttgcgggccaggtagtagacggcggtgtcctcgcgtacatagcaaaaaacatagccctcgtccgagatgaggcacacagcggtcttcttctgctgatccggcgacaacacgccctcgttcacgaagcgacccacgaaggccaggcgcgtctggcaacacaggtagtgactccaagccttcacgtcctccggtttgaagtcctcgtccgtctcgatctcctgcagcactaggttccagcccggcggccagaccacgggcaacacctggcctgcgttgatgcgcacgtaagcttccagacagcccaggccgaactcggccgtgagcgccaggctagccagatcgctcatgtgacgcgccgagtcagtgggcgagcccgggggcccgtcgcacaccacgctccgtcttcttgtcctcaccgcggccagcgtggcgaggacactttccgcgcccgaggctgtatcttcggtttgcccgccggagccggccctcactatataacgtcccgcccgggtctcctccatgtatgcaggtaagcaactgagccgaacgcacctcagcagacgagaggatgtcgtcgcggcgtcgcagctcgtcacgtcgctctggcgaaccctcgacggtgatttatatcccctcgagcaacgaggacacgccggcggatgaggaggcggaggacagcgttttcacgagcacgcgggcgcgcagcgccacggaagatctggatcgcatggaggccggtttgtcgccctacagcgtctcctcggacgctccgtcgtccttcgagctcgtgcgcgagaccggcggcaccggcgccgccaagaaaccgagcgaaaagaaacgatcgtcgtcgcgtcggcaaccgcagatcgcagcgggcgcgcctcggggctcgccggcgacacccaaggccggcaagtcgcctaaagtctcgcgaccgcctagtgtgccctcgctgcccgagaacggcgccggcggcggtggcgacgataacagcagcagcggcggtagcagcagtcgcaccaccagtaacagtagcagaagtaccagtcccgtggcgccaggtgagccgtccgctgccgagggcgatgagttttccttctgcgacagcgacatcgaagactttgagcgcgaatgttaccgggtcagcgtggccgacaatctgggcttcgagcccagcgtggtcgcgccgcagcacgtcgagtatctcaaattcgtgctgcaagactttgacgtgcagcacctccgccgcctcaacgaatgcatacccatgccggccttcgcgctcaccagcctcgtcgaccccgtcttaaacaacgtagcgcctggcgagcgcgatctcacgcgtcggataatcacgcacgcggtgatcatcaactattactacgtggcgcaaaagaaagcgcgccacatggtggaggccatacggaccaccgtgcggggcgacacggtacgccgggtagccgcgcaggtcaacaaccagagccgttcggggcgtgcggccgcgctagcgcttcattttctcacgtcacgaaaaggagtgacggacggccagtacgccacgtctctgcggcggctggacgaagagctgcggcatcgcggcacgcccgaatcgccgcggctcaccgaggtttaccagacgctacgcgattacaacgtgctcttctataccgcccactacacctcgcgcggcgcgctctacctctatcggcaaaacctgcagcggctcaacgagaaccaccggggcatgctccggctgctttcggtcgaagagatatgcgaagagcacacgctcaacgatctggcgttcctagtaggcgtcgagcttatgatcacgcactttcaacgcaccattcgcgtgctgcgctgctatctccagcaccagctgcagagcatctcggagctgtgttacctcatctatgtacaactgccgtcgttgcgcgaagactacgcgcagcttagtgacgtgatctactgggccgtcagtcaaaactacgactacgcgctctacgcgagcacgccggcgttgtttgactttttacgcgtcgtgcgtcagcaggacgccttcatttgcaccgactacgtgtactgcgccctgcgtctgctggcctgtcccgacagacctattatcggtgacaccggcggcagcagtagctcccaacgcctcgtaggcgagtttatggtgcgcgatccgctgttgcgcgacccgcgcgccacccacctgcgccagaaactcatcacccgcgacatatgcgtggcgcggttgcaagcgcagccctcgagtcgacacattccggtcgaacacacgggtgtctcctccgtcaccctgctcaaaatctttagccaagtcccccccgacgaacgcgaagaagacacgttacgcgagatggctcttaaagcgtttatggaagcgaacggtaatcaccccgaacaaatctgccgatccccaccacccccgctgccaccgcgcgactatcctcaacgcgacgagcgggaccgtcaccgtcgcgaccgccgcgacagcggggaatactgttgctgatggtgggacgaaacagcagggcggaacagtttatgatagaaagtcacaggaaagtatgtgttgttttttttttaatgtaccaagaataaaaagtgcgtctacgaccaaagcggtgtgtggacgctcgtcctctctgtcttctccgggtttttttttcacgtgttttttccttcctattttgttacggcaacagcgctgatggcacgttgccggcttcgaacatcgcgtcggtgatttcttgcttgcccggcgtcacacggtgacgtagcagcacgcggctcacgtagcaggccgactcgcggatgacctggccgtcggcgtcgcgtcgcaggcccgagcggttgccgtgacgcagtctgccctgcgcagcgcgctccacgtcttcaaagtagctgtgtagcaggccgcgctccagcagctgcggcagcgagtcggcggcgcgcactacaaagttctcacggctgatctcgtagcacagcacgctgccgtcggccgccacgccggccacgctgcggtcccaactgaaaaggttggcgagtccgatggtgccgatgacgcgcaactgaccctgggtcaccaccagcagcttccagtattctacgtcgcgcggggtgaggatggtctcctccacgtcgcagacaaacaacgtgtagccgcgcggatagggcagatccaggtggcgaccgcgctggcggcgcataaaatcgtctaaattcaaaccgccgtcgggtgcgcgcctactcgtcatcgccgcgccttgtcggtcgatgaccccacggtgcttataacgcgccgccgcggcttcatgtggcgtgacctccgacctcgtgaggccgaaaacggcgtacatgaagacgctcaaacttttgaatgtgggcccggtagcgcaccgagggccccggggcggcgacgacggcgggcccgagttccagcggggccttgcggcggcagcggttggcgtggttgctcagctcggcgtccgagagcgccgagctgaactgcggcagccgcgtgcgatcctgcggcgcgtccccgtgtcgcagcgagtgccagagcaggcgctggacgcgcgccgtctcgggcgtcggcggcgcgcgacagccccggcgcagcttgaaaacgtgcaggcacagcagctcgcgcttgatgcgcagcgacacgctgcggtagtcgggaatccgctgcaccagctcgagaaagtcgcagaaggtctccacgaacgtgtcctcggtgaagcgaatgcgcttcagatcgtggacgtgtttgcgaaaccgcgacagttctcgacgttgcacggggttctgagcgagtcccttgcgcagcagcgcagcctcgcctttaaacagcctgatgagccgctgcacgtccccgctcaacatacgtatacacgccgtgtactcgtgacgtatactggcgcgcagcagccgaatgatacgcagggccagcacggcgttagaggccaggtacatggcgtagccgcgacgcgggttggcacaggcccagcccgcggggagcagaaagtagtcgtcgatcagcgtctgcgaccagtcggcgaagcccaggtcacgtgatacgctgtcctggacgcgggccacgtcgccggccgtgaggtggcggatcgccggcaggtgaaacgcgcccaggtgtcggttgcgctccagcctcagctcggcgtgctccaaacgggaatggtgggacgccaccgcggagggcgacaaagaggagtggtcattgccgtcgtggttaccgtcgtggttaccgccgttgtcgcgcccgtcgccgcactcgcaaaaggccgcgtagaggtccttcaatgccgcttcggctcgcgccataaacgtggcgtggaaaaaaacggcggcgcggtgcgtccggtacttgacgggcaacccgcggcacagggccgccggcaggcagcggccgatgagttcgcgctcctcgggctccagaaacaggcacagggtgccgtccaggcgcaggtacagctcctcggtcatcgagcatagctgccgcaagtaatgggtgcgcgtcccaaaggtcttgtaatcgagcaacgtgcacaccacgtattgccccgtggccacggccagagcgatgcgtttggcggcacgactgatctctggcaagtactgcgcctcgtgcaccagacggcggaaagcgccggcgttgagccagcgaaaatgctgcggatcgggcggcaagggcacgcctcgaagcgcggcccagacagcgaggtccgactcgagcgtcagaccgcggatgtcgtacttgccgtgcgccgtagcgcaggctgaatggaccagacagctgcggcgaatgtacaccatggcgtgcttgggatgtttgggcgccggcgttttctttttctgaccgccggcggccgccagatcctcgggcgtgcgacacaacaggccggcgcgcacagcctcctgtcgattacgaatcggcgtcaggtaggcgcgcaggaactggtgacaaaactcctcatcatcacgacagtcgtcgagatactcgtacgtggtgagcggatcgcgaaataggcgctcgtcaccgtcgtcatggtcttctttagcctgctcctccggctgctgggttggcagtggaggcggcggctgatccacggggttcatgactgagaggaagaagaaggtggcggcgaagcgacgcggagcgacggcggtaaagccagacaccggctatatagctagtcatcacagtctcctccttcacgacgcccccgtgccgctcacgctatccagcacgctacggcccgaaaacacgtactcgctgacgtcgtacgcgggcgatgtatggctgctcaccggtttcgcggcgacggttgcgctcgagtccaacggcgagaagcaaaaacgccgtgggcaacgaaaccagaaggagccctgacggataaaaccgcgcagcgtctcggccaacttaaccagcatcgtaccgtacagcagtacgtgaatgccgccatgcgcgtccataaatacggctttgttcacgggttccatccatccgatgactacaaaatgggcctgttctagcacgccgatcacgaaattgttggcctcgtcggcctcggccacgttccacgagccgaaagtgaaagtacaagcgggcgagccgcccaggcggatcttgctaccggcgtggagctgacatacgcgcagcagattggcgcggtcgtgcagtatctgggagagttcgtacatgcccgcaaaggtgtgcttaaaccacgcgccctctacgatctcatccacgtagtcgcgctcaaagaagctgtacacggcaaagaggccgttctcaaaaaactcgccgaacgagagccccagcacgtacaccttgtcctcgccgggcaggtacgcaaaggcgtgcccgtgcccggagacccagatctcgggcgccgtgtttgcgtccggcacgcattcgtacacactgacgaggccgataaagtacaagcggccagcctggcgcaggcacgagaagcgccggtaggtcttgtgatcgcgcaccaccccaaagtactgagtgtcgcccagcatgatgccgtgcagcggcggccagcacagcgggagccaacgacccgccgtggcgcgcacgtagcgctgcaggtgaaccccgctcgcacgctcgcgcggcttcgggcgcttgtgggtccaggcatcacgcagaccgcgccagatgctgctgaacttgggctgcccgcgcagatagagcgacgagagcgagtcaaagtagcccacgacgagcctgtcgggagacacaagagcgcgaaaatcaaacctagagcgacgacggtgaaaaaaccgaccagaagcgcgtgtctcaaacacgctactttcggttataaaaacaccgtcgccctatttctgggcgcgtgtacactgatgactcacctacgctttttgaacggcagtctcagctcgggattggcctcgtacagcgagctgcggtccacggggccgatgctctcgtagcgaaagtcgtcgatgagcagcgccagccccacgcgcacgaagcccctgaggtcgcgcgccagccgcaccaacttatcctgccccaccagcgccgcgtacacggtgcccgtgtcgccgcagagaatccgcacgcggtgaaagaaggtcttgtcctcggcgccctcaatttcgcccagcggcatgacgggctcgcgcgtgtacaacgaacgttgaaagcggcgcagcatcgaggccgagagccccagatcgcgcgccgtgcgcagcactagggaatgcttctcgggccagatgagggtcagttgcgcctcgcggtgcgcctctacgtaggcgcaacgagcggcggtgtcctcgcaggccagcaactcgcggaaagccagcagcgaacgtaggtagcggccgcgagcggaggcgcgcgagcggcggcacagctcggcccgatggtcgggatgcaccaagggcacgttaggttgcagacgcgcgcagatggattcgtgcaccgggtcgcagcggatcatgcccttggcaaaaaatccggccagatccgaggccaactcgtacaggcagtcctcttgcgcgtcgtaggcgaacacggcgccgtacgcgtccacgaacacctggtaccggcaggtggcgtgcgagaccgtgccaatgagatgcagagctcggaattcgccgaaaaagtcgttctggcagtgctccagatcgatctcggtcagcgagtgcggcgaatgctcgcccccgaccacgtagatgcactgcgagggccagcccagcgacacgcacgagccctcgaagcgccgcaagtaacgccgcaggccctcatagtcgcgtcgcacgcacaggtcggccaagtcgcgcgtgcaaaagacctcgggtaccaagcagcgtttgcgacgcggccgacgcgcgtgcccaggcagaggaggaaggcgcgacggcggcgacgacgaggaggaagacgccgtggccgccgagcagcccttgcgacggccggacatgccggcagtccgcgacgatccacaggagacaaaaaagcagaagcagcagtagcctcggcgacccgctccaccccgtcctccacacgctcagccgcgactgaacgccggggcgcgccgctacttgggtttttatagccatctgccccccgtctcgggcacccgggagcgatctacggagacctgacagcagttgggcaacacaagatagggaaatacaaagacacttttaataaaaaacgagactactttgtgtgtgtgctccgtaaactgtttattctccccctccgcttcgctctggatgggctccgggtccgtcaacacgcgactcgcgcggcaaaaggcacgctgttgacggcgcgagagcccgtcgtgatagtccatcatgccccggagatcgtgcacaaagcagctgtcgccgcgcagaaaccgacgcagcgtctccacgtgctgcagctgccggcgcgtatcaggagccgtcatcgctgatgtcgtcatcgccctgacaggcgcgtagatggcttcgcgagatcatgcgcgttttcaaccgccgtgacacatcaggtccatcttgagctggcgccgggcctcgcgcaggtgttgcacgcgttgtgagcgggaggcgagttcggcttcttgctcgaactcctgctgctcactgtccgagagggtgcgataaaaggcggcaaagtcctccaagtcggctacatgcgccctgggtctgacgctccaaagcgtacgcagtctgatgaagcggacccatcgagcgtcacggcacgccgtcttgaacgcggggcccgggaagaggttcttctccccggcgcgctcgggccggcgaggccgacgcggtttatatacaccgtctcggacggcgggacgccgagcccgcgccgcggccgctcatccggagacggcggaaaccgcgacgccggaggaaacggggaccggcaacgacggcggtggcggcgaccagattatgggggacaaacccacgcttgtgaccctgttgaccgtcgccgtgtcgtcgccgccaccgtcgtcgccgctgccgctcgtcagcttcacggagctgttgttaccgccgccgtccgtcgccgccgctgcggtggcggcgacagcgacgagcgaggtgggcgagaaaaccgcggagcaagaggtagcggctgcggatccggagaccgggaatgagagaagagaaaacagggagaacgaaggaggggagacgaggacgacaggcaccaccgcggtcaaaaggtcgcacgacggtatccctcgccaactggcagagcgcctgcggctgtgccgccacatggaccccgagcaggactatcgtctgccggcgcaggacgtggtgacctcgtggatcgaagcgctacgcgacgcggaccgcgacaactacggtcgctgcgtgcgccacgccaagattcaccgttcggcctcgcacctgacggcctacgagtcgtacttggtgtccatcaccgagcagtacaacacggcctcgaacgtgacggagaaagcttcgtacgtgcagggctgcatctttctctcgtttcccgtcatttacaacaacacgcagggctgcggctacaagtacgactggtccaacgtggtgacgcccaaggcggcgtacgccgagctcttctttctgctctgctccaccagcgagagctccgtggtgctgcaaccgctcatcaccaagggcgggctctgctcgtccatggcggtttacgacgaggaaaccatgcggcagtcgcaggcggtgcagatcggttttctgcacacacaactggtcatggtgcccttcgtgccgcacgcctgcccgcattacgccgtgcctttcacgacgccgggaaagccgggctgcggcggtgctccgagcggcgttgcggggttggaggaggcggcgccctttggacgggtcagcgtcacgcggcatggcgcgacgctgctatgtcgcgtggaccatctgacctggatcagtaagcgcgtaaccacgtacggacacaaaaaaattacgcgctacctcgcgcagttccgcggcacgatggacgacgacgaggcagcgctacccggcgaggacgaagcgtggatcgcgtccaaaaacgtgcagtacgaattcatgggtctcattttcaccgtcaacgtggattcactatgcgtggacgcggaacagcgccaactgctgggcaccgtggccacctccttctgtcaccgcgtctcggacaagatcacggcgcgcaacatgccgcgcgctttttccttctacctgctgacgagcgcgcagcgcgggtacgacctgcgattcagccgcaacccgtcactcttttttagcggcgacgcgctcaactgtccgcttctcaatgagcccaacgtgttttcgctcacggtgcacgcgccttacgatatccacttcggggtgcaaccgcggcagacggtggagttggacttgcgctacgtgcagatcacagaccggtgtttcttggtggccaacttgccacacgaggacgccttttacacggggctcagcgtgtggcgcggcggcgagccgctcaaagtcacgctgtggacgcgcacgcgttccatcgtgatcccgcagggcacccccatcgccacgttgtatcaaattaccgagggcgacggtaacgtgtactcgtacaaccaccacacggtgtttcggcagatgcacgccgccggaacaaccacgttctttctgggcgacatgcaattgcccgcggacaactttctcacgtctccccatccctgaccctccgtccgtcctcctttcccgacacgtcactatccgatggtttcattaaaaagtacgtctgcgtgtgtgtttcttaactattcctccgtgttcttaatcttctcgatcttttggaggatgttctgcacggcgtccgacggcgttttggcgccccccatgccggcagaacccggttgcggccccgtaccgctcttctggggcgacgataggtcgaaagccaccgttttcatgcccgtcgtgctcttgacgggggaacctacggcggcggtccccgtcgagcggcgtgattgcaaagccgcgctcgcccccggtttcaggatggagggggaggccacaggcggcgcattcgatacgctgcttttggccgtagacgacggtgggtaaacggtggttaccgcgggatacgtcggcgtggtcgaggcggcccggctgctgccggacaggcgacccggcgcgctaccgctcacggggaccgagggcggtcgacctaccaccgccttgccgcccaaagtaggtttcaaggaaggaacaccgacgcggctgccccggcctttcaccggagacgggggggcactcttggccggggacggagaggctgacgaaagcatggacagcggcgatgtggcgggggacacgacatcatcctccgtgggcgacaaaacggacgccgaggctgacggctgtcgagccgaagaagcggaagaggttcccgcgccagaagtcacgttccttgatgacgtcgttttagacgaagccggttgaggttgcaacagcgtggcgggtaccgtcgacggcgtgcccgacacctgtttctctagccttccctgaaccggcgtcgacgtcaccgtctgcgctcgggcggacgcgtgcggcgtcgcgactcgcttgcccagcaccggtttctggctcgtggatgtcgtcgtcattggagacgataacttagctttacgtattctggacggcgtcgactgctcgggcgtctgactgggaggcgaaatgacgtcgttgttgtaatcggacgacggtgttgtgtgtcccaggctgacgacggagccggtgtccgaggagtcgtcgtcttcctcctcgctgtcttcgaccggtgactctgcagtttggtcccttaaagcccaaacctcatcagcggcgtcccgagacgctgtttgtgtcaccgcggcgcgtggagtcgacggcctccgaggggtggtggacacggtgttttgagaagccgtggaagtcgtaggcatcctgaagggattgtaagccaggtgaggattcttgagggcccacgcgcgttcgcgcggccagttggcggggttcatatccccgggcaacggcgccgtcggagcccagggcgagttaccgttgaccggggtttgggtacccgcgaaggtaggtgtcggggccggagcgggggccgtggaaggattgacaggcgtcggcgtgaggatggcagcgccggcgccagcaggaacgttaactccggcgccgaacgtcaacgtcggttgctcgaacttgtacgcggtggtgacgggcggtttggcgctcgtctcggtatccgtgatgtccaccagcgtgtcggtgaaacgcggatcttgacggttggggggatagccatccgagctgtcggaatcctcgtcgcccgagaaaagatcccctctggtctccgtgagcggcctcacgtcccacgcgctgtcccgacggacccttcccgggctggccttggtcacctgcggggagacgagactgaaagccgcgtgacgctgttgttgttgcgggatgttcaagggaccgctggtcggtttctgactgcccgaggataacaggccgctgaaaatgctggaaacaccgccaccactagcggcgcccttgccgctagttcccggtttcttgatgggcgtaaagatgtttttctcgtcatcatcatcgtcgtcgtcctcatcggcactggagccaaagagcctccgggaggcgctcggtttacgtgccgggggcggtggttgctgctgacgttgctgcaggttctgctgcctctcctcccaagccttcagctgctgtttctcacgctgcaccacctcgtcgtccacccgtttctgccgctcgcgacgcttttcctcttcgtcgtaatagccgacggccgccgaacgggcagcgtgggcttcggcggccggtgccagagaaccatgggcctcgaagcggaacggtttgtgtcccttccagggactggcgatccagctccagccgtccagcggctgcgtggggacatgtttcttgggtaccgacgagaaggccgaaccgccgccgagcgagaggagattggcgtcatcgtcaaactccaacgacggcgagcgcgcgcccaaaaacgtgtgcgccgactgtgggaagctgtccacgtagatatcaaagtcctcgatgagcagctccaacagcgtgtcggccgagtcgccgttttccacggcgtgcttgaggatattgcgacagtagttggaatcaaaggaaaggcacatgcgcagctccttgaccagcagcttgcagcgctcctgaatgcgcgccagacatttgcgctccagctcctcccaagacctgcgcacgttcatgatgagacggcccgtgtacacgagcttgttgacggcgttgaccagcgccgtgttggcgtgccggtccaggttaaggtcgagcggtttcacgcagaacatgttacggcgcacaccctccaggttttcttcaatgcgctgcacctccgtatccttgaggtgcacaaaggcgatgggttccgtctggccgatggctgtgaccagcgtctcgcgcaccgacatcttggccagaatgaccgcgcttacgagcgcgcgttccacgatctcggcatcgtggcgcacgtccgtatcgaattcggtacggtctagcacagccaggtggtcacgcgccttaccacgatcaccgaacgggtaagtgtagccgcgacgcgccacggccacgcaacgcacctcgaactcctcgagcactgaggagaggtcggggttgtgaaaacgcagctcgcggtagtatcccaaccaaagcatgagctcgttgaacagcaccgtacgccggtgcaggcgtttttcgccacattttttcaggatcttggggtgtgcctcgagatccacgtcgggcttttgcgtgagatggcgcagaaagttgaccagggctaccacatcgcgccgctgtagaccgataaactgcaaactcatgctggcttttctccagaacccggaagcgtcgtcgccccggactgcgcccgcggtctgctattcgcccacgatggacaccatcatccacaactcggtgagcgccccacctagagggagggggggtagtttaatagcggaggcggatacgcggttttcttttaagcgccgctgacttgtttcttctgttttttcgccccgtgtgctgttccgcccagacccgcaacaacactcctccgcacatcaatgacacttgcaacatgacagggccgctattcgccattcgaaccaccgaagccgtactcaacacattcatcatcttcgtgggcggtccacttaacgccatagtgttgatcacgcagctgctcacgaatcgcgtgcttggctattcgacgcccaccatttacatgaccaacctctactctactaattttctcacgcttactgtgctaccctttatcgtactcagcaaccagtggctgttgccggccggcgtggcctcgtgtaaatttctatcggtgatctactactcaagctgcacagtgggctttgccaccgtagctctgatcgccgccgatcgttatcgcgtccttcataaacgaacatacgcacgccaatcataccgttcaacctatatgattttgctattgacatggctcgctggactaattttttccgtgcccgcagctgtttacaccacggtggtgatgcatcacgatgccaacgataccaataatactaatgggcacgccacctgtgtactgtacttcgtagctgaagaagtgcacacagtgctgctttcgtggaaagtgctgctgacgatggtatggggtgccgcacccgtgataatgatgacgtggttctacgcattcttctactcaaccgtacagcgcacgtcacagaaacaaaggagtcgtaccttaacctttgttagcgtgctactcatctccttcgtggcgctacaaactccctacgtctctctcatgatcttcaacagttatgccacaaccgcctggcccatgcagtgtgaacacctcacactgcgacgcaccattggcacgctggcgcgtgtggtgccccacctacactgcctcattaatcccatcctgtacgcgctgctgggtcatgattttctgcaacgcatgcggcagtgtttccgcggtcagttgctggaccgccgcgctttcctgagatcgcagcagaatcagcgagctacagcggagacaaatctagcggctggcaacaattcacaatcagtggctacgtcattagacaccaatagcaaaaactacaatcagcacgccaaacgcagcgtgtctttcaattttcccagcggtacgtggaaaggcggccagaaaaccgcgtccaacgacacatccacaaaaatcccccatcgactctcacaatcgcatcataacctcagcggggtatgagctttcctgttactttattcagaaagcaccagaacccgtcgccatttcccctcatatacggtacacgtccccctgatctgtcatcacggtacacagatttcgcccgactgcggacgccgacggccaatcgcgtggcgtaggagtggcgccccggcttcattataacgccacgtcggagcccctgcgcgccacaacgccgtccggcgcaacttctgtctcggcacggtacgataaaaacaacgtcccccgtcgacgttgttttctccgagcggtgatcgttcccgtccctctcctccctccgcggcccccacggcggcggcctgctcgcacggacctatactattaccgccccaccgccgtcgtcgtcatgaacttcatcatcaccacccgagacttctccaacgacgattcagtcctgcgagccgccgagatgcgtgacaacgtggcaggctcgatttccaaagcgtacaagggcacggtacgcgccgaaggcaagaagaagctgctgctgaagcacttgcccgtgccgcccggcggctgctcgcgccgcaacagcaacctcttcgttttctgcaccgagcgcgactaccgcaagttccaccagggcatcgcacagctcaagcgcgcgccggccgaactggacccccacgagatccagcaagtcacggccagtatccgctgccgcctgcagcccagtctccgcgagccgcccacgccggccgacgagctgcagacggctgtgtcgcgcgtgtgcgcgctcttcaaccagctggttttcacggcccagctgcgccactactgcgagcaccaggacaaggtggtgagctacgcgcgcgacgagctgactaaacgctgcggcgaaaaatcggcgctgggcgtggaagtgcatcaactggtagccctgctgccacacgagcgccaccgcgaactgtgccacgtcctcatcggcttgttgcaccagacgccgcacatgtgggcgcgctccatccgtctcatcggacacctgcgccactacctgcagaacagcttcctacacctgttgatgaactcaggtttggatatcgcacaagttttcgacggctgttaccacagcgaggcctaccgcatgctcttccagatcggtcatacggactcggtgtcggcggccctggaactctcacacggcgcggcggccgggccgcccgaggccgatgaaaacaacgacgagggagaggaggacgacgacgagctccgtcacagcgacccggcgccgcttcacgagtccaagaagccccgcaacgcccgtcgtccccgcacacgcgtgccgcctcacgagcaaaagcccgaagaaaacgaggaggaagaagaggagctgtttccctcctgcaaggcaaccgcagcattcctgcgggcagaaccctccgtctccaacgacgacggcaacggcggcgaacgctgcgacacgctagcgaccgccctgcggcatcgcgccgacgaagaagacggacctctagccagccagaccgctgtgcgggtcgccgcgaccccctcaccttcagtcaccccagcccttacccccgtcacgtcccccataaccccgttgtgtatttaacgtcactggagaacaataaagcgttgatttctcaagttccgctctggttttggtttcgttttcaaagggagccccatcatggcccaaggatcgcgagccccatcgggcccgccactgcccgttctccccgtggacgactggctcaactttcgggttgatctatttggggacgagcaccggcgcctgctgctcgaaatgttgacccagggctgctccaactttgtggggctgctcaactttggcgtgcccagccccgtatacgcgctggaggccctggtggacttccaggtgcgcaacgcttttatgaaggtaaagcccgtggcccaggagattatccgtatctgcatactcgctaaccactaccgcaacagccgcgacgtgttgcgggacctgcgcacgcagctcgacgtgctgtactcggatccgcttaagacgcggctgcttagagggctcatccggctctgccgcgctgcgcaaaccggcgtcaagcccgaggacatcagcgtgcacctaggcgccgacgatgtgacattcggcgtgctaaaacgagcgctggtccggctgcaccgggtacgcgacgcgctggggctgcgcgcgtctcccgaggccgaggcgcgctatccgcgcctcaccacctacaacctgctgttccacccaccgcccttcaccacggtcgaggcggtggatctgtgcgccgagaacctgtccgacgtaacacaacgtcgtaaccgaccgttgcgctgcctcacctccatcaaacgcccgggctcacgcaccctggaggacgcgctaaacgacatgtatctgttgttgacgctgcgacacttgcagctgcgacacgcgctggagctacaaatgatgcaggactgggtggtggaacgctgcaaccggctttgcgacgcgctttacttttgttacacgcaagcccccgagacgcggcagactttcgtcacgctggtgcgtgggctggaacttgcgcggcaacacagcagtccggccttccagccgatgctgtacaatctgttgcagctactgacgcaactgcacgaggccaacgtgtacctctgcccgggatatttacatttcagcgcgtacaagctgctgaaaaagatccaatcggtctcggacgcccgcgagcgcggcgagttcggggacgaggacgaagagcaggagaacgacggcgagccgcgcgaggcccagctcgatctcgaagccgatcccacggcgcgcgagggcgagctctttttcttctccaagaacctgtacggcaacggtgaggttttccgcgtgccagaacagcccagccgctacctgcgccgacgtatgttcgtggaacggcccgaaaccctgcagatcttttataacttccacgaaggcaagatcaccaccgagacgtatcacctccagcgcatctatagcatgatgatcgagggcgcctctcggcagacgggcctgacacccaagcgcttcatggaactcctcgacagagcgcctctgggccaggagtcggaacccgagatcacagaacatcgcgatttatttgccgatgtttttcgccgtcctgtgaccgacgcggcttcttcgtcgtccgcgtcttcgtcgtcgtcctcagcatctccgaattctgtttcgctgccgtctgccaggtcgtcatccacacgaaccaccacgcccgcgtccacgtacacctcggccgggacttcttctaccacaggtctcttgctctcttcttccttgtcggggtcgcacggcattagctccgcggacctggagcagccgccccggcaacgacgccgcatggtcagcgtgaccctcttttcgccctactcggtagcctacagccaccaccgacgtcaccgaaggcgacgcagcccgccacccgcaccccgagggccggcccacacacgcttccagggacccgacagcatgccgagcactagctacggcagcgacgtcgaagacccgcgggacgatctggccgaaaacctacggcatctctgaaagcggtttttcctctttttctacgtgtctgtctcaagatgagacgtcgatatcaataaaaataccgtcgacgtggtttttttaacagtgtggttttctttattgactagcgaagtacacagtttacgagtagaaaagacagggaaaggttatataaaatgctgtattatatacaaaaacatgcacataaacaaacgggaccatcgtgctcatcatcccctccttgatcagttgttcatgtaaacgtgtggcggggtgaggggcggcatgccgttggcggcgccgggaataatgtgccgtcgaccgacgtcgcacaccttgaaacgccgtcggcgcacgcagcggtcgcaggacgggatatcccagaggaagcccatgtaggtctcggggtcctcgtcgtgaaagcggtaggagagttcaaagtggtgcaacgagcccgtccgagctcgcagcttctggcgaacaccctccacgtcatcggtgcacagcgacagtgctgggctgtcacacagggcctgaagctcctgcggccacaggtgcgtggccaggggcgagtccgtcgtcaccagtttgacgcagtgcatcaggttctcggtgatggcgtcgtacaggcgactctcagcctcctcgtgcgtcatcacgtttcgaggcagcgacagctcgtcgtcgtcatcctcgtcaaacatgatcatggggtcaggggtttttttgggatgttgacaggtgggtgtcttttccagacgcacgatggcctcacgccggccgctgaaacggtggtttcggtgtcccttctttcccatgacgcaggtgaacataaccacgtcctcggccaaacggtagacggcgtccatggcggggtcgtagccgtagacgacgccgaaagtgtccaccaagacgtactggcgtacgaggaactctttgcgttctggcacctcgtggcccagcgcgcccaacaactggtggtaacaggtgatgcgcggcacggtacggatcatgagctccatggtctggatgctgccgcccgcgcggacgacgctgaaggatgtttccttgaacttcataacctctgtgttgtgggtccagaaggcgaaatgggtgtcgggacactcatcgaaagggtcgtcgatggtgtaggaagcgtagcctcgcttggtcacctcggccgacaggctctccacgtcaccgcggtagagcatgacggcgttccagtagtcgtcgtactgcaccatgggccgctggtagtcgcgcatagtgtggaagtggtcgcggtgacgaaagccgttccgcagaaagtccttcatggtgggtgccagctcgtagacgcagtcgcgcaggtcatcgtagcagtagatgccgccgcgctgcccgatgagcacgatgagttggtagcgcataaagcccggaccctcgacgaagccaaaggggtgcaggtactcctgacagcagacgtaagcacctggtagagaatagaaaaaatccacgcacgttgaaaacacctggaaagaacgtgcccgagcgaacgtcctctttccaggtgtcttcaacgacgtggggcttaccttgcgaacagacggtgcccatcttgcccacgaagggccccagggcgctgcgcgaacggagctggatgaagcagcgttcgggccaggccacgtgcagccgggtgccgcattcctgctccagaaagtcgttgagaccgttaaagtccccggctcggatggcgatgcagccgtaggccatcagcgtgtcccgtaggtcgtccatgacggactcctctaccttcgctcgccgacgctgcgcttctccagccaccgctgcggtcgacagactcctccgtccgccttcggagaactacggcgcggcggcacggcctttatagacactatcagcgttgacgtcagacgatccgatgaacgtcgttttttgtgctggaacttccctcgtcccgacaaatgtagcggaaatcttcaagcaaatcgcgacgaagtccgatgaggaggatgcaaaagaggctgagcaacgcgatgctgcccgccgccacagtacatatgctcaacaacgcccagtgtcccaaggcgcgacttttggctcggaggagagccgaacggcggtttctccacatgacggacaacgtggtccagtacgtccatcctttgcattccggtgtccagacgggaagcgttgtcatgttatttcccgtaactgtcacgttatgttttgttttgtttctcgtgagcttaacggtcctcttgagaaatcgcgggcacatgtcttgtagaaagatataatcactttccgcgtatttcgtcagtgttgacatcacggtggtagtgttttctgaagaagtagcgttgtcagtgacgtttgtttcttcccaacgtacgtatgattcgaacggactcgtgtgcgctattgcccgcaacacgtagctgtggccggtgaagttgagcgtcagttgtcccacggtcacgttcgtgtcattcctaaaacatgctacttctccgtgaacttccgtgacgtttatctcacgactctcgttcaagacacgcaggggaaaccagccttccaggtgatactgaaaaccaaatttaagcatgacgctgtgccatttccgtcgtgattgattaaacgttacattcaagggcagtctggcttcggtcccgagacaggggccgttgtagatttgcgtgtgattgcgtgtgcagtttaggtggcagttcatgctcgtggtgttggaagtgcgattaacgtccgtaccgtggtacgtacatcggaccgaaacaccgtgtcccgtgctccaaagcagcgtcaacaacagccacacagaaacctacgtggagacgacacgggactttttattgacggagactcacgtttctaccctcccctttcccgtaggtaaaaacccacgtttatcacacacgttgtttttacctgaaacccgcgcagcccgtggacgcgacaaaaaaccgcggcactagaaagaaaatgaaacaagtatgtttattaagcagcatgtggggctaataggggggataactgaggtatagcaactatgaaaaaatactacaaaaaaaaaagctgaacatggtcatctagcagcaaagttctccttctagaccacgaccaccatctgtaccacgtcgccctccccggccgtgtacacgacatccttcaccacgaccggcggcagcggcggcgacgaggacaactcgctctcgacggaggccgggacgacagaggacgggggggtggtggcggcggaggacgaaggggtggcggcggcagcgggatcttcttccgacacgggcaacggcaggctcggcggcgcggacagcacccgttgcgccggggcgtgagaaggctgagccccggtggcctggatgtgggccaacgaattggctcgcagcgagtcgcgatccacgaaggtcataggaattttcccttcgcggatccgccgctcagattccaggatggcgcgcacgtagctgttcaccgacttggcaaaagtgcgcggcccctccgtattcttgtcgcgacgcgcttccagcacctgcttttcgtagtccagctggtggaagaccatcaccaggtcgtccatagtgtgcgcgtgctgacggacgtgggagcgcacctccaccgggaacaaagcgttccaatactccagcacgatagcaccgtgccagaactgcgccatgctgggcgccaggaaaaacaggataccggagtcgtaggcgaacacgtcccacttgggcgtcatgaacaacaccagctgacgcgtgggccgcaccgaagcttcctcccaggcctcgatgaccccgaacatgatgagctcctggtccaacggggggcagtgtcgctccagccaactgatcttgctcaggttcatctgcagaaactcgtacgaagggtcgcagatgcacacgtagagacccgagtcgtgccgcagcctggctccgcgcttcatcagtttcctcaccgcgtagcgaagcgccaccttgcccaacgccgacgcctggatcagtccccccacgtccatctgcgtctgtcgccactcggcctcgtccagcaggctcatgatagcggcagtgctatgcgtggtcgtagtcatcctttctatccttctctatgaatagcagcaatagcggtaaagtcccttcttatactatcccggagtctgtggtttttttgtttacccctgcttactggtgagactgctgggggccgttgtgctgcagcatccgagctcgttgccgccgttgccacaggaaccggtgtctccgcagggcctttttgagggcttcgcaggcttctcgcgcaagtcctgagaggccctcggcgtcgatggggttcacctcgggcgtccgagcctcgttttcttcttcttcatcctccctttcctcctccgtgtcctcccgctctgtgtcctccgttacgctctcctccccggcctcggccaagagcgcggccaccaagtccacggaccgctcggtctccgagttctcaccgtcaattacgccatgttggcggcgtaaccggtgccgagaacgccgggtgagcgcacatgcttttttctttcttaaccaaggcgggagaggatcttcaaggcgttttcgctggatccagcggtagctaaagtaccaaaaggccagcaggcccacgctacctaacagattcacgtagactggagacataattaaagaaagaagtgaaacccgcgtgtgggtctcacgtcgtcttgaaacaccgtcttatatacatgaagatgccggacatgacgcgcccaagacacgtggggttttccccttaggcgacccggtttcttaagatgtttttcatcttcgcacgcgatgtactacatcaaagggtcggctgaccgaccgcattgacgcacagtttccgagtacgcgcgtctcggagcacctgacggtgagccacccaactcacgcggataggggacaacactgacgtgaggggcgattcacgtcactgacgggaataagacgggtgagggatttccacctttttcttaagtgtgactctctttacggtaaatcgcacctgtgacctcttaacccctcctccctggtacccgataaccgtgaaaaacacacaccacacgtcacgacaccgatcgattttctttattcttagtgtgatgataggtaagggcactcgtgaggatgtgcaattatcattatcaagcctttttcaaggcgtagtgatgatcgttgggcagaacccccaggctcctagcgatctgggaatagaaggaggagaacgagcccagggccagaatgcccacagtgtacatggcccaggtctccagaccgaacgtggcgggtcgcagcttcagatggtaggccacccgctccgagagttgtgaatgctcgttcaggcaacaggactgcaggtgggtgagcccaaaagcgctttcgtttacgccgcgcacgtgcaccgtctgggccgggcaatcctggtgttgcgcgcgaaagtggtcctgacaggaaattccgtctacgtggcggcgcgtgttgttacccacttcgatcaacaacgtgttatcggcaggatgatgcgagaacgcgacgacggtgttgttggaggtctggcggcaacagtacacgtcgagcgtcatgagggccatgtcgccttggtggtacacggcgtacgcccaaccctggaacacgagcggacataacggaccgtgagcggacgtcacggcggcggttgttaccgtcgtctcggcaggagaacacaataaactcctgatcctcatacacaggagtccaaccgtcagaattaaagtccgcggagccataaccgcgcaagtgaagccgatacgagtgttgctgaatttgttcattctgccgactgttgctcacgagcgttcggaggcggtgccacaggctgttggccattaaaaagtcctggcccgaatgacgacaagacagagcccgaggcgaagaaaaaggcgcccgtcatgaagacgtaggcaggggaattcccatatttttatggcttcttttaaaagtctgtatccgactccatccggcgcttttcccaaaccgtggtctcctcgtcgtccgactcggtacccaggaggtggtaagtcttttgccgcacgtagaaagctttcaacgtggagcaaaagatgagaataaagaccccgaaaacgaaacaaaccacgccgatcatgccgatgcagacgttcatgtcgacgtagccggcggtgctgttggcggtgcggcaaaagagtgtcatgtcgtgcgtgcacaaaaaacaacacacaccacaggccaggtcgtagcgtagttattattccgtagcagcaatgatggtacagtcaagcacatgctctatccccgttaccccgatgatgcttgcgtccccgttgttatattggcactgtcccggttaatcaccacggtgaacaccacggccaagaaaatgatccctaatatagcgaccactaagagagcaaaagtccatttccagccgttgtcaaagtacgcccccgtggtgggatgcatggtggcgggcatttccatcatgtccatgtcgaacgtgtgtcgcggcgacggcgaactaaccaggcagtacgggggtcgatagggcggtgggctgcagtcgggtggtggcggcggtggcgtggaaaccgtcgtcgggcacagacccatggcctgctcgtaggtggggggcgcgtcgtcgtgatcccggtcgcggagcatcggcgtgggctccatgtcggtggcagtgacggcgacggtggtaactgtggtggagacggtaccgacggcgtccgcggttcaccttcgagcaaagagccccttctttttgcgcaaacgacggcaaaacagttctctgggacaaccggtggcgcggtaagcgggtgccacgctttcagggtgggtaaaacagtcgcgggcgaagcagtagttgttgcagaaccgcaagaacccgacgcgaaagaagcccaggagtccgcgcgccagaaagtgcgcctgccgcgtctcgggatgcacgccgaagacggcgccgctctcgttcaccagtatggagatgtccaggcgctgctgcgactccaccggcacggcccgcaccacaaatacctgcagcacgttcagcgagcacgtctcttttaaccagttgccgtgggccggatcctcgtaagtctggctcccgttcaagacgaccgtcgtcagcgcctcattaccgtctcgccagctgaagatggaaccctcgcgcttcatgcacaggcgccacaaggccagcaggtcgcgcgccaacatgaactcgcgacccacgtcgccgccggtctcgaagcggacatagcccagttcttcgcgcagcggcgcgtagttgcgcaggccctcctgcacgaagccgcggaaaccggaccgcgacaccaggtacagcgattccaccacgggcgagtagacgtagacgcgaccgccttcgccgatgagtacgggtagcggtgggcggccgatggcttcgcaacgactcacagtgcccaccggcagcaggaacttgtcgcagcacaggaaggtcttctccaaacctttaatattgagatgtccaaagtaaccaacgcgtaacaggtcgcagtaggtgaagaaccaaccgtttggccagctgagacgcagcaccgtgccgctgacgcgacgaaccagcttctgcaggtccttgcgagcgtcggaggtgacagagcagcggaaggtctcgttaaccagctcgacagccagcgcgtcctccagcgtgcgttccttcatctcgtcgttgatgctctgacggcgccgccggatttcgtcgaaacgggccgcggaggcggcgaccgacgcggaggtcgtccgaacgccctctgtgacgctgccgtccggccagtcaagaaagctaaggctggcgctgcgccgcctaaagtgtccgatccgcgcgggacgtcgctgagggacggtggctggtctgctggggcgggtacggccgcgggtgtccgcggacacgttagttatacacggaattgagtcacgtggcacgttgccagctgaaaccgccgtcgtctccgccggcgttttctccatcacgggaccgcgccgtgcgcgcgttcccaggcacgcggcccgcgctctagccgcacttttgcttcttggtgttagggacgaactcgaacgttacagaatcctcgctgtcgctctcctctttcgcgtcgttgaagtaattgccggagttgcgatccaaaccgccgcctcctcctcctccgccgccgcccgatccacctttggacgtcaggtagctggtgatcttgtgctgctcgtatttttccttggaggaaagaccgtggtcgtgatcaccgccgccgccaccgctgctcattttccgcgtaccggaaccaccgccgccaccgcggtcgtgcttcttgccgccaccgccgccacctcctcccagaccgccgagacccatgggctcgttcatgagatcgttatccagacccgggccgtcgtcatgcagaccgccggcattggccagcgaagagaggctgccgccaccaccgccgccgccacgcgacttgccgctgttcccgacgtaatttttgtcgaagggatcgccacgctggaaaggttcctcggtgagaaaattctccacggcgaacagaccgttgcggctggccacgtacaacagcgtgtcgtgctccgtaactatacgcaacgtgcacggcagtttggtgacggcgcaattgagcagcgtctggtagaagttcttcagctgcacgttgatacgcatgtttttcacgccgtggaaactgacgcggttattggctgtgaattccagctcgctgccgttggtcaggataaacttgatggccggtggaccggcgtgcaccagaatctgcacggtgcccgtagggcagggcgcttttttaacgttacgcttgacgcgggtatgcggcccgatccacttaagcaggtcggccaccacgccgaaatctagatccacgtgcacggccgaattctcgctttcgcgcacaatgtcttggccgtgcacgcaggccgagctgaactccatattgaaatcgggcgcgcacatggagatcttggccgacaggtccgagatgtcctgcacgtagaacttggtcaggtccttgctggaagtcaggtacatgaaattacccagcagcggcgtggaattgttaatggtcttgggctgaaacgacttgtcagtgatgtagaggcatgagctgttaaaagtgatttttgacacgcagtgactgcgtaccgtttgcaagataagcgacggcgtgggcaagaaggtaaccgtggtgttctccttgagcgcacggatcacagatcgcagctgctggatagccgtcttgtacggcttcagccgcagcgccagcgtcggcggctccgagaggcgcgtcttgcgatccatcccggacagcgtgcaagtctcgactaaggagcgggcgcgagcgagcgaaagttttatagagagcacacacgacgaccgggaacgctgcgaagacgcccggcgtctaataatacagccgcgccgagccagcgggcccccgactaagaggcacagtacttatatactccgaccttaaagcgccagtggtaccacttgagcatcctggccagaagcacgtcgggcgtcatccccgagtcatagtagaaaaccagggccacgcactggtccacaaacacgctcaggttcacggccgccatttccacgtcgttttggatcgccggtgccgcctggaacagacactgcgtcgccttgccctcctcctggtgctgctccaaccacgcgtaattcaccacgggcacgcgcagcggcctccgcaccacggtggggaagtaacactcacggttgggcgggcacaatgaccacaccgtctcctcctcgaacacggtgccgcgcgaagcccacactgacggcgtcacgccccacagatgcgccacctcgtcgtcgggacccaccgccagaaactgacagttgcgcaatccgaactcgagcatgtcggcgcgcagcgcttcccagcgcgcgctggcgatggagagccgcggcaaccgatacaattcgaaaatgaatttgccctcttgatagatggtgcgttcgaaccactcgcagcgcggcaaacccgacttgcacaaatcgacgctagcgcgcaccgcggcaaagtacatgtgctcaaagatgcgctcgatcaagtcccaagaggcaaagtacgtgaaccctaaccgcatgagcgccgtgtgcaagccagccacgccgatgtgcagcggacgcagtttttccagcgcgctctctacccaccattcggacgccgacattagcgcgtccaagcgcgcgttgccccaaaccaccgcctcggtcaccaactcgcgcagcacgctcaaatcaaagtaacgtcgcgtgttccccaaaaccacgtcgggtagatgcagcttctgctcgtcgctacgcgcaaacacgcagcgagccacgttcaccgtcagccgctgcaccggcatgtcacactcgccaaagtggcacgacgccatatcgggactcaagcacggcggcaggcacacgctgtcggccataatcgagtacttgactacgtgatggacaaagaccaccgaggcacggcccttgagcgcgcacagcaacatctttttcagaaaatcgtccgtgttcacgaccaccttggggcacgattgctcgcagcgcgaatactctttctcgaaagccgactcctgacccaggtccgagagccgccgggagacaggccgcccaaacagcgagtagcgctgctcacgcgcacggtagcgcttcattaacacgctaggcacgttgaaagcgtagcaaacccccgtcaactccgacgtgctttctttgagaataaagttaatcacgcggatagcggccacgtcccacatgtccacaaacacacgtaccacgggtcgatgcacctccttctcgcgtatcaaatcgcagtatccccccaggcaacgaatcacgctgttcacatcggcgttaagtcgcgttacgttcaccgacacagaaacgccgcaactcaaggtactcatccacttgcacatggccgcccaactggcgtcacgcgagaaagggtcggccgagatcagaaagtcgtactgcggcacgcgatcgaaacccacggtagacatggtgaaggtggacagcgacagctgcccatcgcgacagcgcttcaacaccgattccaacacctcgccctcgaaacgcgcatccagatggaaacgatagatgcgcgagtgcctactgttctcgatagcggccgtcaacgccacggcgatgcgcaaaaacacgccgcccgggctctcgtcctgtccgtgcagttggcgacacaccttatccaaacacaaaatggccgcgtacaagccccagcaaccggccaattccacaaaacgcgccgtctcctcggccagcttgggtagatcctccatgtgacgcagcacaaaacggcgcaccgactcatcgcacagctccgaagcgtaacacagtggcgtgcggctttcacgcgcccagttggctttgaaataaaagcgacccaacagcaggtcgcaacgcggcgagtgacgaatcagacagggaccgtggcgcataatgagctgaaatagcctgaaactgcccaaaccggcactgtgccgcgacacggtgtccatctcgcgccacagcgcgttcctgtcggacggcagctcccgcgccggctcctgtacgccgcaaaagcgaaacttgccccagtagccgtgacaatgacactttttgcccatcaacatgcgcgtagcttgtatcggcggcgatactttgcagagcgaagccccgaaatcgtcctcctcctcgacactgtccagctccatcctggtcgcgccggccggattaaaggtgctcagaccgctactcacgcgtccaccgcgactgggcacggcgggaccgctgtcacgcgtcaacgacagcacagacggcgtgccgtcgggagacggcgactcgggacgccaactgacgacgccgccaccactcgtaaaacccgctacacatgctacaccgctcgatacgttggtatttccagcggacgcttccttgtcacccccgggcagcggcccctcctcgagctcgctgtcatctcccccgatagtatcagcggcgacctctgccgacgattcctccgtctcggtttccgcgctgcggcttggaatcctacctggccggcaccgatgtgcgggcaccgaggacacccgctgttcctcgtccgcgtcagccggattcataagtttacgaggaaaataacaaagaaatcaggtagatttcaataaagtgagtctagatggcgccgacaactacggtttataaagtctgtgtgcgatgtgtttttttcttctgtgtctcctccccgtatgctgtcagcgccgctcagacgaattctcgaaagtctcccaattcgacgctaaagttgtccaaacggacgacggacagtttgagttctttgtgtaccaggaacgaggtgtgaatgtcgtcagccaggcaccagcccagcttttgtatgaccccggtacacagagggatctggcgcgggcgcgtgatgcgacggttgacaaagctacagcgctcgcgggcgaactttccgcgtgcaacgtcgaccaaggtctgccagtgtgcgatgctggaggtgagcacgtagatgccgggacgtgtttcgggcccgtcatagtcatagacgatgattaaatacacgtattgcagccgtccccgggtctcttcccacgtcaggtacatgtctttcggtatcatcaacgcgaacacctccgttttgagcgtgttgtaaaggtagccgcgcatgacgcaggtgagcaacgaggtgatgcccagcgagacggtcttgacgcagcccagcgtctcgaggcggcggtgcagcagatgcgggcccaggtccagccactgcagcgcggcgcgcgcggccgaggccgtgtacacgctttcgagcaggcagcgcgtgctggccgagacgttggaggcgcgaatgcctaacaggtaaaggctaatgtagaggtgtcgcggcgagtcgcaacccgtctccatgcggatgagcagcgcgcccggctgcgcctcgaactctaccaggccctcgggcacgaagaaacgcgccgtgagcgcctggtgatcggcgtggtagagatagcgaaccgatatagtatttacctcgcgtttggctttgagcgccgtcactagttcattgtcctcgtcggccgggtcgcgcggccgtttggccaccgcgcgcgcgtccatgatggcgaggcgcacggtagatttcaaaaagttgatagagcagctgcgggcacgggccacggacaaagcggaggcgttaaataccgtgagccaattggagatcggcgcggtggatgcccaggacgtgaccgcgagcgccgtgcgcgccttcgtgggtgcgttgccgagctcgggctaccactttggcttcgtgcgtcagaacgtggtcttttacctcctaagccacgccacggtacagacggcgcgcgacccgctgtacgccgccgagcagttgcacgaacagctggaccgcttcctgcgacaccagcacgacggcggcggagacgaggaccggttgccgttctaccacaacggggccacgctgacggctttccagaagctgttgcagaccctgcgcgagatccagaccgtaatagccgaacagagcggcggcaccgcggcggcggcggacttgatcgccagtaacaacgcgtcgaccgagcgccgcggcaagaagggcggttcgagttccgggggccagcagccgctggtccgccgggtgatcacgcagctggaaacggctgccacggaggcgcggccctacgtcaattgtcgcgccgtggccgaactcctggacctgacctaccagcggctcatctactgggcctgcacgctcatgccctacgtgttgtttcggcgcgacaccgacaccgaactggacacggtgcttctgatgcattttttttacacacactaccgttcggttaacggcgatttggccgtggagtttcaaaactacgtcaagaacagcgtgcggcacatgagctctttcgtcagttccgatatcgacggcgaccagaagcccggtgccgaacacatgcgtgacgtcagctacaagctgttcgtgggtaatctgcaagcgcgtgacgccagcggcctcatgtttcccatcattagcacgcgcatctccaccgtgaacctttacctgtcgcccgaacgtatgtttttccacccgggtctgatctcgcgtctgttgagtgaggaagtttcgccgcgcgccaacctagacgcttacgcgcgcgtgtgcgatcgcgtgctggaagaccacttgcatacgccgcgacgcgtgcaacggctactagatctgacgcagatggtaatgcgactggtggaactgggtttcaatcacgatacctgcgcggcctacgcacaaatggcgctgatccagccggccagtcagaagagctcgctctttgtcagcgagattcgcgagaaactcatacagatcatctacaatttttacacgtttttcatgtgcctctatgtgtacagccccacgttcctgttcgaccaccggcggcggttgattttggagcagcatcgatccacgttgatcggctccaaggaggaactacagcacgtctggagcaacgtgacactgaacgtcaatacgcactttgcggttcagtacacggaagaagactttgaggcacatacgaagggtgccacggaggcggagcgcgagtacctgtatcgggacctgcacagcaagtggggcgtgcacctgtttaccttgcgtccgtctcgcggcgcggccggcgcggcctcgcctttgcctccgcttgacggcgtcacacgctccgacatcttacgcgaatgcgcgctcgttaatctgaacgaaggccgcgtcaactacgcctccctgctagccttcagccatcatcccgagttccccagcatcttcgcgcagttggtggtggtaactgagttctcggagatctttggtatcccgcagggcctgtttcaagccgtgggttcgccgcgtcttttcgcactcattcagctgtgccgtgtattgttgcccgagcaggtgacgctgtaccagaacctggtctccatctacaacctgaccaccttcgtcaagcacatcgacgccgcggtttttaagacggtacgcgattgcgtcttcgacatcgccacgactctcgagcacctcagcggtgtacccgtcacgcccaatgtggacctgctggccgagctcatggcgcgctccgtagcgcataacctgtacaccaccgtcaacccgctgatcgaggacgtgatgcgcagcagcgccggcagtctgagaaactatctgcgacatacgcgactctgtttcggtctggcgcgtggccgggcgcgcctctcggaggacggcgtgacggtgtacgtggaggtacaaggtcaatacggactacgcgtacccaccacgcgtttcgtagaacagttgcgcgagctggttcgccgcgatcggctgttggccgagaatctgcgcggcttgaacgagcgcctgctgagtgttcgcgtgcgcgtacgtcagatcagcagcgacacagaggaagtaagccgacacgccaagggtcaccgcacggtggcccagatgagcaaggcgctcaaaaagacggcctccaaaatcaaagtgttggaaacacgcgtgacattggcgctcgagcaggcgcaacgttccaatggcgccgtcgttaccgcggtgcaacgcgcgctagccgtctttgacgtactaagtcgcgagaacttggaacgccgcggcgcacagctctgtctgacggaagcgacgagcctactgcaccgacatcgcgcgctagcgccgatgacctggcccgcgggcacgggcgttgcggcggcggccgaagcggatcgcgccttacgcgagttcttggaggcgccctgggaatcggcgccccaaccgccgcgactccgcatgacgcccgacaccgatcacgaagaatcaacggcaggcgcgacgtccgtaccggaggtcctgggtgcgcgctacgaacccgcacacctggccgcgagcgacctattaaactggtacatcgtccccgtaagccaggcgcagcaggacatcttgtcttcgatcgacccgcccgccggctcgacatcggtgtccctgccgccggcctcgccatgaaagtcacacaggccagctgccaccagggcgacatcgctcgctttggagcgcgagcgggcaatcaatgcgtctgcaacggcatcatgttcctacacgccttgcacctgggtggaacgagcgccgtcctgcagaccgaggcgctggacgccatcatggaagagggcgcgcgtctggacgcgcggctagagcgcgagttgcaaaagaagctgcccgccggcgggcggctgccggtctacagactgggcgacgaagtgccgcgccgcctggagtcgcggttcggccggaccgtgcacgcgctctcgcggcccttcaacggcaccaccgagacgtgcgacctggacggctacatgtgtccgggcatcttcgactttctgcggtacgcgcacgccaaaccgcgtcccacctacgtactcgtcaccgtcaactcgttggcgcgcgccgtggtcttcaccgaggaccacatgttggtctttgatccgcacagctccgcggaatgtcacaacgccgccgtgtatcactgcgagggtctccatcaggtgctgatggtgctcacgggcttcggcgtgcagctgtcgcccgctttctactatgaggccctttttctctacatgctggatgtggcgaccgtaccagaggctgagatcgccgcgcgtttggtctccacctatcgcgaccgcgatatcgacctcaccggcgtcgtccgagaaagcgcggacacggcagcgacaacgaccaccgccgcaccttccttacctccgctgcccgaccccatcgtcgacccgggttgccctcctggcgtggcgcccagcattcccgtctacgatccctcgtcctcacccaaaaaaacacccgagaaacgccgcaaggacctcagcggtagcaaacacggaggcaaaaagaaacccccgtccacgacgtccaaaacactggccaccgcctcctcctccccctcagcgatagcggcggcctcttcttcgtccgcggtaccaccgtcctacagctgcggcgaaggggccctgccggccctgggccgctaccaacagctggtcgacgaggtagagcaggagttgaaggctctgacgctgccgccgttgcctgccaacaccagcgcctggacgttgcacgcggcgggtaccgaaagcggcgctaacgcggcaacggccacggcgccgtccttcgacgaagctttcctcaccgatcgtctccagcagctcatcatccatgccgtcaatcagcgctcgtgtctgcgtcgcccctgcggtccgcaatcggcggcgcagcaggcggtacgcgcctatctgggcctatccaagaaactggatgcctttctgctcaactggctgcaccacggcctggatctgcagcgcatgcacgactacctgagccacaagaccaccaaaggcacgtactcgacgctggatcgcgcactgctggagaaaatgcaagtcgtcttcgatccctacggacgtcagcacggcccggcgctcatcgcctgggtggaggagatgctgcgctacgtggaaagcaagcccactaacgaactgtctcaacgactgcaacgtttcgtaaccaagcgaccgatgcccgttagcgacagcttcgtctgcctgcgacccgtagactttcagcgtctgacgcaggtcatcgaacagcgacgtcgggtgttgcaacgtcaacgcgaggaataccacggcgtttacgagcacttggccggcctcatcaccagcatcgacattcacgacctagacgccagcgatctgaaccgacgcgaaattctgaaagcgctgcagccgttggacgacaacgccaagcaggaactctttcgcctgggcaacgccaaaatgctagagttgcagatggacctggaccgtctgagcacgcagctgctgacgcgcgtgcacaatcacatccttaacggctttttgccggtagaggacctgaagcagatggaacgcgtcgtcgagcaggtactgagactcttttacgacctgcgcgacctgaaactgtgtgacggcagctacgaagagggattcgtcgtcatacgcgaacaactgagctacctcatgacgggcactgtgcgcgacaacgtaccgctactgcaagagatcctgcagctgcgacacgcgtaccagcaagccacgcagcaaaacgagggtcgcctcacgcagatccacgacctgcttcatgtcatcgagacgctggtgcgcgacccgggcagccgcggctcggcgctgacactggccttggtacaggagcagctagctcagctggaagcgctaggcggcctgcagctacccgaagtgcagcagcgcctacagaacgcgcaactcgcgctaagccgcctctacgaagaggaagaggaaacgcagcgtttcctcgacggactctcgtacgacgatccgcccaacgaacagaccatcaagcgacacccacaattacgcgagatgttacgtcgcgacgaacagacgcgtctgcgactcatcaacgccgtactgagcatgttccacacattagtgatgcgactggcgcgcgacgagtcgccgcgaccgacgttttttgacgccgtcagtttgttgttgcagcaactgccacccgactcgcacgaacgtgaggatctgcgtgccgccaacgccacgtacgcgcagatggtcaagaaactggagcagatcgagaaagccggtaccggcgcatccgaaaaacgtttccaagcgttacgggagttggtttactttttccgtaatcatgaatatttctttcaacatatggtcggacgactgggcgtcggacctcaggtaacggaactctacgagcgatatcaacacgagatggaagaacagcacctggaacggctagaacgtgaatggcaagaagaggccggcaagctcacggtaacttctgtggaggacgtgcagcgtgtcttggcccgggcaccgagccatcgtgtcatgcatcaaatgcaacaaacgttaaccaccaagatgcaagactttttagacaaggagaaacgtaaacaggaagaacagcaacggcagctactggacggctaccaaaaaaaggtgcagcaggatttgcaacgcgtggtggacgccgttaagggcgagatgctctccaccatcccgcaccaaccactggaggccacactcgagctgctcttgggcctagatcaacgcgcccaaccgctactagacaagttcaaccaggacttgctgtcggcgctgcagcagctgagcaaaaaactagacgggcgaatcaacgagtgtctgcacggcgtgctgacgggtgatgtagagcggcgctgtcacccgcaccgagaagcggctatgcaaacccaagcctcgctaaaccacttggaccaaattttgggtccgcaacttctgatccatgagacgcagcaggccctgcaacacgccgtccatcaagcgcagttcatcgagaagtgtcaacagggcgatccaactacagccatcacgggcagcgagttcgagggcgactttgcacgctaccgcagcagtcaacagaagatggaggaacaattacaagagactagacaacagatgaccgagactagcgagcggctagatcgctcgctgcgccaggatcccgggagcagctccgtcacgcgtgtacccgagaaacccttcaagggtcaggagctggcgggtcggatcacgcccccgcccgccgacttccagcagcccgttttcaaaacgctgctagatcagcaggccgacgcggcccggaaagcgctcagcgacgaggccgatctgctgaatcagaaagtacagacgcagttgcgacaacgcgacgagcagctgagcacggcgcagaacctgtggactgatctggtcacgcgccacaaaatgagcggcggactggacgtgaccacccccgacgccaaggcgctgatggaaaagccgctggagacacttcgcgagctgttgggcaaagccacgcaacaactgccgtacctgtcggcggaacgcacagtgcgctggatgctggcctttctggaggaagcccttgcgcaaatcaccgcggaccctacgcacccgcatcacggaagcaggacccactaccggaacctgcaacagcaagctgtcgagagcgccgtgacgctagcgcatcaaatcgaacaaaacgcggcctgtgaaaattttattgcacagcatcaagaggcgactgccaacggcgcgtccacgccgcgggtcgacatggtccaggcggtggaagcggtctggcagcgactggaacccggacgcgtagccggcggcgccgcgcgtcatcaaaaagtgcaggaactgttgcagcgcttgggtcagacgctaggcgacctagaactgcaggaaacgttggcgacggaatactttgcgctgttacacggaatccagaccttcagctacgggctggactttcggtcgcagttggaaaagatccgcgatctgcggactcgttttgcggaactggccaagcgacgcggcacgcgtctctccaacgagggagtcctgcccaacccccggaaaccgcaggcgacgacttcactgggcgcctttacacgcgggttgaacgcgctggaacgacacgtccagctgggtcaccagtatctgctcaacaagctcaacggctcatcgctagtctataggctggaagacattcctagcgtgcttccggcaacacacgagaccgaccccgcgctgataatgcgcgaccgcctgcgtcgcctatgcttcgcgcgtcaccacgacaccttccttgaagtggtagacgtcttcggcatgcggcaaatcgtcacgcaggccggcgaacccattcacctggtcaccgattatggcaacgtagcctttaagtacttggcgctgcgagacgatggtcggcccctggcatggcggcgccgctgtagcggcggaggactcaagaacgtcgtcaccacacgttataaagccatcacggtagccgtggccgtctgtcagacattgcgcactttctggccacagatctcgcagtacgacctacgaccctacctcacgcagcatcagagccacacgcaccccgcggagactcacacgttgcataaccttaagctcttttgttatctggtgagcaccgcctggcaccagcgcatcgacacgcagcaggagctgacggccgccgatcgcgtaggcagcggcgagggtggtgacgtaggggaacagagaccgggccgcggtaccgtgctgcgcctgagtctgcaagagttttgtgtactcatagcggctctgtaccccgagtacatctacaccgtcctcaaatacccggtgcagatgtcactaccctccctcacagctcacctacatcaggatgtgatacacgcggtagtcaataacacacacaaaatgccccccgaccacctccccgaacaggtcaaggccttctgtatcacccccacccaatggcccgccatgcagctcaataaactgttttgggaaaataaactggtacagcaactgtgccaggtaggcccgcaaaaaagcacaccgcccttaggcaagctatggctctacgccatggccacgctggtctttccacaagacatgctgcagtgtctgtggctagaactgaaaccccagtacgccgagacatacgcctcggtgtccgaattggtacagacgttgtttcagattttcacgcaacaatgcgaaatggtgaccgaggggtacacgcaaccgcagctccccaccggagagccggtgcttcagatgatccgcgtgccacgtcaggacacaaccaccacagacacaaacacgaccacggagccgggacttttagatgtttttattcaaacagaaaccgccctagactacgcgctgggctcctggcttttcggcatacccgtgtgtctcggcgtgcatgtagccgacctgctgaaaggccaacgtatactagtagcgcgccacctcgaatacacgtcgcgagaccgcgacttcctccgcatccaacgctcccgggatctcaatctcagtcaactgctccaggacacgtggaccgaaacgccgctggagcactgctggctacaagcccaaatcagacggctacgcgattacctgcgtttccccacccgcttagagtttattcccctagtcatttacaacgcacaggaccacaccgtcgtacgcgtgctgcgaccgccctccacgttcgaacaggaccacagtcggctggtgttggacgaggccttccccaccttcccgctgtatgaccaagatgataactcatccgcggacaacatcgctgcgtctggcgccgctccaacaccgccggtacctttcaaccgcgtgccagtcaatattcagtttctgcgtgaaaacccgccacccatcgcgcgagttcagcagccgccgcgccgacatcgtcatcgagcggccgcggccgcagacgacgacggacagatagatcacgtacaagacgatacatcaaggacagccgactctgcattagtctctaccgcctttggcgggtccgtctttcaagaaaaccgattgggagaaacaccactatgccgagatgaacttgtggccgtggcgcccggcgccgccagcaccagtttcgcctcgccgcctatcacggtgcttacgcagaacgtcctcagtgctctagaaatactgcggctagtgcgattggacctgcgacaactggcgcaatccgtacaggacactattcaacacatgcggtttctctatcttttgtaaccgacactgacagtagcgggtaataaaaacaataggatttttatcgtttttttatgttacaaaacaacgtatcactttcacggtgatttattcttgctattccttttccccttgggctgtcagcgccgggtgcgcgacacggctaccatgcgcaacaggtccagcttaaaggcgcacttgtcattaaacaggctggacatgcgcgtgtacttgctcagcatggtggccaacaccgggtgggtggcctctgatatctcggtcggcagctccaaaacgacgttaacgacgtgacggtgtttttcgtcccgcttgttggccaccgtgggtcccggcgcggtgttagacatggggcaggccgtggggggaggacgaagaggaagccgctgctaaaccgccgcgcgcctgctgcacaatgtggccgccgacgtggcaggcggtctgtttaaccagcgcgcagccccgacacagcggggcgccgtcctcgctttccaaacagctgtcgcggtactcgcccgtctgacagcgcgcgcacagcaggccgtgcccgtgcgaagtgaggcgcaggagacgcgggaccgtcacgtcgcgtaccaccacagtggagtcgcaggtgcgtgccgcgcagggcagaatgacgtcgaaagccagccggtgatcgtacacggcacaagccgcgttgaggcccagcacggctttccagcccacgcgtacgcagcgctgtccaaagagcgtctcggagacgagctcgtagacgcgctgccgcaccacccgctgactgccgcagagcgagcagtgcacgagctcggcgtgcgtgttgaagatgacgctcttttcttgacggtcccgataatagaacatcgagttgagcggaaagttttgctggcagtgtagcttttccttacccaggttgaggcagtgtccgcactgccgacagaccacggccaccagcgagcgcgcgtccagatggcgctcgcacttgagtcgacacagacaccagagcggcaggtcgatgacgctgccgatgaggccgccgcgcagcgcggcgctgagtgcaaagaggacgatcttggtgggctctacgtgacgcgcctgctgtccggcgcccgcgtgtcctaccgccgcagctgccgccgtcgagcctcctccgcgcgtctcgtcgtgcagacccagtgcccgcaacggcaccaggtatcgcggacacgtgtcgcaaaacgtctgcaccgcttgtcgggccagtacgtagagcgggtttccgcagggtaccttcccggcgtaccggcgcaaggctgcgatgaggccccgcaactgcggcgaccgcggctgccgttggtgacaccactggttacggtggtatacggccaaatcagcgcgggcgtcgaagcgcttggcgcgtagtaatgctaggcacggcgagctggtggggtgaagcacgggcagccgaaggtccaccccgaaaaggaaacggtgaaggtcacctagcagcgaggcggtgacaccgtccaacaacgcgtgcagccgctcgggcgggtagagccgcagacggcgcagcaggtagtcggtgtcgtagcgttcgaaacgcagaaaggccatcgtgcggacggccacggtgtgcagacagtccatgctgtagacgtaagcgagaaacacaaagtagggcttggtcataaccatacgctgaaagagcgccgtcaccgcctcccgctcggcttgccgacacaccagccattcgcgcaggaagcgttggtagagacggtcgcccagctcgcgattcagaaagcgcttatccgtcacgaagagatgaaggacgcaagaacgtggcacgtgatgcaccagctgctgctggaggaccgccgacgtctgcgccgcaaactgcgccggtggctgcgacgtttctaccgccgcttcctccggctgcagcgcaccgcggccgatcaccagctgcacatggaaatggtcctcgtgaacgcagaggggcgcgaagagacggcgcagagcctggtggaactcatcagtcgcggtgtgcggagcgtgtcggagacgacgactggccatgaccgcgccacagcagagccagcaccagcagaagagccagcaccagcgggcccagagtcgcaaagcgcgcgggcagccacggcccagactgcggtcgcgatggcccggagcgcgctcgccaccacgatgacggtgcccaacgataaccagtccgctccaaggacggcgcgcacggcggagacggcggatgacggtgatgggtcgacacccctcgccgacgactcacgtgctcctccagaggccgacgcgcggaccctccgacgtcctggcccgccgctgccgctgccgccttcccttctcccgccagagccagcaactcctcctcctcttcatcagcgtctccctcgcttgcgcatccgcatcgtcccatacaggcctcacaacgacacagccgccacgaccccgccgccatgggtggcggcggcggccgaggcccggcagcggcgccgccagcggcgaccatggtgggagagcaactcggatgacgaggaggaggagggggagatgcggtccgagaggaccgctttcccgccgttcgcgtaagcgcggccgacatgcgggcgcgccacagggacggaccgctgccgctgtgactgcttacggtgacgtggttccggaccgccaacgacgtcgacgcggctttcttggcgtacagctcgcgcagcagattctcgtactcgccctcgttttcgggtccgaaggcgatgagctcgatgttgaagaccgacgccgaattggatttgcgcaccacgcacttcgtcagcactccgtaggccgagggcttgatctcctcgatgtccttgagcgtgacgatgagcgactcgttcaccttaagcacattgaactcacctacgtggcgcgccggcgaaacgagcttgacgggcgctcgtacaaaacagcagagggagacggcgcagccagtgtttttaaagataaaacaaggcacgtggtctgtgcggctctcccagtagctgagtagatactcgacacaatagaccgtgtctgtcttgagcatggcgtcgcacaccgagtaattggggtttttacagatgaggccggcatcggtgacgcgcagctcgctgggacccaacttgaggatacgccgcgtggcctgcaccagatcctgatggagaaccttgttcatctccatcgcaccgacgccaccgccgatttatttacccggcgccgactcgtcttttccctccaggattccgttaatgtccatgagcttgctgacgatcgccgttaatagttgcgtcttctcacggaggatctctccgtgactgcaggtcgcgcagtcgccgtgcacgtacttgaggaaggcggcgtacttctgacccgcgttcacgaaatttaagcgcgcgtccagagagggcagcaacagatcgtagacgcgcggcagcatcggctcgaactgtaatagcagatcgtcgtcaagatcgggtagcgcgtgtccgtcttcaccgtcctcgtcgtcaccacctcccccctcgagcccaccgctcgtaccagccgcgggctccgcgtcctcgtcgatcaccagcggtcgcgtcggcaccggagaatccacgtcatcctgcacgtcgttttcctcctctccgtcgtcatcgtccagaaacggcacccgctgcttagcccaggattccggttttagaagctccacatcgaagacgagagtggcatgtggtgggatgatgcctgggtgcccagtggcaccataggcataatctggagatatagtcagtttggctctctgacccacactcatctgggcaaccccttcttcccagcctcggatcacctcctgcttgcctagcataaacttaaagggcttgtttctgtcccgggaggaatcgactttctttccatcttcaagcatcccggtgtagtgcaccacacaggtctggccgcgcttggggaaggtgcgcccgtctcctggggagatggtttccacctgcactcccattcttttttccgcgtcctcaatcagcggcgccgatcgccatgaatccgagtacccacgtgagcagtaacggcccaacgactccccctcacgggccccacaccacgtttcttcccccgaccagcccggccccgtccaccagctccgtcgccgccgctaccttgtgcagtccgcaacgacaggccgtttcgcgttacagcggctggagcaccgagtacacccagtggcactcggacttgacaactgagctgctatggcacgcgcacccgcgtcaagtacctatggacgaagcgctggccgccgcggcggccgcctcataccaggtaaatcctcaacaccccgccaaccgttaccgtcattacgaattccagacgctcagcctcggcacctcggaggtagacgaactgctcaactgttgtgcggaagaaaccacgtgcggcggcacgcaatccaccgtactcaccaatgcgaccaacaccactagctgcggcggagccgtcgccggcagtagcaacgtaggacccgccggcgcttcggccgcctgcgacctagatgcagaactggccggcctcgaaacctcggcggccgactttgaacaactgcggcgactgtgcgcgccgctggccatcgacacgcgctgtaacctatgcgccatcatcagcatctgcctcaaacaggactgcgaccagagctggctcctcgagtacagcttgctgtgcttcaaatgcagttacgcgccccgtgcggcgctcagcacgctcatcatcatgtccgagtttacgcatctgctgcagcagcacttttccgatctgcgcatcgacgacctgttccgacaccacgttctcacggtcttcgatttccacctgcactttttcatcaatcgttgctttgaaaaacaagtgggcgacgcggttgataacgagaatgtcaccctgaaccatctggccgtggtgcgggccatggtcatgggtgaagacacggtgccttacaacaagcctcggcgccacccgcaacagaagcaaaaaaacaacccttatcacgtcgaagtgccgcaagaactgatcgacaactttctagaacacagctcacctagccgcgaccgcttcgtgcagctgcttttctatatgtgggccggcaccggcgtcatgagcaccacgccactcacggaactcacgcacactaagttcgcgcgactagacgcgttatccacggcctcggaaagagaagacgcaaggatgatgatagaagaagaggaggatgaagaaggaggagaaaaaggaggagacgatccgggccgtcacaacggcggtggcaccagcggggggttcagcgagagcacgctaaaaaaaaacgtgggtcccatttacctatgtcccgtacccgctttttttaccaagaaccaaaccagtaccgtgtgtctgctgtgcgaactcatggcctgctcctattacgataacgtcgtcctgcgcgagctgtaccgccgcgtcgtctcgtattgtcagaacaatgtgaagatggtggaccgcattcagctggtattggccgatctgttgcgcgaatgcacgtcgccgctcggcgcggcacacgaggacgtggcgcgctgtggactcgaagcacccacctcgcccggaggcgactcggactaccacggcctgagcggcgtcgacggcgcactggcgcgacccgacccggtattttgccacgtcctgcgtcaggcaggcgtcacgggcatctacaagcactttttctgcgacccgcagtgcgccggcaacatccgcgtcaccaacgaggccgtgctcttcggacgcctgcacccccaccacgtccaggaggtgaaactggccatctgtcacgacaattactatataagtcgacttccgcgacgtgtgtggctctgcatcacactcttcaaggcctttcagattacaaaacgcacctacaaaggcaaagtgcacctggcggactttatgcgcgatttcacgcagctgttggagagttgcgacatcaagctggtggaccccacgtacgtgatagacaagtatgtctagcgtgagcggcgtgcgcacgccgcgcgaacgacgctcggccttgcgctccctgctccgcaagcgccgccaacgcgagctggccagcaaagtggcgtcgacggtgaacggcgctacgtcggccaacaaccacggcgaaccgccgtcgccggccgacgcgcgcccgcgcctcacgctgcacgacctgcacgacatcttccgcgagcaccccgaactggagctcaagtaccttaacatgatgaagatggccatcacgggcaaagagtccatctgcttacccttcaatttccactcgcaccggcagcacacctgcctcgacatctcgccgtacggcaacgagcaggtctcgcgcatcgcctgcacctcgtgcgaggacaaccgcatcctgcccaccgcctccgacgccatggtggccttcatcaatcagacgtccaacatcatgaaaaatagaaacttttattacgggttctgtaagagcagcgagctactcaagctctccaccaaccagccgcccatcttccaaatttattacctgctgcacgccgccaaccacgacatcgtgccctttatgcacgccgaggacggccggttgcacatgcacgtcatcttcgaaaaccccgacgtgcacatcccctgcgactgcatcacgcagatgctcacggcggcgcgcgaagactacagcgtcacgctcaacatcgtgcgcgaccacgtcgttatcagcgtgctgtgtcacgccgtctcggccagcagcgtcaagatcgacgtgactattttgcaacgcaagattgacgagatggacattcccaacgacgtgagcgagtcctttgagcgctacaaagagctcattcaggagctgtgtcagtccagcggcaacaacctatacgaggaggccacgtcgtcctacgcgatacggtctcccttaaccgcgtcgccgttgcacgtagtttccaccaacggctgcggcccctcctcctcgtcccagtccacgccgcctcatctccacccgccgtcgcaggcgacgcagccccaccactactctcaccaccagtctcagtctcagcagcatcatcaccgtccccagtcaccaccgccgccgctgtttctcaacagcattcgtgcgccttgacactgtacggcagaaaagccggctccaagtgcaagcgccgcggcagcaccatgtgcaaaaacttgtccttgcgcgcggtttcgccgccgggaaagacgggcgacagcacgttagttacagccttgagaacctgctcaaagtacttgtcggcgtgaatgggcacgccgtgctcgcgcacgtagctcggatcttcggctacctcgtagttgcacacggccgacggtggtttccgcgccctcttctttgccggctctcctcctctcctgttgctctcctctaccccgccgccgtcagcgtcgtcgtccgtgccatcaatcgcgtccgaccgggaaaccacgccggcggttacagaatcaccgttgtcggaggaaccctgcggcgccgtccggacaccgggcgccgtcagaacgtaaaagacccgatccccgaccgagggtagctcctcagaacgggccgccaatcgcttaatgacggcaatgtgcggcaggttagattgacggtacagcgagatgtccttagagagcaccgacgaaagcaccaggtcctcgacacgcacacggtgcaggtacagatcgtcgcgggcctgcaccaagcggcgtaagatacgccagaaaccgcgtggcacgccgtacttcttgacttcatcgagtgagaggcgcgacaggcgcacggctgcttccgagacctcgcgatcctcaaagagcagcgagaggacgtcacgcgtgacgcccttgacgaactcgcaggccgtcttgcgcaccagatccacgcccttcatgctcagacccgaggcgccctccactttgccgatgtaacgtttcttgcagatcatcataagagagacgaagaccttttcaaactccagcttgacgggctccacaaaaagacaggccgtcacgtagtgcgccaggctgggcccacgcgccaccagagcctgcggcgtcaggccacgaaagcggacaaacacgctgtccgtgtccccgtagatgacccgcgcctccacccgccgttcgttcgagccccctgacgatgtttcgagcccctccggtaacgcgctgctctcctccgaatccccctcccgcgttcccactacatagtcttcctgattaaaaaaattgtgcaaaaaacacggctctgaaaagttgtctttgatgaaccgcgccgtgcgctctagcatgtcgcgaccgatgcgcgtgatgctggcggcgatgggcagacacggcatcataccgttgaccacgccggtaaaaccgtagaaagcgttgcacgttactttgagcgccatctgttccttgtcgagcagcatacggcgcacagggtcttgacactcgcgcatgcattcgcgcacggcacgccgctgcgaaacccacttgttgagcagttccgagagcaccgagacgcgcaccgaagcacgcacaaagcggtgggtcacgccgttctctagcgtgacgctgtatacgtcggcggggtccacagggtactcgccacccggcaccagcagggtggagtagcagaggttgtgggccatgatgatggaagggtagaggctggcaaagtcgaacacggccacggggtcgttgtagtaacccacctcgggctcaaacaccgtggcgccctggtacgaaaccgccgcagtaccgccggcgccgtgattgtcgttggaaacgccgacgccgccactactgccggagccgacgctgaaaacgccgacgctgctactactgttactgccggagccgggtgaaacgccgtcctgactggacggcgcagattgcaagggcggcgacatctgaaacatagccgccacagaacccgcgtcgccgggcacagcggcggtagagatgatagcagcgttaggtgacacagcaacgctattcgtttcgggcaccgtcgtacctttgctgtagtggttgggcaggataaaatcgcggcaggcgcactcgtccagcagcgaggtgtagatacggatctgctgtccgtcaaagatgacacgccgcaacggaattttagccagccgcgcgatggccccggcctcgtagtgaaaattaatggtgttgaacagatcgcgcaccaatacggcgtcctgcagacagtaacggcctacctgggcgcggccctcggcattagccacgaaacaacgcgggatgtccttgtaagacaggtcatccttgcgttgccgcaggtaaagctcggccatagtgttgagcttatagttgggcgagttagtcttggccatgcatacagggtacatgtcgataaccaccgaacccgcaatatacaccttggtggcggccgtgctggccggattgttgtgagaagccgagggaaaagcggcggcgtactgccgcttaaaacccacggcggggctgtgtaaaaagaaacggccgccctgcgccgtaggcaacttgcagaagcgctgcgagtccaccttatacaggtactcgagacgcgtgaggatgtacttcaagtcaaaagagttgatgttgtaaccggtcacaaaggccggcgcgtaccgttgaaagaaaagcataaagcccagcagcagctcgtattcggaagggaactcgtagacgtccacgtctgggcccacctgcccgcaggtgccgatcgtaaagagatgaagacccgagtgcccaaagatcacaccctccgaagtgcagccccgaccatcgttcccgtttgggatcccctgatccacggcggtgtttccccccgtctcgtagcacacgcacgagatctgaatgacaatgtcatcggacttctcggcgcagggaaaaccaccctcgccgctcatgcactcgatatcgaaggacaggcatcgatagcgcggccacgagctgtcgtcgggcacagccaccaggtcagagacatcgcagtctacctcgatatcacaagtcgacgcgcgaccctgctgccgccagtcgtaacgattcacggagcaccagccgaacgtggtgatccgccgatcgatgaccaaacgcgtcagcggatccacacggacctcgtacacgggaaaaccctgctccagcagatactcgccgatttttctggccatggtccagttgctgatagacacacactgcaaatcgggcacgggtcgcgtcccgtacccatagatggaggtcttggtggccggcgtgacagacacggcgtatggcgtccgcggttcgggcactagttcgcccacgctggcaatgacctcacgcagcctatcggtgtcgctgtactcacagtaaaagtagctgcgctgcccgaaaacgttgacgcagatactgtagccgtgttctgtggccccgaagaaacgcaacacgttccccgaaggcaccagatgctgacgatagcgcggcgacacgttttcgggcgagtcgaagaagagcacggcgtccgtctgatcgtaggtgtgaaaacgaataggtcccaccacgcgacccaccagggtctcgcgccaaggacacggccaaaccatgtcatgactcaacaaatgtttaatctctcgatagaacatgagaggcagccgtcccgtcttatgcttgatcaaccccgtctgaccgtcgaacatgacacctcgcggcacgatctgcaaaaactgtttctgtggcggccgcttgcccgagccctgcgcggagccgggctgcgaacgctgacgccggccacccgcgaccgcaccgccggtcacgccgccgctcagatacgggttgaaaaacatagcggaccgtgagaggctgacagcttacgaagcaaaatcacaaagaaaatacacatgcagcacctagatatccagtttaaccccgtatatcacaagtctctgtgtcaatattttttgtctagtttttttttcctcctggttcagacgttctcttcttcgtcggagtctttcaagtgtctgtagccgtttttgcgatgtcgcagccggtctagcaggttaggcttctgtcccttgtcctgcgtgccagtctgtccgtccaaagaatctgtaccgttctgctgcgctcgctgctctgcgtccagacgggccagggccagaagcatctggtaagcctgctcgttggtgtaaggcggagccgccgtggatgcatcagacgacggtggtcccggtcctttgcgaccagaattataaacactttcctcgtaggaaggcggagcctgtaacgacgtgtctttggtgctgcccgacgtcacggtggtcccgtcggcggacaccagatagggaaagaggttctgcagcggctgcgtgcacagacgccgctgtcgagtatagatcaaataagtgataatgactacggctatggccacgaggatgatggtgaaggctccgaaggggtttttgaggaaggtggcaacgccttcgaccacggaggccaccgcgccacccacggccccaatggctacgccaacggcctttcccgcggcgcccaggccgctcatgaggtcgtccagacccttgaggtagggcggtagcgggtcgactaccttgtcctccacgtactttacccgctgcttgtacgagttgaattcgcgcatgatctcttcgaggtcaaaaacgttgctggaacgcagctctttctgcgagtaaagttccagtaccctgaagtcggtattttccagcgggtcgatatccagggcgatcatgctgtcgacggtggagatactgctgaggtcaatcatgcgtttgaagaggtagtccacgtactcgtaggccgagttcccggcgatgaagatcttgaggctgggaagctgacattcctcagtgcggtggttgcccaacaggatttcgttgtcctcgcccagttgaccgtactgcacgtacgagctgttggcgaaattaaagatgaccacgggtcgtgagtagcagcgtcctggcgattccttcacgttcatatcacgcagcaccttgacgctggtttggttgatggtcacgcagctggccaggcccaagacatcacccatgaaacgcgcggcaatcggtttgttgtaaatggccgagagaatggctgacgggttgatcttgctgagttccttgaagacctctagggtgcgccgttgatccacacaccaggcttctgcgatttgcgccagcgcccggttgatgtaaccgcgcaacgtgtcataggtgaactgcagctgggcgtagaccagattgtgcaccgattccatgctggacaaatgagttgtattattgtcactcgtacttcttctggtcctatgagtgatattcagactggatcgattggccaaacgttccaattccaccaaagatttttgcttgatgccttgccagaacaccaccagaccgccgctggtttcgaagacggacacgtttccgtatttttcatatgtttgattgtatgaagtattgaaaatctgctgtaacttatttatagcctcatcacgtacgcagtccagcgcggagtcggacatgttcacttcttgtttcttagacagaaaagttgcagtcattttggcagaagaaaagtggtacgagtcttcggcttcggaacggatagtacgttccgaggcttcccagaaggtgagctggcaggtgacattcttctcgtcctgtatatcccaagagatcaccgagtcggcacgttcgagaaaagccaccaacctatgggtttctggcgcagcgttgggtcttccaaagtcggaaacgatggtgtagttcgggaaaatgaaaaacttgtcggcgttttctccaaagtagctggcattgcgattggttccgttgtagaaaggagaaatgtaaaccacatcacccgtggaagttgcaaaaaaatgataaggatacttggagcgcgcagtagtgatggtcagcatacagttcagattacaggtctcacgatagagccaggtgctgccgcggctgtgccactgatccttgaccgtcacgtaacgggtactgtgggtgttggaataatcgtcgggaattaattgcatggttttgttttcataactgtccctatgatatgccacgaaaaccgtgcctcctataacgcggctgtaggaactgtagcattgagcaaacttgttgatgtgatgaatctcccacataggaggcgccacgtattccgtattgctgcccagcagataagtggtgtagatgtaagcgtagctacgacgaaacgtcaaaaccttttggtagacccgtaccttaaaggtgtgcgccacgatgttgcgcttgtagaccaccatgatgccctcatccaagtcttcattgataggcttcatcgaggtgcagatgatattacgttcaaagcgaataagatccgtaccctgggccatagaacacacgcgataggggtacttggtagtgttgactcccaccacatctccgtacttgagggtagtgttgtagatagtctcgttggctctatgactgacggcttcagaagacgttacgtgttgagaatagactgaccgggtttgagcagacgtcgtacgagaagtatggcttccattgtgagtagaagaagttgcatgggaagtactagaagaggaaaccgcagcacccagacagacgatacacaggttaacgcagactaccaggcaccagatcctggattccatgttcgtcgcgggccaaatccagcagcgatgaggcgcgtcgtggtctcttgcgtgtcgcgcggaccctccgggaaacacccgcagtcgaggaggagggatacggacttggcagccaaggtcggtccggctccctgaagacacccgagacggccgcggcggccgtcagggtggagggcttggccacgggagctgttggcacgtcgccactctcatccggtctggacagatgcctgtagaggaggagatatagatctttggacttataaagacttccttcgtgacgaagcagcagcggccactctttgttatacgtgagaatcacatctctgtccgggtgcagttcgtcgcgcaggcacgcgatcgagagttgtttcccgaaagtttcattatatagtgcgacggagagcacgagctcccgcacgtgcatccacatctccttctgcagcacgtttaggtcctgacagtccgaaaaattgaaaaaacccatatacttcaccaccatccactcactgggatacacggtaccttccgcgcatttgaccaaatcgtccttgacgtggggtagtacgcccgcgttgtcgcaggcataggccatgtccacattgtgagagaggggataacgatcggtgcagtgggtgaagaggggcccgttacacaactcgtagatctgctgacccagtagcgggagggattccacaggcagactcttgtggatcaggttattgaccacatacaggtgctcatcgtaggtgaactgatcacccacgtccaccacgtcttggtcctggtggtattggctgcggtacagaaacccattcatgagcttagagataaagtccagacacaagggccccactagattgacatcgatgagcttgctagtcagacgctcctgcgttttgatgcaacggatcaccttgccatagcccacctccgagaccttctgcaggtaggcgcgtttgcgcacgttcacctcgcgagtgacgttgtggatgcgggagcgcgcgtccaccaagtcgagagcctcgtgttcgtcgcagttgcgcacccgtaagccgttctcgctgccgtcgccgtcctgcccattcacccctccccctaccactttcttgcctcctccacgagcccggccgccgccaccgttattcctctgactgtgagtactgctgttgctgctgttgctggccgtcatcaaagtcgtacccgtccccgacatcgcctcccgtccacgcaggtgaatagcctcgccctcggggccgtcgccccccgtgccatctggcagcggacgtcgaatctcctcgagaatatgcttgattttggtgtacatctcgttgctttcgtggagcttgttgaacaccgggttgtcctcgaaagcttgaatgctgagggatgtgatgaggtcgatgatcctgttgggggcggcaaagaccgaccccacgaacatgcgctcctccccgtccaacgccttttccccgagcacgaagatgtcctccacgtcctccccgtacagatggcgactgatgccgttcatgagcgcccggcacagctggtgatacacatttagctgctggatggtgatgcccacccgcttgacgataacctccgaggtacgggaccagtaggtaaaatccgacaaggaatatattcgttccggtatatccgtaaacaggttgtactccctcagcgcctcctccgcctcctggatgtagctgtggtaggccgatgaagaagagaataggcttttgagggccgaaaggactccagccaagtgggggatgcgcgttgtcaggtccagcaggtcctgctccaccgtctggatattcacatcggactggcttgacggacggtggaccgctatatggttgcacagcaagccctgcagccgcttgttcagcgagcggccctgattcgggatgatggtcagctcctcgtagcattgggcgcatgtcgtcccttcgacgtacacttcctgacgcgccaccggcgagatgccgcataggcgacggaggagctccagcaactgcgcgcagacctccaggccggcctccggcgccaggatcccgtacacgtagttcattttgcacaggaagcgctcgatgtcgttgagtgtggccagactgacgctgaaacggacgttgtccgtaaactggagctccacggtgtgatggcgatcgcagcgatccaaacggaggacggtacggtagaaggccgcccggtccggctggcgcgagtaggccatcagcgcccgatccagcaaagccgtatcctcgtgcagcgccttcagcagcatctccaggtagagcgtcagcaacgaactctgcgtacgattctgcgccaccacctccgggtagatcttccggtacagatacactatagccgccgcgtttctcttgaacggcgtggactccgccagtaacacgttcggatcgcagtactttagacactccagctccatggcgtattcgttgcatttcgaacacactacgcatagtttctgtaacaaattcatctccatgactcgactcgctcacgtacgagacgctgtcgtccggtctggcgccggccagagacatggagtcggtgcacaaataactcgcgggccgctcgctatgccgactgacgttgacgttaatatataacgacgtcgtcgacgacgcgggttctgctcccgaagctgttgccgccgcttgcggcgcaacctcctccaccaccgccgccgccggctcctccgcctcgggcgacgggggctcggagatgaccggctgtgtctgacactcctccccttcctcaggcggcccgggcgccgacgcgaatgtcggagtttgccagcgcggcggcggtctctgtctctggtgccgcggcgctaaccttcggggctgttgctgctgttgatgatgcgacgccgtctgtcgccgctgttgcggcggtagctgatacggtgtcgcctggtgctgctgtgtcggtggctgctgttgctgctgttgttgcggtctgaaaagcggccacgggggctgcgactgttgttgctgttgttgcgatgctcgtggctgcggcggccgttgtcgcggcgtttgctggcggttacaaccggctgcgtttggccggcaataacccgctgcccccgccgcccccgctgctcccgccgacgccgccagcctcgtcttcgccggcgttcacgagaaagcagccacctcccgtctcgccgggcacgccgaagcaaatggagttgcccgcgacggactcgccgagaagaagaccgccacccccgacgccggacgccgcgccgacgccactgggcgcgaagagcgccgacaggtcgtgcacctcccccccggcggcgtccgttaatcgctgggcgtcggcgtccagcacgcgtcgcaagttctccagcgaaaagtcctccacgccctgctcctgcaacgcggcaaacttgtccatcagcgacgcggccagcgcctcgcagccatccacgaagaagagcacatcgtcggacgcggggatctcctcgcgcacgctcagaatctcgtacacggccatcacttcggggtcgcaatccaagttctcggcgtccagcgccagcatgacgcggttttttataagatccgcgtcaaaaagcacgttctcgcggcgcgagcgtttgatgagcacgtcggccagacgcgtagccaagaggtagcgctggcgcatgaaacgataatcttggccgctcatagagctcacgttaaggctgcgttccacaccgttgcccgaaaagtagccgatctgcccaaactgatagatctccttgctgttgttgatacccgcatatttttccacgctcacgggcacggtcaccaaggaacgatgctcaaaaacgctccgtaccaacgattcacgcgccacagtggcggccatgggcgccggcacgcctgcggtcttcaagcccttgacatgcaacgcaaattcggcgggcgacgagaaccgcggactagcacctaacacgtgaggaaactgcgcgtggttctgcgtcgttaagcgcgtcgtcaacccgtgcagcgagccgatgtagtctttgaagccataatagcagaggaatttgttatggaaacggctttccacgtaactcagcacacagtctggcgccacatccagcagatcgtgctcctgatagtcagccgtcacagccaccagaaatttgacgaaagcattgaactcgcccatgtcacctatgggcacattcttgggcaacgcgttggaacagaccttctgccaaaactgtaagcaggggagaccacattcaggaaagagtcgctcgtgatgtcgatacagcagaaatcccaagcagcccttagccggattacgacgcggaacgtgatcgcggcgaaaaaacacgctacccgcgttgcccttgcccgcgcggtagatgggtcggtttttcacccgcaccatgatcaacgtgggtaccgacagccgcgagagcttgatctccatgggcaccacggcgtacgtgccctgcgcgtacagcctaaagtccagcaggcggtcgtgatccgaattcttggacgacttgatctgcttggtgaagagaaagcccttgcgcgacgacgtggtggagaacgcgccgtgaatggattgaaaatgctgcgtcatccatttggataccaagttggtggtcaacggattgtccacaatgtatgaggtagcggtaataagcgccacgttctggatcacgtaaaagacggatctgaaataggcgtaggctagcagcggctggaaggccacggcgtagggattcagatccaggttgaaggcctgcgtggcgcccgccacctcgtcgcggctgctcttgaggcgcacctccgaaacgaaacccagggcctcgtcgtccacaaacttgttgagcgccgaaaagacggccacaaagtcgcttttgccgtgcgcgctaaaggtatcctcgcccgtcacggggtcgatgagccgcatcttgcggcagtaatccaagatgcgattgagccgataggtacggtccacgctagcgcccaacatgcgaccgccgcgccccatcattcccccggaatccccaccacccccaccaccacgaccgccacccagaccgtcgctcgggcccccgctcacgtctcgtccaccacccccgccagcaccgccgcccggaaccccgtcgtcacctttgccgtccaaacccccgtccttggcgtcgacgttgtaacgccgaccgaagctgcccaaaatatccacgtcgttgagaaaacgcgactgcacggtgatcacgcagggctccttcttgggctgcttgggcaccacgggcaagcgggtgcgcacccgcacgaaggccgtctgataacacgtgtggcaacaagtacccccacaggcctcgcacagccccgcggcgcagcccaccaggtgattcgtgagcgtcgacgaacccgacaagcccgtgttgtacaccgagacacgattcagataccagacgaagcccgaaactagctgcggacacgtgccacacaccaacgccaaatgctgcggcccatagcgttcgtccttgagcggcgcgccctgaaacttgagcaccttgcgcgcgtcgttgtagacgtcttcgcaggccgccgacaacccgttggtgaactgaatagccttgagcaacgtctcctgactggccgtaccgccggcgctgggatgccgcgccgacgactggagatacaccagcctgtgctggtagagcaccgaattagcgctgaagaccaaggcggccacgtgcgtcgagagatgcaacttgagctcggtcagcgcgcggatcagatcgcggtgatcggttgcgttggtcactaaaggccactcggaaaagagcatagattcggcaggttggtaagccgaatcgaaaaataccgaggcaaaactgaaggccaactcgcaaaccaccgcgtcactcagcatcagatgatccttttccagactgctgagtcgctggctcatgtaccccaagtagcgcttatgtggcgccagcttcaccgactgctgactgtcgtgcacaaactgccgcaacgccgcctcgatcagcacacgcggctccgagaagcgcagcgattgacaccatgacgtgtacacgtagtagaaaagcgtctcgcttacggccggcacgtagagccctcgcgcctccacaaaagcgctgcgcgcatccagcgagacctcgtcggcttcggcgtcaagctgcaacgaattaaagagcgtaggcgggtacaacggcacgcgcaccgcctcgccgccgtgcagtcgcaccgtggtcgcctcctccacgcatggaatcagctgaccggcaaagagaaactccttcaagccgttgcccaccaccacgtgcacagtcgtctcggacgcctgacagcccaccgccgcgcacaacgccgccagatcggtaggcacgcgatccgcctcgggcatgtaagcctccaacgcgtacttctggcgggcgtcctcgcacagccgatgcacgtctccgtgatcctcggtaaaagccacgatgccttgcgtatgatgaaagtagagcgcaaaaggacagaaggacgtgactttcgtgagcaccccgccgtcgtaacaaagcacaggcgtgcgcacagagacgccgaaatccgcctccaccgtgagccccgccaacaaaggagcgatcaccacgctcgaggaacggtcgcatagcgagagagtggccagaatctcctgcgtttctgcgttcaacctgctgaagtagagaaaagccgcgggccccaccggcgctagcgcggttagttcctcgtggctcatggtggatgaacggaagacaatggctacgccgccactgagtgaattttataccaaggaaaagttcagcacgtcatgtttgacgcacgacgtctgagacaccaccgtggccaccactgcggtctggctgcggttgcggaccaccaaaggcgacaaccgcaacgatcccagcaattcgtaagaaaagctaaccgctacggtcaggtagcctctcgcagccagaccgctagccgacgcacccgcccgcgaaaatagcgtgatgttcgggacggctttgcgtcaccgccaactaacgtcggtagtcgagcacgtcgtttatcctcagcacaccgtccgatcacaatccgttttcccactcagtcgcacaagcagcacataaaaaccccacacagggcacgtgaaaacaccgtccctagaaaacggcgttttctgtcctaccgtcacccgtatacacaggcaaatcccaatcccgatccccgaaaacaccgtacggtgtttgtgacctccaaaatcacatcagctaacaaaccgtgaaaagtcacgtttcacgaacacggtgtttttaaatcacaaagaaccgcctgacggtttacaagcagaaacaccgcaccacggtggtacaagcgcgatgaatctggtctcgcaacctcaatcgccgctatcaccaccgattttcgctgcgctccgccgacaaaacgccgtacaagctacacaccccaaaaacccgcgcgcctacgggcgccaaacctgtgtgttatctcaacgtcacaacacgacacaaaccgcgtaacgtggtttcccgaacacgtacgcggcacagacccccgacacgtactcgaagaccttacagtttacgagtcaataaaacaggaaaagatccgaactttaaaattgtgtgtttttattttcccatccccctctttttaccaaaaaacacatttttcgtcttgtaaaaagtaactttcgcccattgccatgaaacaccgtgatggggaacggtgttgtgtgtcgactgacgtcactacggcgatcagtatcgacgtcgtgtatacataacggtgcccggtgtttttattcggggcgttgtcgcgtcttgatgtaatgtaacctgaaaccgccgtgcccaagaatgcggaagccagcgtgtaatcataacggggttttgggtacaatctgacgacatctggcggcgagcgtacaccatcgaatgtggcgatcgccggctctacgtcacaatgacgcaaaaacacactgtaaaacccgcgtagacagctttcctggtcaacgagcgccatctggtgtcggcataagaacaggcatcaaccccgtggccggcgaggcggtgagcacttttgttggtcacgtgaccatcagcgcaggaagcgaggcccgtagaaccgcccaagaggcggtgccagatgccaacgtcataatcacaaggtgatttgttacgtcacgcgcgcgcacgcacgcgcgcggtagaatacagcgatccctagtgaagccacacccattacgtgtagccatatccgcttacgtatacagccacacccctaggtacgccaccttatctaccaatcacagaaacggatatacaatgacccctccctagactccaccccttgtacggaaatttcagataggtggaacccgttagggttccaccgtcctcggtgtacgtacaggcttctccgtctaccggaaatatacacctgctgacgtagacgctactcccggatacgcgtcataagctactggaccctaggggggagtgtctacagggctacgtgcacgcccccttacctagggtatccgcccccttcctctgttttggcctagtaaacttaacgccgccgcttctcacgtgacccctgacaagcctacgtcacactcgcgtgaccacacccactccggatatacgtcatcctgtggaattccggacatacggtgacgtagcgagcgtagcgagctacgtcacgtatgcgtgcgtcatctccggcggaaatcatctctgatgacgtagcgagcgaagcgagctacgtcatcagtccgttttacgtataccggatgctaggcgacgccccgtaggggcggagcctagcttccacccctaggatgcataccctatatagcataattcttctaacgaaacgttctacgaaaacggactggcggaacgggaaccaccgtaacccccccccctcacccccccccttctcctccggaaccggggggggcaaatttttaccaaatttgggcaaccatgatttccaatgggacggcgtttccgtgcgcatgcgcagtcggggcgagtttttggttgtcagggcgttgccacgcggattatgggatggtgactcgagtgcgcatgcgccggggatgccgcatggaaaacctatatataaggaggggtgaaccaggggccccggggcgcatgcgcgggccagggcccgcgggagggtcgccctgcgcatgcgccggtaaaattccactgtgtgtgtcgtgcgcatgcgccagtatttttccactagaggcggtcagtgcgcatgcgtcggtaaaattccactagatgtgcgccgtgcgcatgcgccggtatttttccactgggcggccgcacctagggagcgcgagccccgtgccgggcatgggccgcggcggtggaaaattaccgctccgcccacctaggcggggcatctgaaaacctataaaacccggcgtgcccgccgccccccggcgcagtccgcggcagggttccggccgtgctgcggtccgcacgctgcgcccgctcccgcctgcctcccgccctaccccccaccctccccggccgaggcccggcgccggtccgtccgcgggcccgtcccaccgccctggagcaccatccggggccgtgggccgggcaccgggcgcggcccgctccggacctcggccgggggtccctcccctccccccgctcgacccccccatccgacggcccggccgggctgggacccccgcaccggggtcccggttcccgtccgtggcccggggggacccgagcgggggcttcccacccccaccccgctcctccccgggctccggcccgggatccctcgctgctcccggcgacctccgccggcttcccggtccacccgccgcggaatggacgggacccggggtccgcgcccttcccctccccccacggggggctgggtcgcggaccccggttcctaggctcgttccgcggtgggcgaccggggatcccccacccagctccccttcccggcccgccttgctggcttttgggcccctgcgggctttttttttccggctgggggtcgcggcggtcggccgacgacgacggtaggtgggccgggtggacggtggtggggacgggcgacgccccggctcgacggcaatcggtcccggaaggttgggggctgggggcccggtcaggagctccgggagcggggtcgaccgcgacggcttccgggtctcgcggcggctccctctcggcggctccggttgggctcccctcccccctctcgagggtccggccgccagtcgtgaccgggggtccctcggcctagccgccggctctcggtccgccttatcctgggcgttggcctgtcccgtgacgctcccctcccccgctgctccccaaaaaaactccgcccgaaccgtcgcggcttgctggccctgggcgtggtcccccactcccctccccccatcggccgcccagccggggtcggcgcctcggaccccaccaggctgtggcgtgtgtgctggccgatgcggcggcgaggttgggtgtggccggaagcgctcggggtcgacggtgggccgccatgacacctcaattgtcgtcagtacgcccctccacaatcaccgtccccacacgatgggcccggcaggtcacccaacgttggttcaggcccagtcgggttttttccccggcacgaacgcacgtccccgtgggctccacgcgttttccaccctttcctggaggggtccggaacaccgtgaatccacggggagggtcccggcacgggccgaggagaccacgaccgtcccacccggcgtgtcgactcgtccgagacccgggaagggaacaggccccacctttttttcccttctccgattttgccgtggaaaacccgtgaaccgatacgggtgcagacggccgaaaaaaatcgagacgacaatatgacggcagggcgcgatcttctcccccatccgacaaaaccgtgtcccttaaaattccccacctttctctgttcaaatggccccgaaactgtaaaacaccgtttgaccgcaccccaaccggcgccatcttggtgaccttctcgacggttctctcgctcgtcatgccgttctgagctccgacatggcggacgagagaaaatggcgtcgagagcctaggagcgtttttgctccaggcgggtaaaaaaatagcacgataacttttctgtgcttttttttgagacgttttagaagagcttttttctgctcagagcgaaaaaatgatagccctgaaaatctcgacgagtctggccgagcggcgccatcttggaggaggggcgagtcgcgggcaccgcctcggtaccccctggccgaggcgagtccgcggtcgccgcctgttccgtgatgctacctagagggcgctgtcgaggcgactcttcctgttttcgccctgagggctaacggtcgctgacgtcaaaccatctcgtgctcgctgagtcacatccggttgttgacaagcgatggaggaccgcacccaaagtgcgccctctagtcatcgcgcctgaccccttttataaactgctcgaagaaaagaacaccttatgtgaaaaaatacagaatgatgacaagttcatccaacacaaccgctcaacaacgccatatctatcagtgtccaaaaactatcttctatcctttgaaactataaatgctgcctatatacatatttagtatccaagactcttaccacgtagacgaaaagaagtgatacaatgatcttgacgtgtatcgtctatatcgtgctagatatattcagataagacgcgcaaaccatagatttctcatcagtatcatgaaagacctatagctctatatacgaacctagtcattttaggacagccgccggagaagccgacgagggatcgggcgggtgcagccagaacctcacgcccgatcccgcctccggtaggcgatttgcatctgtttggtaaaaagctcataagtctgtatgtgacctatatatattatacgctatgtacaccgaactgtcgctgttgtataagaagaaaaaactctccatatttatatcgtctgaatttttgcttgatagacacgtgtttggaactctgtccccccacgttttcactgtgtataacaaaaatatgtgtttctcaaaagatcttgaggtgtttgaaaacgggggaaacctgcgtttgggtgctctaagccccggactgggacgtagccggcgtccggcacctatatttttctatttttttttacaaaatatatgatgaaccaagaataaaactctagctctcgtctatttttaatatgctctacttagaacctttttaatgacagaatgaactccatgttatacgctctttatatagtttctctgcactaacctttaaaaccgtatccttccctgttgtacaaatcatcttttgatacacaatgatgacctgatatccctccatatatatgatcggatattattccgttagacttgtcctccttttttttcctcatctcctgtatctggagatatatgttgaccaccaccgccatgaccaccaaaaagctagccgtcacgactagaaatgtgtaggattcggactttccgttcgagaagaaaaagagaccgcgtctctggacgctctttttgtcagtctgaatcgacccgggatacgtaagagagcggccctacatcggggggcgctcgagaccgacgacgttccatctgaccagaaaaaaaaaggcacccctcggtggcgacctctcaccatcgtttgcccgtccgcccgtccttcgtagccatcatcatctcaggctctatcggtaccatcgttgtcatctgaaaaaaaaactgcctcacccacctgcgtaaaaacaccatctttccggaggtgcggtaagacgggcaaatacggtcgtgccgaggcaaaaaaaacgcaccatcgacaccacaccctcatgagcaccacctgtcggtgttggtcgtcctccatcgttctctacgaacatctcgacgcccgggtgacggacgacggcaagacgtcccggagaagacggtgttctctcgggcggtacgctctctggatctataatatctatagtagctaaacgagactgtgagtacgacgaaccacatcatcttttttttatgttgcttctttagaaaatgacttatgtcgacgacactcggcatcagccatctcgtgaaacacgctcgcttttcgtctctccaaggaacactgggtccgctgaaagggaccgtgtaccgaccaaagcaaaaaacacacacgtagtaacatgatcaaccacgtctgaatgacacgaaaacacaatcgtataacgctctattcatggaacgaacttggaataaaaaaaccatcgcaggccagaggctaagccgaaaccgtccggggaagcgggcgcgagttttccgacttagcctttggtgctcgttgagcctcttttttttttctgattctctgaagaatcaccgtcacagccctatgacgcgaaatcaattgctagaacataaacgttctcaacaggtatgaaatgaacaaactagatgatgctataaccttatattgtgtgtatatagataggtgtgaaatttgtaggataaaaagtgtcgttgtatgatgcacaacgatcgtgaaactggagactgtagctctctaccgaatgcaaatacacaaatgacatcgattcccgtccccacataaagaaatgtgctttactgtgaaagaatgaagaagattcttgttcctcgtacgacggggccctcgctcgtcgtgcctcttcccccctccgggagaggggacgtcggggccctccgtcgcaccgggccgaagccagtgaaatgtttactacactgtcatcagaatatatgatgtatattatttcctccaaactcctcaccatagccaccaattcgcatcacttaagaaagtagtagcaaccgcggcggcggcgaccggccggtcgtcgtctcctcgtcctcaaatgttgtacatgtgcagaaaaatgtgtaaatacgtgttatttatcccatgcgtcttgtacatagatatatgtttttatatacgctatttatactttatatatccttttgcataaccatagacagtcaaggattttaatgatttgctcatccgcctttgagccatcgcttaggagttagttcctctatgttctcggcccaccttttcgactacagtagcaaacccttgtactaccaccccgataaaaaccacatcatcatcgtcaccacgacctggaaacgacacacgttcccccccaatcttgggcatgtgtatatataaaaagaatgggagggagaggacgtggggctcgagaagaaataaacgccaagctcgattcgaaccaaaaaaccacatgtgtattgtgctttgtttttttttttacggtgggggaaaaggagggggccgtcattaacggaaaccgtgtatggggtccggacacgaacagtacacagcttatggggaaaaaagctcacagagagaaaaaacaccaagctcaggcacgcgtacatcattattatcatcatcggatatctcaccacgggtcatagtagtaccaaggagtgtgtaacaccattttttcttttctttgtaacgggataagggacagcaatcatcacgcacaacacccttcactctctttttagtcatccatatcatcgctgtaacacagcatgtcctcgtaatcgggcgtctggcagcgcattaccaccgagtcgtcttcttgcggtaccggtggtggtggtggtggcggcggcggctgctgctgctgggttgccgtcgtactgtgattaccgttggcggactgcaccgggatgatgggctgcttgtggggaacctggggtggactgccgccgtgagaaggcgacggcgtcatcaagttaagctcaccacggtgactccggacaccggcgaggggcgccgggggactgggagggaccgcggtcgtcttgtagacgacggtgtccccgtgtcgatccgtggctcgtaccagatcttgactgctagcgtcgtcactgtcttcgtcctcttccagctcgccctcagagtagtgctgctgtggttgcgacggtggctgggcgggaggagcggcggcgatcattggagagggatgtcgatgactcccttctctgtcctttttatcgtaggctgtcagcgttgctgggtccgtcctgctttccatatttgcgtattgctcatcggtgggatgaatttggtctcctccccgctgttgtccgccggcagtggcgtggttgctggcggttgtcgttgtcgtaccggcaaagacggtgagatccaatagcgactgctcgtcgaagggacagtacgctatcatgaaacgatagggtgccaacgcgcgttggatgcgcagttcgcacatctcgttctgacactcgtggcactgcagggcgcctaggatcaggtccgagacagcgccgcagcggtaggtacccatggcgttgttagtatcgaactggtcaaaaaattggggcgtaccggtgacttgcaacgcgcgacggcgtagcgagacggccacgcgcgagaaagagcacacataggccatggcgcggtgcatgggttgcgagaaggtctcgggcggacgcttctgcagatcgcagacgtcgtcgcgtagccaggcgctcatttgaccgggcttcttgactagccgtttgagcgtgctgcaatggtcgccccagccgtcctggtggtccaggatgcagcccaggtccaggttgttgagtttgttgaagagtagctgacgcatgccgcccaccgtctccagatagggatcgtgcgggttgacgggtagcccgtgcaggtggtggtacttcatgtagctgagcgtttcgtcgatgatggccagcaacgtgtgcaagttgggagcgttgtacacggcgaagatcttttccaccaccagcttgcgcagcaacggttcctccagccaatcgaactgttgacgaatgtgcaacaggtagtcggtgtgcatgagctcgtcgtgtgacagcaggatgcgaccgcgcggctgatgatcttgcgggaaggcggtggggaccttgagatcggcggggtagggtgccagacgtagactctcggccgtgtagcgctgaaggtcgtaaacgggcgaggtagaactcggtgaggtacccgacgaggcggcgccgcgctgcagacgcgctctttttttcttttcgatcaaacggctgagttgctgtagttcgtcctcgtccatggcgtccagttcgtcgtcaataagcgccagcatctgttgttgttgcggtccggcggacgatccgtgatgattattggctgaggaggggtgagaagaaccgaaagtcgtaggacaactgggaactcggcgacgaagatgcgtcgaatcgccgccgtgatggtgcggttcgccgtcatcgttgtcgtaagacttaccgtagtgggggttaaggggcaccgaggcggacgcggccacgcgtcgcttgaaagaggaggacgccctatgtccgccacggaagcccgcggtgcccatgatgatgtgtccgccggtgcccccgagtgcgtggcgggaggagggtggaaggggaggaggatagtggtccggatcgccttcggtatcatcgtctttgctgtagcggggtcgtcgtgcggggacgcagggtcggtgatgatgcgaggcggcgccgacggtatcttccgcgagatggtgttcgctggcggctgctccgttccgtgtcgacggcgaggttggacttcgctcgcgtcggaacttccgtggcacgggttcgtaatccagacagaagcgccgtgcgcgacgggcgcggcgttcgcgctcgctcagggaagataacgacggagcgtcgtgacggccgcgtgagtgcagctccatggccgccgtcgctaggaaggtcacgttcgggcacgctgatgtatatatagatgagaccgctgccggggggcgggtcaccggcgccgtggaaagtgaggctcagacggcggtcgccggcggcacgggcgcgtcgggcggtctgattttgatggaaatgtggacgtttttggcgttggagtgacactttttggtgaaacagcggctccagaggctggcccagagcgcgtagctgtgctcggtgcgcaggtcgatgaacacctgcacggtctcttgcgggttgcggtgcgtgtagttgagacagcgaaaatcccgcgtgcgcgcgccgtcgcgccgcttgacggccacgcagcaggcgccgtggggctgaaagaggaggacgtggggcgcggtaaactgctcgctgacgtgcggttcgtagtgttgcgtgaggtgctcgagcagcggcggccacacgcgggtgacgacgagccgctgcaagtccgtgtcggaaatcgcagcggcagtggcgccgtcgccaccgtacaggtgataggcgagcacctcggtgagaccgcggcgtcgataacgcgtcacgttaagcgagcgcgtctcgataaagttggcttcggtcgaggggcagattttgtcgcgtacgctgagaatgacgcgtggcggcggcgacaggggcaacgcgggcaggtcgtgcggcgggtggtggtgaagcaggttacgcagatccagttgggcgcgcacaaagcctagcgggtgttcgcggtaggcgtcgggcacgatgaacagcggcaacagacggcgatgcatgaaatagccgtcgtcttggtccattttatacatgtagggcagacgtacagagcgtccatggtggtagatgcctgtgtctaggctgctctcgggatgcgagatggggtccagcagcgtgtgcagttcggcgtcgagacagacggcgtgattgagcacctgcgccacggcgcgtaaaacgctggggtgtacggcgacggtgcaggcggggaacggcgtgatgatgcgcagccccagtttgcccttgcagcggcagtaagggggtgacgtgtcaacggaggacgttgttttttggaaaacgccgttatccgggacgttatttttatcctctttcccgtcttcgtcttcctctgtgtcgcgctcgtcccggtaatcgagatagtcgtcgtcatcgaaaggcgcgccggccgcgtccacgggcacgctgttgggtgggcacgcgcttttgaagaaatagaccgggtgccggtcggggtgcgtgtagccaaagaggctcgcccatacggtcatccagacgcgtcgtagtccgcgacatagctcaaagacggtgtgtcgcgccagaccggagacgccgtcgcgcagccgtaaatcaaagtcggccacaaaattgaagacgggcagacgttcgttgaagacttcgtgtcgcgtgtagtagaactgtgtctcggggctggtgctggccacgtcgtcgtcgtgtagccacacggtctcggtcagggcctcgtccgagaaacggctgtcgggtacgtgacggagcaggtcacgcggaaagaggctgcgatgccaggtttcggaggccacggcgcagaagacgtgctggtcattgggcaggtgtacgcggtagacgggcagcggtcgctccagcagcggtgccagcgcgggctcgggtagcaggtagcgacgttgcgagtaacgcgttagcgtgccggtggtgtaagtctgggctgtgcgtagcgaggcgcatagacgtaacaagccggacagggagcgttccagcggggagaagacagactcggaaagcgtgttgatgcgttcgagctggcgcgccagctgcgtggaggtgccgaagaagcccgccaggtgcgtgccgtcgatgcggccgccgtagccggccagccccaagccgtgcgggctggtcgccgagtggggggattcgtcgagacgcagtaggtgcgtctccacgtagtcgtgtagaaagttgtcgagcgagaagtatttttgcatgacgtccagcagctcggtggaaagccggcggcccagaaaacccggttcgcgcgtgcactgcgcttcgggcgccgcgtcagcgtcgtaagccaccacgcgccggtactcgagcaaccgcgcgcgtgccagcgccgtgcggtaggccaggtagacgtagtgcacgcagaccgtgtcgggcagacgcgcacgttcgcggaacgcgttgatctgcgtgtccacctgctctagctcggtgtagtcgcggcggttgcgcgcgacggcgtacgccacgaaagcggacacgcgctgacggaagggcgagcccagtagcagacgcgcgaactcgcccatggaggcgtgcgtggggatgatggtgcccaggtcgcgcgtgcagaagctgcgcacgtactcctccacggtggagatggtgctgtactggccctcgaataggtagtaggccatggtcagcagcacctggccctcggtgtgcccgaagacgctgatgaaccacgagggcgaggtggggcagaggaagacctggttgagatgacgtagcacggccgcgtggtgaaagtacaccaggtgcttgaattcgcgcacctcgccgccgtgttcgggcgagagcacgggcgtgcggaaaagatgccggtagagcggttgcgtctcggcctcgtccagactggcgatgagcgccgagagggggatgggctggcgcgcggccaggtagcgcgagagctgcagcgtttcgttgttcacggcgaagacgggcgccacccgccgcgagtccgagcacttttgcgtctgtaggcagaagtaaacacgtcgcgagacctggtgtttgaccagcagggggaagacgcagtggtccgtcggtgtctgcgagagtacgttggcgactatatgagcagaatcatactctgttgcgaacagaacgagcgtcatcgtcgcgccggcacgatgcagctggcccagcgcctgtgcgagctgctgatgtgccgtcgcaaagccgcgcctgtggccgattacgtgctgctgcagcctagcgaggacgtggagctgcgcgagctgcaggcgtttctggacgagaactttaagcagctggagatcaccccggccgacctgcgaaccttttctcgcgacacggacgtggtgaaccacctgctgaagctgctgccgctctataggcaatgccagagcaagtgcgcgttcctcaagggctatctctcggagggctgtttgcctcacacgcggccggcggccgaggtggagtgcaagaaatcgcagcgtatcctagaggccctggacattctcatcctcaaactggtggtgggcgagtttgccatgtccgaggccgacagcctggagatgttgctggacaagttctccacggatcaggcctcgctggtggaggtgcagcgcgttatgggcctggtggacatggactgcgagaaaagcgcgtacatgctcgaggccggcgcggctgcgacggttgcgccactgacgccaccggcggtcgttcagggggaaagcggcgtccgcgaggacggggaaacggttgccgccgtgtcggcctttgcctgtccctcggtttcggactcgctgatccccgaggaaacgggggtcacgcgtcctatgatgagtttggctcacattaacaccgtctcctgtcctaccgttatgaggttcgaccagcggctgctggaagagggcgacgaggaggatgaagtgaccgtgatgtcgccgtcacccgagcccgtgcaacagcagccgccggtcgagcccgtgcagcagcagccccagggacgcgggtctcaccgtcggcgctacaaggagtcggcgccgcaagagacgctgcctacgaatcacgaacgcgagattttggatctcatgcgacacagccccgacgtgcctcgggaggcggtgatgtcaccgaccatggtcaccatacctcctccccagataccctttgtgggttccgcgcgtgaactcaggggcgtgaagaaaaagaaacccacggcggcggccttgctgtcctccgcgtgaacagcctggcacgttttggaaaacgtacgtgatcacggacacgacgagtacggggtttctcatagacgtactttattaggtcagggatgacggggaggtttcgggccgacgtcaaaaataacgtcattcgtgttgacagggctttctgcgtcggagctcttttcatcttcttctgtctcgtcgacgtcatcgtctaccggcgagggtgtccgttgcagcaacgcgtgctcgggcgtgtgggtgaaaccgatgtcgggggtgggcggcacgatcatctgtcctagggggtgactgcccaccggcagataggtaaagcggtgggtggtaaaaaccgctttggctacggtggtgtgtggggagatgcagacggtggtgtgcgaagtgttgaccaccgtcacgccggccgcggtacccgggagccagatggtgggtcggatgatgagatccgattgactaaactggcgcacgcccactatgagggcgcagataccgggcgcgtgcacgtaggccgcgtcaaaatagacggtttgcgtgtgacccggaccgatcaccagcgtctgacgggtacgtaacgaaaagaaacggtgttcgttgggcggcggcaagttcatgagctgccagggttctggtacaaaacaggggaaaacgccgatatcgccttcgatggtgcccggaaagatggactgaaaagtgtcgttgaggttgacgacatccaactgcgggacttgcagcctggattccagcagctcgggcatgcaaacgaattgcgcgtccaggcatttgtaaaaggtaatgccgaaaaaaccttcggggatatagaggctgacgcccagcgaggtgggcactttgcgctcgcgtgatagccaaatgatgtgtttattgtaaaaggccagctgcgtgtggcattgtttgacgatgaaactggaaggcatccacttgtaaggaactttgagcggtgacggtaatggcgacgacgcttcatcctctcccggatgctgctctttgtcgtatttctcctcggtcgattggggcagcgtaaatgtggtttgaaaatcgctatcgctagcgaaacgcacgcagtaacgcatgttgacggatttctcggctaggatgatggagcctgatgacgatgcggactcttccttcattattaacgtaggggtctcccagaatcgctgaaaacgggagcgcggcagccgcgacagtaccagttgagagtcgattcggtcggtcaacatcgtaagcatcgtggcggtggtgtgatggagtggaacacactagtattaggtcttttagttttatcggtagtggcagagagttctggtaacaattcatccacgtcaacctctgcaactacatcaaagtcttctgctagcgtatcaactaccaaactaacaacagttgcaacaacttctgcaacaactacgacgactacgaccttatcgacaactagcactaaactcagttctaccacccacgatcctaatgtgatgagacgacatgcgaacgatgatttttacaaggcgcattgcacatcgcatatgtatgagctctcactgtccagctttgcggcctggtggactatgcttaatgctctaattctcatgggagctttttgtattgtactacgacattgctgcttccagaactttactgcaaccaccaccaaaggctattgagggtggacagatttacagcccggcggtgttccggcggggtaaggtttacatacgtgggtgaccggaggctaaagttacgaatctcatctagaaacagcagcgagtctagatagtcccacaggggatctataaatgttctctgaaaccccattgatggtgacgtaggtgtagttttgttactatcggaagctgttttgttttccacgaacatggtttcgttgtaatataaggagctcatgtcgagagtaccgtaaatagtgtacggcgtttcgttacggattagtacgtgcgtgtttttcataaattctgacacggcggttcggttgcggcttggttcacaaaaaggattttgccggtaacgtagagtggtatacacccacgttgctaggtcccttaactgtgtggccataatggacttcataaagctgctatcaggacgataagcaattgtagacgtggaaacccgccttgcggcggtagtaatactataagtcacgttagtagtgacgttgagagcggcagacgttgtataggaaaagtatggcgtagtagtactctgagttttcttagcttttttttcgaattgttccttaacgggcgcttgtttacgttttagttttcgcatagtgttttttaacttggtgccgttaatatacttggggacgcgaaatagattccggctcatggcgttaaccaggtagaaactgtgtgtacagttgcgttgtgcgtaacgtaaaagcagggcggttaaacctagaaaataaatcgtttgactatctacgttaaccttagtcggacccacgtacaatttggtgttccaacgcggtacattgaaaaacatggggttgaacgtggtgaaattaccgcaaccttgttcgccagtatcattacgtttggaaacgtttagcatttcggaaagacaagtcatggaaggcacagtaccacaaggtgggggtctgaatgttatcgttttagccgtatgattgtactgtgagtaaacgtattttgcgggttttctaagctgggtactataaaaatcaaaccacagataggttatactataattctgaatggggcccgctaaaatgtagtattgtggaaactctgtcatgttcatagtgagatttttaaccggttgtttacttacattgtattttgtagaaatagtcgtttctagttgtctcaaaatttctaacttaagctgatctaatttatatttgcctatcttagacagtaccaagcccctccaaggacgattataaagcgcttttgacataactttacagtttatgaaagaaacaagcaagaaagatatagatattagaaacaccatcttagggacgtctctcaccatcatctcttttctccccatgacagaggaggagaccccgcaccgtccgtctgccttgtggtttggcttgcctgcgtgtactcactgctgattctggtcgttttgctgctcatctaccgttgttgcatcggcttccaagacgacctagtctcccgcaccttggctgtgtaccaagcttgtatccagggcccgatatgtaaccagacccataacagtacctcgtaaataaagacgcacagacctcacgcatatagtaccatcacaccgtgtggcgtgtactttattacaacgagcaagagtgcccctaagtattggggcccgtaccgttttagaagattttgtgtgaatgtctttaacttttctgtcccttttctcataaactgtcaggttctacagtcagcatgtcttgagcatgcggtagagcagatagatgccgatgatggccgatagcgcgtagacggacatcatgaggagacgactgtcggtggcgtccacgacgacgtcagttacttctaggaccgtaccgtttttcaaaagcatgaggtagtgagttcgcggagatgagaccaccacttcgttgtagggatccagggcgaaaaggacgtcgtccgagtcgtgcatgtacatgatgttgatgacgccttgcgtgtcgtcgtattctagcagggcgctttggcaaaaggcgcagttttctagtgaaatgttgagcgccgctgtgatgctgtgtgtggtgtgcatgttgcgcgttagttcgcatttagtttgactgtccgtttgggtgatgatgaggctctggcctacgacggtggtggagacagggtaggagatacctttgatcaggtactggtttgttacgacataactgacgtgttcggagacggttagcgcggagaaggattcgccgagcggcagacaaaacaggtcggggaaggtttccagcgtgcttggttgcatggtagataggatggagagggcggcgggaacggtagcaggaacggtggcatcggggaagagacgcgtgaggcgttcgagcgagtgatcgcgtcgcccgctactggaacagggtgtgtacaggtcgctgaggtattcgtggtgcggatgagctagcaactgcgtaaagtgtgatagctcggccaatgaacagaggcccgtttctacgatgaagatttcgcgtctctccgtcgtatgtaccaacatggagtggacgaggctgcccatgaggtagagttcttggcgcgcgaaggctgaaagaaaagaggccaggtgcgttttgtgtaattgtagggcaaagtcggcgatctgtcgtagtgcccactggggaatgagatgttgctgattctgtttagaaagtatgtagaccaggcgtacgaggctggtgatgtcggtgatctggtccggcgtccagagggctcgtttggccaggtccacggctgtgggatatagcagcaatgtggtgcgtggtggtgtttgtgagaggcaggtgatcataaattcttgtatttgtaagagtgcggcctggcggtctagggctcgtgggatggagatttcggtgccggcctcttcttgtcgggctgccgcgaacagtgctaatgcgtaggcgaaggccatttctaccgtgcggcggtccaacatttgacatcgaccgcttttgagtacgtctacagcgtaacggtgaaagctgttacgtaacagtgcgctgaggtccaggtagttgaagtcgagtgcggcgtcgagaaagtccgagtctttgagataggagtgacggtttagttgagctttcttaactagtaccaggagctcgtgtttttcagtttgtcgtagtataaagttgtcgcgttgatagggcgctttgaagagtacgcgtggaagatgaccgaagataagcagcatgggtgtgtcgtcgtctatagataccgtaactacgaagaagtcctcggtcagtgtgattttaacgtaacgtagttcgtccatgaggtaaaagccctggtgcagacagggcgtaacggtgctgaaaagcagatcgtgtccatcaaagaggatacaggtctggttaaagtgtggccgatgtagtcccgaggtggtgtgcgatcccttccagtcgtgtggagtggtttggggtggcatccaaacgtgaggtattgacagatcaatgggcggtggcacggtggtgggctgctgacccaggctgtcttgtgccttcagctgctgcgaaaaagatcggtagctggccaggtctttggataccaatgcgtaggtgttaagtctctgttggtatctttctagggtttcggtcagatctacctggttcagaaactgctccgccagaggacccgcaaaaagacatcgaggcatatggaatacatagtattgattatagctttggaaaaagttgaaactgatggcgttttccctgacgaccgtgctgttacggaggctgctgttgtaggtgcactgggtggtgttttcacgcaggaagcggatgggtctcccgtaggtgttgagtagtaggtgaaatgcgtgagggtccagcgcttcggatgcggcgtccgcgccatatcgttgcgaaggtaggtgactgaggaggtagacggtgaagacagtgaggtagggggggaggccgggccgcatagcgcggctgcgccgctgggttcagcggcgtgatccaggtggtggttggcgttacacccgagagaaggagagaaaggatcccaggaaggggcacccgggtgtggcgctacgggttacaaaagtcgcgtctctgtctatttaatacgatgtcattggccgctgcgaaggaagaagaggggacacgcgggtaagccatgccgtccgggcgtggggacgacgctgattcgacggggaacgctctgcggagattgcctcacgtgcgtaagcggatcggtaagcgtaagcacctggacatctaccgtcgcctgttgcgggtctttccctcgtttgtggccctcaaccgcctgttgggaggccttttcccacccgagctgcaaaagtaccgtcgccgtcttttcatcgaagtacgattaagtcggcggattcccgactgcgtgttggtgtttttaccgccggactctgggtcgcgcggcatcgtgtattgctacgtgattgagttcaaaactacgtactcagacgccgacgatcagtccgtgcggtggcacgccacccacagcctgcagtacgccgagggcctgcgccagctcaagggcgccttggtggactttgattttctgcgtctgccgcgcggtggcggtcaagtctggagcgtagtgcccagtctggttttttttcagcaaaaggccgatcgcccatctttttaccgggcttttcgttcgggccgtttcgacttgtgtaccgattctgtcctggactatctgggacggcgtcaggatgagtctgttgcacaccttttggcggctacccgtcgccgtcttcttcgaaccgcacgaggaaaacgtgctgcgctgccccgagcgcgtgcttcggcggttgctggaggacgcggcggtgacaatgcgcggcgggggctggcgcgaggacgtgctcatggaccgggtgcgcaaacggtatctgcgtcaggagctcagggatctgggtcacagggtgcagacttactgcgaggatctcgaagggcgcgtgtccgaggcggaggcgctgttgaaccagcagtgcgagctcgacgaaggaccgtcgccgcggacgctgctacaaccaccgtgtcgtccgcgttcttcgtccccagggaccggcgtggcaggagcttctgccgtcccacacggtctttatagtcggcacgatgccatcacgggacccgccgccgccccgtctgacgtggtcgccccgtctgacgcggtcgccgcgtcagcggccgccggtgcttcttctacctggctggcgcagtgcgccgagcggccgttgcccgggaacgtacctagctactttggaatcacgcagaacgatccctttatccgctttcacaccgattttcgcggcgaggtggtcaacaccatgttcgagaatgcctctacttggactttctcctttggtatctggtactatcggctcaagcgggggttgtacacgcaaccacggtggaaacgagtgtaccatctggcgcagatggacaacttttccatttcgcaggagctgctgctcggcgtggtcaacgctttggaaaacgtgacggtgtatccgacgtacgactgtgtactctccgatttggaagccgccgcctgtctgctggccgcctacggacatgcgctttgggagggccgcgatccgccggactccgtggcgacggtgttgggtgagctccctcagctgttgccgcgtctggccgacgacgtgagtcgtgagattgccgcttgggaaggccccgtcgccgcgggtaacaactattacgcgtatcgcgactcgcccgatctacgctactacatgcccctaagcggtggtcgtcactatcacccgggcacttttgatcgtcacgtgctggtgcggcttttccacaaacgcggcgttattcagcatttgccgggctacgggacgataacggaggagctggtgcaagagcgtctgtcgggccaggtgcgcgacgacgtgctttctctctggagtcgacgtctgctggtcggcaagctgggtcgcgacgtgcccgtctttgtgcacgaacagcaatatctgcgttcgggcctgacctgcctggctggcctgctgttgttgtggaaggtgaccaacgcggatagcgtcttcgctccgcgcacgggcaaatttacgttggccgacctgctgggttcggatgccgtagccggcggcgggttgcccggggggcgcgcgggcggcgaagaggagggctacgggggacggcacgggcgggtacgtaactttgagtttctggtacggtactacatcgggccgtggtacgcgcgcgaccccgcggtcacgctgtcgcagctctttcccggcctggctctgttggccgtgaccgagagcgtgcgcagcggctgggatccctcacgtcgcgaggacagcgccggaggtggcgacggcggcggcgccgtgctcatgcagctcagcaagagcaaccccgtggccgactacatgttcgcgcagagctccaaacagtacggcgatttacgtcgcttagaggtacacgatgccctgctctttcactacgaacacgggctagggcggctgttgtcagtgaccctgccgcgtcaccgtgtgtccactctgggctcgtccctctttaacgtcaacgatatttacgaactgttgtactttttagtgttggggtttcttccgagcgtggcggtgttgtaatttccaccacgtgtcgctcgctgcataaagggcgaacgtcctcggagagggtatattcgttcggcgagagcgggcggcggtggtgggtatgtccccttctgtggaggagactacctcagtcaccgagtccatcatgttcgctattgtgagtttcaaacacatgggcccgttcgaaggctactctatgtcggccgatcgcgccgcctcggatctactcatcggcatgttcggctccgttagcctggtcaacctgctgactatcatcggttgcctctgggtgttgcgtgttacgcggccgcccgtgtccgtgatgatttttacttggaatctggtacttagtcagtttttttccatcctggccaccatgttgtccaagggtatcatgctgcgtggcgctctaaatctcagcctctgtcgcttagtgctctttgtcgacgacgtgggcctatattcgacggcgttgtttttcctctttctgatactggatcgtctgtcggccatatcttacggccgtgatctctggcatcatgagacgcgcgaaaacgccggcgtggcgctctacgcggtcgcctttgcctgggttctttccatcgtagccgctgtgcccaccgccgctacgggttcactggactaccgttggctaggctgtcagatccctatacagtatgccgcggtggacctcaccatcaagatgtggtttttgctgggggcgcccatgatcgccgtactggctaacgtggtagagttggcctacagcgatcggcgcgaccacgtctggtcctacgtgggtcgtgtctgcaccttctacgtgacgtgtctcatgctgtttgtgccctactactgcttcagagtcctacgcggtgtactgcagcccgctagcgcggccggcaccggtttcggcattatggattacgtggaattggctacgcgtacccttctcaccatgcgtcttggcattctgccgctctttatcattgcgttcttctcccgcgagcccaccaaggatctggatgactcctttgattatctggtcgagagatgtcagcaaagctgccacggtcatttcgtacgtcggttggtgcaggcgttgaagcgggctatgtatagcgtggagctggccgtgtgttacttttctacgtccgtccgagacgtcgccgaggcggtgaaaaagtcctccagccgttgttacgccgacgcgacgtcggcggccgttgtggtaacgacaaccacgtcggagaaagccacgttggtggagcacgcggaaggcatggcttccgaaatgtgtcctgggactacgatcgatgtttcggccgaaagttcctccgtcctctgcaccgacggcgaaaacaccgtcgcgtcggacgcgacggtgacggcattatgagcggcggcgctgtacggcagcggggagaaaagtggcagataaatcacgtcaggttcacacgtcgttagccagcgtcggcatatgaagggcgcgggcggccagtacggcctctgggctgagacaggacgaggcagggtgagaaagaggaggatgggggggaccggggtggtggtgctgctgctgttgtgggtgcggacggtgcgggtgccgggacagcgtgccggcgaacgttctgtaatcttccataataaaagtaaaaatgcccgtctcgtgtcgactccgctggatctcgaaggcgtcgggggtaatgcgcatcttgccggtgccgatgagataaaagtaccacattttttgacagatgatgcgaatcaagggttcgtacgcttcggcaccccagtggcgcgtgaagaaggccgccagacgaaacaagcggtgtccgtagagcgtgcctagggagaagaggatgttgccgttgcgcgccaggtcttcggggaaaacgaccggcaggccggtgtggcgctgcacaaagcgcgtcagcagtccgccgctcaagcgcgggtgacacaggcgctggctgagacgggcggcgcgcgtttcatcgaacacggccgcctcaaagtccagccccgggaaggcctggcgcagttcgcggtacagatgaggccagtagggttgcggcgtcttgcgactaagcacggcgtggtccgagacacccaggttgttcatggtttcgcgcagtagcagcgtttcgagaccgcggtgaaagaggaggacgcagatgaggcgtacgatcttgagttcttccaaacgcagcgagctcagcggctgtccgcgcgacatcttctcgctaatctgtaatattagatgattggcgcaagtaaaggagaatttgcccgtgcggacccgcgggacggcggggttctcttcgtcgcgggccatcatcgttcgctcggtgagcgggtagcgacggtgacgacaatgacgatggacgagcagcagtcgcaggctgtggcgccggtctacgtgggcggctttctcgcccgctacgaccagtctccggacgaggccgaattgctgttgccgcgggacgtagtggagcactggttgcacgcgcagggccagggacagccttcgttgtcggtcgcgctcccgctcaacatcaaccacgacgacacggccgttgtaggacacgttgcggcgatgcagagcgtccgcgacggtcttttttgcctgggctgcgtcacttcgcccaggtttctggagattgtacgccgcgcttcggaaaagtccgagctggtttcgcgcgggcccgtcagtccgctgcagccagacaaggtggtggagtttctcagcggcagctacgccggcctctcgctctccagccggcgctgcgacgacgtggaggccgcgacgtcgctttcgggctcggaaaccacgccgttcaaacacgtggctttgtgcagcgtgggtcggcgtcgcggtacgttggccgtgtacgggcgcgatcccgagtgggtcacacagcggtttccagacctcacggcggccgaccgtgacgggctacgtgcacagtggcagcgctgcggcagcactgctgtcgacgcgtcgggcgatccctttcgctcagacagctacggcctgttgggcaacagcgtggacgcgctctacatccgtgagcgactgcccaagctgcgctacgacaagcaactagtcggcgtgacggagcgcgagtcatacgtcaaggcgagcgtttcgcctgaggcggcgtgcgatattaaagcggcgtccgccgagcgttcgggcgacagccgcagtcaggccgccacgccggcggctggggcgcgcgttccctcttcgtccccgtcgcctccagtcgaaccgccatctcctgtacagccgcctgcgcttccagcgtcgccgtccgttcttcccgcggaatcaccgccgtcgctttctccctcggagccggcagaggcggcgtccatgtcgcaccctctgagtgctgcggttcccgccgctacggctcctccaggtgctaccgtggcaggtgcgtcgccggctgtgtcgtctctagcgtggcctcacgacggagtttatttacccaaagacgcttttttctcgctacttggggccagtcgctcggcagtgcccgtcatgtatcccggcgccgtagcggcccctccttctgcttcgccagcaccgctgcctttgccgtcttatcccgcgtcctacggcgcccccgtcgtgggttacgaccagttggcggcacgtcactttgcggactacgtggatccccattatcccgggtggggtcggcgttacgagcccgcgccgtctttgcatccgtcttatcccgtgccgccgccaccatcaccggcctattaccgtcggcgcgactctccgggcggtatggatgaaccaccgtccggatgggagcgttacgacggtggtcaccgtggtcagtcgcagaagcagcaccgtcacgggggcagcggcggacacaacaaacgccgtaaggaaaccgcggcggcgtcgtcgtcgtcctcggacgaagacttgagtttcccaggcgaggccgagcacggccgggcacgaaagcgtctaaaaagtcacgtcaatagcgacggtggaagtggcgggcacgcgggttccaatcagcagcagcaacaacgttacgatgaactgcgggatgccattcacgagctgaaacgcgatctgtttgctgcgcggcagagttctacgttactttcggcggctcttccctctgcggcctcttcctccccaactactactaccgtgtgtactcccaccggcgagctgacgagtggcggaggagaaacacccacggcacttctatccggaggtgccaaggtagctgagcgcgctcaggccggcgtggtgaacgccagttgccgcctcgctaccgcgtcgggttctgaggcggcaacggccgggccctcgacggcaggttcttcttcctgcccggctagtgtcgtgttagccgccgctgctgcccaagccgccgcagcttcccagagcccgcccaaagacatggtagatctgaatcggcggatttttgtggctgcgctcaataagctcgagtaagagagacgctatatttagggcttccctctcttttttttctacaccgtgataccctaataaagcacaccgcggttattatcaacgtctctgtgtttttattatttagaaataaatacagggaatgggaaaaacacgcgggggaaaaacaaagaagtctctctctagatgcggggtcgactgcgtggggtgctggaagtggaagcggtgctgatgggtgagggtcgtggcgcgggcacggaccgcaacgtgctgctgatgtctgccgcggtacgcacgtcgccgtccatgtcgctgcgcagataagaggtaggtcgtagtgcggcgtgctgcacgctcaccgttaatggtaccaagtcgtcaaggctcgcaaagacgtgccacgaggggatgacgagcgtgagagccccgttgttaccgcttcgacgtctttgtccggtcaggatcagtgccggggacagtccggcttgggtgtccgagtcctcgtcgccgctggcttcctcgaagccggcaaacatggcttcggacaggggggtcggcgtcggtgtggaggagaggtcatcttcgtcgtcctcttcctcttcttcctcctcttcctcggtgggtggtaatccgggggactgcgggagaaactcggagacggcgccgcgcatgacgttgctccgtggaaagagaccggcgcgcagctgcacctggggacgcttgattttgtccggtttaccgggtgtgagagtccaaaacccacggcggaaaaagtggatgcggcctagcggctgtcggtgttccaaatgaacggcctgatcgccggtcagcgtgacgcggagggtgattcgcacacgatcgggtagcgggccggcttctatggagacgcccgggatgttttccgggaaaaagatggtgtcgtgagtctgattggtctcgaaagcattctggatctgcacgatgtactcgggatgtatgcgcgtcagcgtaaaacttttgggaatcaacagctggaagccgttgtccggcaagcgtcgtaggtgcgggtacggattgtgtcgcgccaccacctcggcgcgatgcgtgtaaaccgaaaagtgcagaaacacgctggtcggcgggtgcggtgagtcgtgatgcagaaacagcatgatccattggcctcgttcgtccgtctccgttttgtggatgtacgtgttagggtccgaacaggccagctgctccagggcgtctaccagcgtcagcgggatggcgccggcgcgaaaggcgaactggctgacaaagatctgccctgcctccaaactgctgtcggttctgcggcgccagttcggcgttacggtcagtcgcacggcccagtggtgagccgtgcggcggatgatggcgcgcgcttccattcgcggccgattttcttcgccgccgcgccgctggctctgaaagaggtgcagtccgctaacgggcacgcggtccagcggcagcgcaaaggccagtaccgagaccgtgttgttttctgagcctggcgtcaggcgtcgtgggccaaagttgttgaggtccaccagcagtcggtcctgttcgcccaccacgcagcggcccttgatgtttaagtcggtcaggtctacggtgtcgtgcggagatttgttctcctgaaaacagcagagaaccgagggccggctcacctctatgttggtacgcaggtccaggagtcgcagacgaccggcttccagcgagccgccttccacgttggtgatgagccgaagcacctggcagtgcaggcgaccaaagcttccgctggcggcttcggcctcgctgatcgcggccgcttccgacgagggtccctcaccgggcgaggacgatgcctgagacattgcgaaggcgggatggggggagggtcaggggatgcgcaaaggtgaacgggtcttcgtgggaggtcgggaagggttccggcaactgtcgcaaatatagcagcggtgacaggtgtggcggccaaaagttgcgtgtctgagtggacgtgggtttttatagagtcgtcctaagcgcgtgcgcggcgggtggctcaacctcggtgctttttgggcgtcgaggcgatgcatggcccgggcaaggcgtcttgccggtggcggcgacgtttgggttgcgcagcgggctgccatacgccttccaattcggcgaagatgcggtagatgtcgttggcgtcccagaagaattcctggtacttcagattctgaccctgaaccgtagccaccatgggcaccaggttgcgggccaggatgccggcctgccagggcggccaggtgaacacggccggattgtggatttcgttgtcggaatcctcgtcggtgtcctcttcgggcgcgacggtggactcggccttaaggcggccgcgtgtcataacgcccgacgtgcacgccgtcgccgaggatgctgatttgcgtttgcggcccgcggaagtggaggcgcccgccatggcgccgccgccggtgacgcggggcgtcttgcgctcggtggttacgagttcttcgtcggagtccgatccgctggtccagacgtcgtcgtcgccctgggcggcaccctcgtcgtgccggtcccaggtgtgtcggtactcaagcttgccctggatgcgatactggctggtgaaggtggggtgctcgctgtactgaggcccgcgctgcagcagcaagtcgatatcgaaaaagaagagcgcagccacgggatcgtactgacgcagttccacggtctcgcgtatggcttgtacctccaggaagatctgctgcccgttcatcaacaggttacctgagatgctcaggcccgggatgctcttgggacacagcagcccaaaatgctcgtgtgaggtaaaagccacatccagcatgatgtgcgagatcttgcccggtttgattatcatatttttgggacacaacaccgtaaagccgttgcgctcgtgggggcgcatgaagggttgcgggttgcgggtcatcgtcaggtcctcttccacgtcagagcccagcgtgacgtgcataaagagcttgccggagggcacgtcctcgcagaaggactccaggtacaccttgacgtactggtcacctatcacctgcatcttggttgcgcgcgtgttctccatggagcaaaccagctcgtgcgcgcacaccacgtgccgcagtgccacgtccttggtgggaaacacgaacgctgacgtgtagtagacgtcgggctctttccactggttctgctgacgcgtccaggccagtcccgagaccgtgagacgcgcctgccacatctgcttgcccgacgcgtgaatcacagcgtcagctacgggcaggtgtcggtgtttgcgctcggccgccgacgggtagtggtgcacgttgatgctggggatgttcagcatcttgagcggcagcgcgtacacatagatcgacatgggctcctggctggggcagatgcttcggcccgtggggttgtgcacgttgaccgacacgttctccacctcgctgcccgtaaagtacgtgtgctgcacctgcagctgattgtcgccgcggtggcatggcgtcgagtcgggcgtgtactgcgataccaagatcagcgagggctggctcacgcgtacgtggatacccgtctgcaggagtcgcgtctcgtgcggcagcaccggcgtatcgccgcgactaaacacggctttcagcacgtgccccgaaatgggacccagtacggatatcatttcgggacaacggcgaccgcgcgactccatgctgcctgcgcgtacgggtgtaggcgactgagcggcgcgccctctgcggccgccgccttacataggcaggcgaccaaacgcggaacccgaaataaaaacgttctacacagagacaaccgcggattattgagtgtctttttttattacaaaaaaaagaggcgaagccccaccgtcaccacaccccatcacacaccaccaccgatttttttttgttttaatcccgtatggcgcggacgcctagtgtccgtttcccattatcagggtcctctgtttagagatcgccgcagaccatggctaaagtgacaggactcgtcttctctgtcgtattttccgtaagcttacagtcttgcggttccgtctccggggacgccagtcgcatgggcagcaggtcctccagcgcgatggaagcgcccagcaccgagagctgctgttgcgacggcgaatgggatgtggaccgcgagtgtagcgtggatttgacttggtgcgtcattgctgacaggcaaccccgattcagcgtatgctttgacgagataaaatagaggcgccccaggagcgcgtcccgtgggaacgtggcgccgttctcgtcgctcaccagtacggttaattccaaccaggagcgcggtagccagaccgtaacgggcattttgagtccctgacggttgtgtggtacaaaaacacccagataaggcccgtaaaagcggcggtagatacgtaacgtgtgcgagttcttcagcgtcaattcgtaagggacgcgcacctccagtccctcgtccgccgcgccggagcgtggcggtacaaagtaaggcagtggcgcgtccgaaaagaagggtcgtcgcaccgtttcgcgtcgcagccgcaggcgaaacgccactgggtcggctggcgcctcggtgcggtcgcaggtcacgttgaaacgtaatatgccgtcttggtatagcgtgagtgacgacagcgtcaggtccggcggtgattcgttcgggtctagctccaatcgtccaaagacggagggtcccaatgtcttggccgtggtttccgagaggcgcgccgagatacggctggtgagtccacgcggccccgagatgccgccttccactcgatgccagcacagcgcgtgtcgtacgcgcaccgtcagcgtgggcgtcagatccgcgtccgttgattccgcggtatcagcgacggaagccgcgttctccgttacgttgtttatatccagcgtcggctcgaacgtgagttctggcagatgcagcgccagacagtcgtgtaacgccgtgtgatgcgcggctttacgtcgtagcggtagccgtttcaacagcggcgtgatgatacggagcgcgaagagattgagtgataggcgcacgatggccatgcgcgtcagttgttggtcaattaccgagcgcaggatatggcagcctgggcgtgcgggaaagagagagaaggccgggcgcacgtcagaatcctcgttagagaccacgcatagaatgccgcgttcacgatcgtcgttgcggtcatcctcgtcctcttctttcttctcttgtttttccttttttttctcgggctcgtgggaagccgccgtttcttcttcttgcaacgtcgcgggggcggtttgagactcgtcgttcgcttcccccaattgcagcggcgtagagagcagaatctggaagggatcccgcaattcttcgggtcggaggtcgaggtgcaactggatcagatggtaggtgccgcggtgcacccgaggctgacggatgtcgtgtttatccgtcagtgtgaggatggtctgcggcgagccgctgtacttgtccagctcgtccggcgttttcaggaggagactgtcgtcgtcggtactggcgacgcccatcatggtcgtggtggtagtggtggcgaggaaagtgagcggcggcgccgacagagctcggcgttggcggcggcattttccgctgtgtcggctgctattgctgccaacgccaccgccgccgcctcgtctggctcgtggccggcgggcccgattccgaaggttggggtcgacgcgtggcatgcttggtgtctgcgggcgcgagagggccggctcagcctttaaatatgcaggtcgcggatttgttatcgggtgaaacgtcacacaccgtgaagacgacctgttcgcggatgaggtcatccagctgtcgcagcatgacgaaaagcgccgacagccgcgcgatctcgtcgtcgggcgacacgtgctgcggccgcgcgggcgtgcgcggctcgccgacgctgcgctcgcggtccagccgcatcagcagctcctggcacttgacgagcagcatggagctgtcctctagcgccaacttgcgcacgtaggtcatggtcagctccgaggctaggttggccaccatggacatggagaggcaggcggtcttcatgtcgatcagcaggtgctggtcgatgaccggatcggggatggtgaaggtggcgtcgcgaaaagtaatggtctgcagctgctgcacggcagcctttacctcctcgtacgaacggtcgagcgagaagaggcccatgatgagtagtcgctggttgatttccagcgccagtggcatgggtacgatccagggcagcaccagctcccactggcccagcgtcagcaggttctcgcgcgccagcggtccgtggaagagcggcggcagcacgcatagcgcgtcgcccttctcccaagtcacgggtcccgtgttgaggacggtgtagagcagtccgtgcgtgggtacgtgtaggaggatctggttgccttctacgcgccgcatcaacgtcagcgtcatattgcgcagcaggccgcgcagtcgtacgtagccgcgggtgtgatctacgaactggtgtaggcccagctggtagtgcttgatgagatgtagacgttgcggaatgggcacaacggccgctactagcttggtcagtttgcctacgtcggcgatgctgagcttgtggtcgaaagtgcagaagatgttggcctccatggccgccatagcggcggtgaaatcctggccgcgacggaggagaggcagagacgaacaacgtctgcaccgggcgcggcgtcagagcgagcgtggcgcgtccgggcccgcgtttgcgtctaggtgactcgccgctaacctgcggtcgtcgccgtcctcctcaccggacggcctcacgagttaaataacatggattgctgcagcgggatgatttcgcctacgacgtagttaccaaagtgcgtttcggacgtagcaaaagccccggcgccacccttgagtttggtctccatcagcgccagcgtggtggtgctgaggatcggtagcgcttcctgcgtcagacggcacgggttttcgatgagttgttccgtgccttcgacgcagacgtactgcgtgtccgtgtcgccgcggatgcagtccttggcgcgtagcaggtactcgtcgatggttttgaagagcgttttgttggccgcgataatctcttctgtgttaaagtactgcgcgcaagggctgtagaatttggagttgtagcctagacgttcgcgatgtcgggtgttgtagagtacgtcgctcagacagccggcttgcgaggcccaggggttgtgtgtggccgcgaaagtctgtgcgtccgcttcgcgatggtcgtagatggccttggtggcggcctccgtgtcgtacggatcgacggccagcatgcaggaggcacgcccgcgcgggttgttggggatcttaaagtaattaacgtccatcgtcaccggcgtaaggattagttcgcacgcggccttttgtccgtgcaccgtggcggcggcattgcgctcggacatgctgccgaacgtcagcatagagatggtctccgtgtctaacagttgcggccgttctacgccggccgcgtgccggatccagcggtccacctcgtcgtgccggtacacgttcatagggaagacgcgaaagaggtcctgcacgcggacgcccatgtcggttcgcacgcggtttacgtaggctacgcaggtatttgacgtgtaacccagacccatgtctacggtgttaatgttctgcgtgacgtggtacgtagtgctgatgtcgcgttcctccttggtcacgatagggttgttgatgataactgacgtgcatgatttgccgctgtagagcagcatgtccacctcgaaggtgtcggtgcgtacggccgtgagtgcgaatcccgggtggatgtgcgccttggtctgcagcaccagtgaaactggtgagattttgtataacatggcggccagcgtcatgactgagtgcaacacgttgggacaggtggccgagtaacgcgaaaagggcgagcgcagccagttgtggtactcgtgcgcgaaggctgtgggtagcgggaaaccaccgtcgtgacggtgatagtgcgggaactcggtcacgtagcgtttaatgtcgtcgctcaacgccgcgcagatggtggggtttgagtagaaacggtggaaaggtacgggtaggctgtactcgatcaacgtcttaggcgccgtcacgacgcagcagccgttgtaaagcacgtgctgacgtgagataaagtccggcaggccctgacgctgcgcgtggtccagaggcgcgcgcacttcgagcaccttgacgtgctcgcccacgaattgcacggccaaaaacagttcacgacaggcctgcagcagcggcgtatgtgcgtcggtggcgacgtcctccaccagctcggtcagcatctcgcctacggcttgacgttgcgccgctatcgagtcttcgggggtgacaccgcttgtgctctctttcgacgtcgtacctgacgtggagaccgcggtggcggccggcatcaggagaaacgccggtcggtaaaagaggtctactagcagcgtcttgaggttgagtcccaggccgcaggcccggttgttggtcatggcgggcatgaggcagagataaaagaccttttgtaacgtccattcgtcgtcggtggcacggtaatcgtccacaaacagcggctcgtcggcatccatggcgcccaaacgcggtacgtccgaaacgccgtggtgtcgcgcctcgatgttggccgggttcaacggttgccggtcggccactacctgtacgccttccatgttacgcggcaggtgcgtaacgaaggggggccacagccggtggtcgtgcagcgcgttcacgtaagccgatagcggttcctcagccagttgaccgttgttaagtcccggcagcgctgagatgcgcgttaccagacgcagcacggcgaccagattgcggtagtgaaagagcaactgcggtggtagggcgccatcagccaggtgttcggcgatcaacgtcaccagcgcgtagctgtgcgcaaaaaccagcagctgacgtgtgtgaaacatgttgacgatacaacgtgctacgaaagtgcggattagcaaaaaagcgtcgacgttgccgtgtaccagcacgtcgaccaggtagcaaagctcggggtaattggggcttgtcacggtggttttgaaaagtcgcaacgtctcttcgtagtcgggtggtggccgcagtcgcatgtgttccatgatctcccaggtgcgcagttcgtggaaggggcccggtgccagtccatctggcaaattaccgatgacgatacgcggtgtacacagcgccaccgtttcgctgttttcctggcagtgcgtaaagtcgaagaaggggtgcagctcggtgtagagcgtgatgttgcccaccttgtagaagtcggtgaccacaaagtcctgcttcatttcgttcaccgtgcgcgggacctcgcgtcgtacgcggtaaaaatgcggtatgcggcgcgccgcaccgcccatgggttcctgctgaaaacgacactcgagcagtcgttgcatggcgggttccgagggcggtccgcgttccgtgaaggtctgtagacagggcgcgggctcgtgcagcaccgggtggcacagcgtcttgagcgcgtccacaaagtctattttttgtacggcacggtcccggtttagcaggtaggccgtggtgggcaacgcgttgcgaacggtgtcgttaagcttaactttgctttccaccgtggtgtaaccgcgatcctcgggcagatacagccctacggggaagaaaaacgtcaggtccacgttacgttctagcggatctttggtatcggtgtttttgtagacgcgccgcaagttttccataatcaccgttttttcgcccagtcggatcacgtccatgctcagcggcgttaagctgtgcgccccggcctgcgaaagcgagtcgttgggcaaatgcggttggcccgaagtcagatgagccttgtacgagttgaaatcggccaggatcgagtgataggatatggcagtgacggcattttcgggactgagtacaaaattgccgtaggtggccggcgccgagaccgtttctttggtgatgtggcttgagagcagcgacatgatgatctgcataacgttggccgtgcttaccatcacgccgctgatcttggcccccgagctcgtggtgtacgtggtggggttgtctaggatgctatcggtggccgcttcggccagacgcgtgaggaacttgagcacatagtcgcgatcgcgcgtgcgattcagcaaaaagagcgtggccagcattttggccttgaagctctgcaagatgttgcttcgctggatgcggttcagtgcctgtcgcgccagtgtggcgttttctaccagcgtctgcaccacaaagtacggcggcgccttgcgtagcagtgtctgtaaaaagctgtgaatcaagccgcgctccatggcgtcggccgtgtttttaagcgcgcgcagcaccgtgtgcatggcttccacgttgaggatcttgtccaagatggtgccctcgaatgtctcgcgcagatacgtgaggcaggctgcgctgagctcgaaggggatggtgatgggggatttttcactgtatttggtgaccataatggtggtctgacgactagtgggcaaaccggcgccgctggccacacgcggcacctgcacgtggaacagcattttgcccgtagtcagtttattgaggtcgtggaacttgatggcgtgcgccgccgcggccaagccgctggtcaaaaaataaacccattccaggcgattgcagaaggtgccgaagatggcttcgaagtgaatattgtaacgctcggggtcatcgccgtagtagatgcgtaaggcctcaaacatctcctcgccggcgctggtcttgacgtgcgtcagaaagtcagtgggaatgcctactttaggcaggagctcgagcgccgaccagttctccatcgcggcggcggcgtgagcgcgaggcgtcggagctcggggaaagcagcgcgacccggagaatggccggcgctgcgccgcgccgcctcggctgtgacgctctaatagtcgttggcggctccgctatgccgcgccgggttttacacgtccccgtgcacgttcgcgcctgcaacctcacccaagagctatcgacgggcgaggacgcccgcttttgtcgtccgcgacccgttaacgtcgaacgggtgcgcgctgtttttgcggctctctaccgtgcctgtccgatacacgtgaggaccgagcccgagcgtgtcaagctggtactgggtcgtctgttactgggacccgtggccgtaccctgtttttgcgacggtgaagtggagggccacggtgaacatctggtacctacgacgcagttttgtcgcgggccgctgctctacgtgcaccgacgttgttgttgcggatccgtgaccgccgggcgcgcgctgtcctaccacgttctcgaaaaccacgtggccacgcatgtgctacgcggattgctctcgctgacggaatggaatcgagaattgccgagcctcttttgcgactgtcctggcggcggtggcgcctcgggaaccgaggaacgctacgctatggcctgcctgccgcgcgacctcagcctgcacctggacgactatccttacctgatggtggaaatcggacgcgtactcagtgtcagcgaggtagacgactacgtaaccgccgtctccggctacctgggcgaggccgcggcgccgcgcatccaggttcactacaagctgctctttggactcaacgtgcgtccgcaagcgccgtgcgcgttggacgctacacgcgacttttttctgctggagctgcaaaagctttggctgggcgttgaatatcaccacgaagtcacgtcggagtttttcggtcgcgtactggctcagctgcatcgcgaccgcgcccgcgtcatgatggcgcttcgcttgcccgagcagacggtgtgccacctgagcaccttcgttctcagtcgcttcaagcgacaggtactgtacttcaagctacaggtgagctacggcaagtgccggactggtcacgctgacagaagtgggggaggggggaacggtggaaatcagggacaccacaacctactgtgttatcgacgccttagcgtcacatttgccgacacagacacggtgtggagaaaccttttctacgtttattacgaactagctcgggatctggggtcccatgggacggaggaccgacccgtaagccgcggttacggtgtttcttgcgcttcgaggacgtcgcgactgtcaccgtcagaatcgacggtggtttcggcgaacggacacgcgctgtcttccaccgcgctcccgacgacgagcgcgggtcacaagctgtcactgccgcgcgacccggccgcagatcgcgttcgacgttacgtatgcattatctcgcgtctcatgtacgctcggtacggggagagatggcgtaaacactgtcaacggcggtcggagacgggagaagaggaggaggaagagacgctggaatcgggggagactgacgccacgccgccatttgactttacggggcagcagctgcgccgggcctatcaggaacaccgacgtcgtaaacatctagccgtgcagcgttacgcgccgtgccgtcgtaagctcatcggcgggatggagtttgccgaggtgacgggcgtgagtctagaccgcatcgccgtcaacgctttcaacaccaaccgcgttatcaatatgaaggctgcgctctcgtccatcgccgcgtcgggtctcggcgtacgcgcgccgcggcttcccaagaacatgacccacagttttgtgatgtacaagcacacctttaaggagcccgcttgcaccgtcagcacttttgtttccaacgacgccgtctacatcaactcgctcaacgtcaatattcgcggttcctaccccgagtttctgtactcgctgggcgtgtaccggctgcacgttaatatcgatcacttttttctgccggccgtggtgtgcaacagcaactcctcgctggacgtgcatgggctggaggaccaggcggtgattcgctcggagcgcagcaaggtgtactggaccaccaactttccgtgcatgatctcgcatactaacaacgtcaacgtgggctggttcaaagcggctacggccattgtgccgcgcgtctcgggcgccgacctggaagccattctgctcaaagaactctcgtgcatcaagaacatgcgcgacgtgtgcatcgattacggtctgcaccgtgttttcacgcaactagagctgcgcaattcgtaccagatccccttcctggccaagcagttagtgctgtttctgcgtgcttgcctgctcaagctgcacggtcgagagaagcggctgcagttggaccgcctagtatttgaggcggcacagcggggtctctttgactacagcaagaacctcacggcgcacaccaagatcaagcacacttgtgcgctcatcggcagtcgtctagccaacaacgtgcccaagatcctggcccggaacaaaaaagtcaaattggatcacctgggccggaacgccaacgtgctgacggtgtgtcggcacgtggaagcccacaagatccctcgcacgcgcctcaaagtgttagtcgaggtgctgggcgcgttgcagagtatcagcggtacgccgcacacgcgcgaagtgatccaccagacgttgtttcgattgtgctcggcggccgcagccacatcgggcctgtgttcatcccctcccccattgtgtgtgtcctcatcttcctccgtcccttctgtcccaacctccgtcagcgttgacggcagttctgaacccacgtcgccgcgagcgcggtttgcatcacgatgatggaagccgcggccgctgccgccgcggcgtttcgtccggaggagcgtccgacgccgggttggcacgacgcggcgttgttaatggacgacggtacggtgcgcgagcacgcgtttcgcaacggaccgctgtcgcaactgattcgccgtgtgttaccgccgccgcccgacgccgaagacgacgtggtttttgcttccgagctgtgtttttattgcagcggtcgttttaaccgcaggtcgtccgtcttctccatctattggcagaagcatagcgatctggtgtacgcgcttacgggcattacccattgcgccaagttggtggtggaatgcggtcagttggggagtagtaggctacggtggcgcgacggtgatgcgagtggtgaggagcgccggggagacgacgacagcagggacgagctgtacgacgtgccgggcatttatatgattcgcgtcaacgacggcggcagcaccggccccagacacgttatttggccgggtaccagcgtgctttgggcgccggacgttgtgatcactacggtgcagcgacgaatctcggcggcgcgcgccctggtgaacacgttccgccaatatttttttttgctggaacggcgctcgcacgaggagctggttctttgtccgcccgagatggaggagcgtctagcgccgctgttgcagagtgccacgcgcggtgattcggacatgtttgacggtgtggtggccagcgcttatcaccgtttgcgaatgagtaatattccgcgttcatccgcccgtctgctggaacactgcgtggggctggcgggtgctaagaagctgctcttgctcgacgtgccgcgtctggagaactattttctttgtcaagtctgtctttacgagctggacgaggacgagatgggcgaggagatgctgggcatgttggccggaaagcccgaggatgccgccgtctcgggcgcaagcggcggttttctgctacatcgcaagacgatgaagctggccgcctgtctgtgtttgttgctcaattcgctgcatttgcaccaggaggcgctggaggccttggatcctccgccgccgcgcgtcgaggagaacgaccttgtcaacgtggtgctgcgccgttattatcgcagtcacggcggcgtgcaggcgcggacgctggcggcggcccgggctttgttagccgactacgccgaaacgttttcgcccttggggagttttacgcgcctgggttacgatcgtctcgtttctgccgatgccggcgtcagtcgccggcacctggtggctctgctgcgtgcctagctgaccctgaaacggatggcgtgtatatcgtcacacaggtaggtggccatgatgacggcgatgataagatcgtccgagatacgattctggcgcttggccgagtaacgcgccgtcgtgccttcggccagcgtgacgcggtgcaggttctgaatctgctccagaagatactcgatggggtcgtggctcagcttgatggtgtaggagacgagctcttgcgaggctttgatgtagcccgagttgaaacgcgagatgaactgttccacggccagcgccttgtcgcggcccatgaggtagaagggctgttcgatgtggttctggtcgggcgtgtggtagaagagcacgcggatgagcgtgctgctctgcacgctctgtcggatgaggcaggcgatgcgcacggccgccgcctggttggtgttgccctccacggcgatgcgcagttcgtccaggtaagggtgcaggctcagcaccgagatgatcatgtgcgccgcgcactcggcgatggctacctcagaactctcggagaggtcgcgcaaaaagaaatgctctaggccgtaaatgagaaactggtgtcggtaggcgcctacggccgccacgcccgtgcccgaggccttgcggttggtggtgaaggccgggtccagatacacgtaaagcgtcttgccgaaataatcgtaggcgttggtgttgagcgtgctgtaacgcaaaatatcgaactcttcgcggctctggtccgtgatgagcacggtgttctgcgagattttattggtaccgccgatgatctcgtccatgaaagcgcccggcataaacatgttggccgtcttgcgcacttgcgagttgaggctgatgaaggtgggcttgtgcagtcggtagcaaggacacgccgtggcgtcgcccttctccgtgaagctgtgcaggtgctcttcgcacacgtaagagaccacgttgagcatgtcaaagggcgcattgttaaggcgcgtcaagaaacacgtggagtcactggtagtgttggtggacgatatgaagatgatcttggtggtattctgggccaggaaccccagaatggtgttgaaggcctctttcttgatgaagtgcgcctcgtccaccagcagcaagtggaagttttgtcctcggatgctctgtgtagagaggagacagaaaagggactcttatgattacgcacgctcgactggaagcctacagagtcggggtggggccggacaggtgagccaggtgagccgccaggtgaggcgggatcgccgtgtgccaaccgggctgcgacctgaaaaccggaaccaatccgccgacaccggcgccgcgtgacgcgcgcccataaaaacgaaagtgtcgtcgtcgcgacccgccacagccgccatgaactcgttgctggcggaactcaaccgactaggggtcgcgcacgccactacggaggatgtttttatctttgtcgaccgcctctttcaacacttttccttccttttccaggccgaggagtcaggcccgcgccgcttggaactggtcgcgtccgtgttcgagcacctgacggtggagtgcgttaacgacatcctggacgcctgcagtcacccggacgtgaacgtcgcggagacaagcaacacctgtcgtccctgcccttctcctgttccctccgcccccaaaactgtcagcggcgctcagacgtcatgtgcgacgcctcgggcgcctgtgacatgaggcacgtccagaacgcgtttaccgaggagatccagttacactcgctctacgcgtgcacgcgctgctttcgcacgcacctgtgtgatctgggcagcggctgcgcgctcgtctccacgctcgagggctccgtctgcgtcaagacgggcctggtatacgaggctctctatccggtggcgcgtagccacctgttggaacccatcgaggaggccgcactggacgacgtcaacatcatcagcgccgtgctcagcggcgtgtacagctacctcatgacgcacgccggccgttacgccgacgtgatccaggaggtggtcgagcgcgaccgcctcaaaaagcaggtggaggacagtatttacttcacctttaataaggttttccgttctatgcataacgtcaaccgtatttcggtgcccgtcatcagccaactttttattcagcttatcatcggtatctactcaaagcagaccaagtacgacgcgtgtgtcatcaaggttagtcgtaagaagcgcgaggacgcgcttctgaaacagatgcgttccgaatatggaaacgcacctgtattcggatctggcgtttgaagcgcggttcgctgacgatgagcaattgcctctacacttggtgctcgaccaggaggtgttgagtaacgaggaggccgagacgctgcgctacgtctactatcgtaatgtagacagcgctggccgatccacgggccgcgctccaggcggagatgaggacgacgcaccggcctccgacgacgccgaggacgccgtgggcggcgatcgcgcttttgaccgcgagcggcggacttggcagcgggcctgttttcgtgtactaccgcgcccactggagttgctcgattacctacgtcaaagcggtctcactgtgacgttagagaaagagcagcgcgtgcgcatgttctatgccgtcttcactacgttgggtctgcgctgccccgataatcggctctcaggcgcgcagacgctacacctgagactggtctggcccgacggcagctatcgtgactgggagtttttagcgcgtgacctgttacgagaagaaatggaagcgaataagcgcgaccggcagcaccagttggccacgaccacgaatcaccgtcggcggggcggactgcgtaataacttagacaatgggtcggatcgccgtttgcccgaagcggctgtggcttctctggagacggccgtcagtactccattttttgaaattccgaacggagcaggaacctcctccgcgaacggcgacggcagattcagtaacctggagcagcgggtagcgcgtttgttgcgcggcgacgaggaattcatctatcacgcgggtccattggagccgccttccaagatacgcggtcatgagttggtgcagctgcgcctggacgtaaatccagacctcatgtacgccaccgatccgcacgaccgcgacgaggtcgcgcgtacggacgagtggaagggtgccggtgtctcgcgtcttcgcgaggtctgggatgtgcagcatcgcgtgcgcctccgtgtgctgtggtacgtcaattccttttggcgcagtcgcgagctgagctacgatgaccacgaagtcgaactataccgggcgttggacgcttatcgggcgcgcatcgccgtcgagtacgtgctgattcgcgccgtgcgcgacgagatctacgctgtactacgacgggacggcggcgcgttgccacagcgtttcgcctgccacgtgtcacggaacatgtcctggcgcgttgtttgggaactttgccgtcatgccttggcgctctggatggattgggcggacgtgcgtagctgtattattaaggcgctaacgcctcgtctgagccggggtgccgccgctgccgctcagcgagctcgtcgccagcgcgagcgctcggcgcccaaaccgcaggagctgcttttcgggccgcggaacgagagcggtccgcccgccgaacagacttggtacgctgacgtggtgcgctgcgttcgcgcgcaagtggatttgggcgtggaagtgcgcgcggcgcgttgtcctcgcaccgggctttggatcgtccgtgatcgccgcggacgcctgcgacgttggctctcgcagcccgaggtgtgcgtgctgtacgtcacgccagacttggacttttactgggtgctgccgggcggctttgccgtctcttcgcgcgtcactcttcatggcttggcgcagcgggctttgcgagaccgattccagaactttgaagcagttcttgcaagaggaatgcatgtggaagctggtcggcaagagccggaaacaccgcgagtatcgggccgtcgcttgccgttcgacgatctttagtccggaggacgacagctcgtgtatcttatgccagttgctgttgctctaccgcgacggcgaatggatcatctgtttttgctgcaacggccgttatcaaggccactatggcgtgaaccacgtacatcggcgtcgtcgacgcatctgtcatctacctaccttgtaccaactgagcttcggaggtcctttgggtccagccagcatcgatttcttgccaagctttagccaggtgaccagcagtatgacgtgcgatggtattacgcccgacgtgatttacgaggtctgcatgttggtgccccaggatgaagccaagcgtatcctggtcaagggtcacggtgccatggacctgacctgtcagaaggcagtgacgctaggcggcgccggcgcctggttgctgccgcgtcccgaaggctacacgcttttcttttacattctgtgttacgacctgtttacctcatgcggcaatcggtgcgatatcccttccatgacgcgcctcatggcggcggccacggcctgcgggcaggcgggttgcagcttttgcacggatcacgagggacacgtagatcccactggcaattacgtgggttgcacccccgatatgggccgctgtctttgttacgtgccctgtgggcccatgacgcagtcgctcatccacaacgaggaacccgcgacttttttctgtgagagcgatgacgccaagtacctatgcgccgtaggttctaagaccgcggcgcaggtcacactgggagacggcctggattatcacatcggtgttaaggattctgagggccgatggctgcccgtcaagaccgatgtgtgggacctggtcaaggtagaggaacctgtgtcacgtatgatagtgtgttcctgtccggtgcttaagaacctagtgcactaacggggtctgacagttcacggggagaagaaacaagaaacaacaaaaaaaaggaggacatggactcgccacggtttgtggcaaggcgtatgttatcatcatggagctactcacgttggtgttgtagcaactggcaaaaagcgccgtgctcttggcgccgcggtggtcgatgctgatcacgttgtccttgttctcgaccacgtagtcgcgcgcgaaggtgtggcggcagcggaactcgacctctttgagcacaaactgcgacacgtgcttttggtgcgccacgtagccgatgctgatgccgatcatgtgcttaagcagaaacgagataatggggatgatgaaccaagtcttgccgtgacgtcgcggcaccaggaacacggtggctttctgcttaaagatgtcgatggaggtctgcgagaggaagtcgatctggaaggcgtggatgaggtactgcagcacgcgattggccagcacggggatcttggtcacggctataaaaaagatgacgtgtatcaataaattcttttgaaacggttcgagtcggatggcttttgcgtcgccctcgacggcggtactgaagccgccgtcgagccactttttaaagtcggtcatgaagttgttgatctgctgaaactgcggatcgcggtagagctcggtcaacgcgtccagcttctggtaggaggcgcgctgctcctcggagcacgggcgaaacgtcagtttatcgagcgcgctcttgaggcgctcgtgaaacagcagctcgcgctggctttcctcgggcgagttgtagtcgcggtggcggccgcagaaggccatgagcggcaggaaggcctcgttgcacgagtgggccagcccgagttcggggtgcatcatctggtagcgcttgcggcacagcgtcgccacattggtgaaggccgtggagatgcaggaggtggggtggctcttgcgcttctgcagctccgcgtagcgctcctggatcttggcggccgagtctccgcgcaacatgatggcggcggcggtggtgcgagcggaggttaggcggcagcggcgagaggagaggaaaaagatggcggccgcgaggacgacggaggatccacccgaaaaccacgttgttgcggacgtggctcgtgggacgggcgccgtcactcgttcgtcttcgtcgtccctagtggtgtcgtcttcctcggcgtcaggctcggacgaatcttcctccgcctctcctctcagtttccccgtctcctccccctcaactgccgtcaggtctccggggtccgccggggtttcaacgtccctgtgctcggtggaacggatggtcgagctgtcggcgcagtctccggccgccgatttctcggtctccgaggcttggcgcttcgaggaggccgtaaatatggcgctggtggcctgcgaggccgtgtcaccttacgatcgctttcgcctaattgaaacgcccgacgagaatttcttgttggtcaccaacgtaattccgcgcgaatcggccgaggtgccggtgttggatagcagtagcagcggtggcgatagcgggccggaggacaaaaagaaaaacgtcgggaataaaaccgcgggggaaaagaacggcggtgggtctcgggccaaacgccgtcgtagacgacgcgctccgaaaaacgacgccgccacgccgtcttttctacgtcgacacgacgtgctggagcgtttcgcggccgcggctaagcctttgccgtcgctttgtgtgcgtgattatgcgttacgcaatgctgaccgtgttacctacgacggcgaattaatctacggcagttacctgttgtatcgcaaggctcacgtggagctgtcactctccagcaacaaggtgcaacacgtggaagccgtgctgcgacaggtgtacacgccgggcttgttagatcatcacaacgtgtgcgacgtggaggccctgctgtggctgctgtactgtggaccgcgcagcttttgcgcgcgtgacacttgtttcggtcgcgaaaagaacggttgtcctttccccgcgttgttgcccaaactcttttacgaacccgtgcgggactatatgacctacatgaatctggctgagctgtacgtctttgtttggtatcgcggctacgaattccctgcgccgacgccgcaggcgacgacggcgggtggtggtggtggtagtggtggcggcggcggggccggcgcttgtgcggtcgagacgagcgcgtcagcaggccgggtcgatgacgccggcgacgaggtgcatttgcctttaaagcccgtctcgctggaccgtctcagagaggtgttgcaggcggtgcgcggccgcttctcggggcgcgaggtgcccgcctggccggcctcgtcgcgcacctgtttgttgtgcgcgctctacagtcagaaccgtctctgtttagatctcgcgcgtgacgaggcgcggaccgtgagttatagccccatcgttatccaagactgcgccgcggctgtcaccgacgtcactttgagccacatcttgcccggccagagcaccgtctcgcttttccccgtctaccacgtcggcaagttgctggacgctctctcgctgaacgacgcgggtctcatcacgttgaatctatgacgtcggtcaacaaacagctcttaaaggacgtgatgcgcgtcgaccttgagcgacagcagcatcagtttctgcggcgtacctacggaccgcagcaccggctcaccacgcagcaggctttgacggtgatgcgtgtggccgctcgggaacagacccgatacagtcagcgaacgacgcagtgcgtggccgcacacctgttggagcaacgggcggccgtgcagcaagagttgcaacgcgcccgacagctgcaatccggtaacgtggacgacgcgctggactctttaaccgagctgaaggacacggtagacgatgtgagagccaccttggtggactcggtttcggcgacgtgcgatttggacctggaggtcgacgacgccgtctaacaggtatagcaatctccgtcacgcctctgttcagattttattaaaaaaaaaacacaacataacgacagtgtcggtgtggtagctagtgcagccttaggaacagggaagactgtcgccactatgtcctccgcacttcggtctcgggctcgctcggcctcgctcggaacgacgactcagggctgggatccgccgccattgcgtcgtcccagcagggcgcgccggcgccagtggatgcgcgaagctgcgcaggccgccgctcaagccgcggtgcaggccgcgcaggccgccgccgctcaggtcgcccaggctcacgttgatgaaaacgaggtcgtggatctgatggccgacgaggccggcggcggcgtcaccactttgaccaccctgagttccgtcagcacaaccaccgtgcttggacacgcgactttttccgcatgcgttcgaagtgacgtgatgcgtgacggagaaaaagaggacgcggcttcggacaaggagaacctgcgtcggcccgtagtgccgtccacgtcgtctcgcggcagcgccgccagcggcgacggttaccacggcttgcgctgccgcgaaacttcggccatgtggtcgttcgagtacgatcgcgacggcgacgtgaccagcgtacgccgcgctctcttcaccggcggcagcgacccctcggacagcgtgagcggcgtccgcggtggacgcaaacgcccgttgcgtccgccgttggtgtcgctggcccgcaccccgctgtgccgacgtcgtgtgggcggtgtggacgcggtgctcgaagaaaacgacgtggagctgcgcgcggaaagtcaggacagcgccgtggcatcgggcccgggccgcattccgcagccgctcagcggtagttccggggaggaatccgccacggcggtggaggccgactccacgtcacacgacgacgtgcattgcacctgttccaacgaccagatcatcaccacgtccatccgcggccttacgtgcgacccgcgtatgttcttgcgccttacgcatcccgagctctgcgagctctctatctcctacctgctggtctacgtgcccaaagaggacgatttttgccacaagatttgttatgccgtggacatgagcgacgagagctaccgcctgggccagggctccttcggcgaggtctggccgctcgatcgctatcgcgtggtcaaggtggcgcgtaagcacagcgagacggtgctcacggtctggatgtcgggcctgatccgcacgcgcgccgctggcgagcaacagcagccgccgtcgctggtgggcacgggcgtgcaccgcggtctgctcacggccacgggctgctgtctgctgcacaacgtcacggtacatcgacgtttccacacagacatgtttcatcacgaccagtggaagctggcgtgcatcgacagctaccgacgtgccttttgcacgttggccgacgctatcaaatttctcaatcaccagtgtcgtgtatgccactttgacattacacccatgaacgtgctcatcgacgtgaacccgcacaaccccagcgagatcgtgcgcgccgcgctgtgcgattacagcctcagcgagccctatccggattacaacgagcgctgtgtggccgtctttcaggagacgggtacggcgcgccgcatccccaactgctcgcaccgtctgcgcgaatgttaccaccctgctttccgacccatgccgctgcagaagctgctcatctgcgacccgcacgcgcgtttccccgtagccggcctacggcgttattgcatgtcggagctgtcggcgctgggtaacgtgctgggcttttgcctcatgcggctgttggaccggcgcggtctggacgaggtgcgcatgggcacggaggcgttgctctttaagcacgccggcgcggcctgccgcgcgttggagaacggtaagctcacgcactgctccgacgcctgtctgctcattctggcggcgcaaatgagctacggcgcctgtctcctgggcgagcatggcgccgcgctggtgtcgcacacgctgcgctttgtggaggccaagatgtcctcgtgtcgcgtacgcgcctttcgccgcttctaccacgaatgctcgcagaccatgctgcacgaatacgtcagaaagaacgtggagcgtctgttggccacgagcgacgggctgtatttatataacgcctttcggcgcaccaccagcataatctgcgaggaggaccttgacggtgactgccgccaactgttccccgagtaaccgggacgcggaacgtgacggttgctgaggggaaaggcaacagagaaggtacaaacccaccggcggggaaaataccgaggcgccgccatcatcatgtggggcgtctcgagtttggactacgacgacgatgaggagctcacccggctgctggcggtttgggacgatgagcccctcagtctgtttctcatgaacacctttttgctgcaccaggagggcttccgtaatctgccctttacggtgctgcgtctgtcttacgcctaccgcatcttcgccaagatgctgcgggcccacggtacgccagtagccgaggactttatgacgcgcgtggccgcgctggctcgcgacgagggtctgcgcgacattttgggtcagcggcacgccgccgaagcttcgcgcgccgagatcgccgaggccctggagcgcgtggccgagcggtgcgacgaccggcacggcggctcggacgactacgtgtggctcagccggttgctggatttagcgcccaactatcggcaggtcgagctcttccagttgctggaaaaggaatcgcgcggacagtcgcgcaactcggtgtggcatctgttgcgtatggacacggtctcggccaccaagttctacgaggccttcgtcagcggctgtctgccgggcgccgcggcggcggacggttcgggtggcggcggctcgcactacacgggttcgcgcgccggcgtctcgccgggcatccagttcggtatcaaacacgagggcttagtcaaaacgctggtggaatgttacgtgatgcacggacgcgagccggtgcgcgacggcctcggtctgctcatcgaccccacgtcggggctgctgggcgcttccatggacctgtgcttcggcgtgctcaagcagggtagcggtcgcaccttgctggtggaaccgtgtgcgcgcgtctacgagatcaagtgccgctacaaatatttgcgcaaaaaggaggacccctttgtgcagaacgtgctgcggaggcacgacgcggcggccgtggcctcgctgttgcagtcacacccggtgccgggcgtggagtttcgcggtgaacgcgagaccccgtcggcacgcgagtttctgctttcgcacgacgcggcgctcttcagggccacgctcaagcgcgcgcgcccgctcaagccgcccgaaccgctgcgcgagtacctggccgatctgctgtatctcaataaggccgagtgttcggaagtgatcgtgtttgacgccaagcacctgagtgacgacaacagcgacggggacgccacgatcactattaacgcgagtctcggcctagccgcgggcgacggcgctggcggcggcgctgatcaccacctgcggggcagcccgggcgattcgccgccgccgatacctttcgaggacgaaaacacgcccgagctgctgggccggctcaacgtgtacgaggtagcgcgcttttcactgccggcttttgtcaatccgcgtcaccagtattactttcagatgctcattcagcagtacgtgctcagccaatactatataaagaagcatccggacccggagcggatcgatttccgcgacctgcctaccgtctacctggtctcggccatcttccgcgagcgcgaggaaagcgaactgggctgcgagttgctggccggcggtcgcgttttccactgcgaccacatcccgctcctgctcatcgtcacgcccgtggtctttgaccctcagtttacgcgccatgccgtctctaccgtgctagaccgttggagtcgcgacctgtcccgcaagacgaacctaccgatatgggtgccgaactctgcaaacgaatatgttgtgagttcggtaccacgcccggtgagcccctgaaagatgctctgggtcgccaggtgtctctacgctcctacgacaacatccctccgacttcctcctcggacgaaggggaggacgatgacgacggggaggatgacgataacgaggagcggcaacagaagctgcggctctgcggtagtggctgcgggggaaacgacagtagtagcggcagccaccgcgaggccacccacgacggctccaagaaaaacgcggtgcgctcgacgtttcgcgaggacaaggctccgaaaccgagcaagcagtcaaaaaagaaaaagaaaccctcaaaacatcaccaccatcagcaaagctccattatgcaggagacggacgacctagacgaagaggacacctcaatttacctgtccccgcccccggtcccccccgtccaggtggtggctaagcgactgccgcggcccgacacacccaggactccgcgccaaaagaagatttcacaacgtccacccacccccgggacaaaaaagcccgccgcctccttgcccttttaactcataaactttcaggtctcgcgtacgattcgcgagtcgggaatgggacacccgtgggtgtttctccgtgtgtatattattttttttttttgtgtgtgtttgcgcccccgtgtgtctaatgtgctgtttgaaacacgtaaagtagctggtggaagaacagataaacctttaataaaaaaaaaagtatgtgctcccgacccacggtctgcgtgtctcttttttatgtccatgtctccaagtctggtgcgggtggcggcggggttaagcgtcctcgaagtcttcatcatcgtcgtcgtcctcttcttcgcggaggcgacggctttccaagctgtcgtggtgactgagcacagcgacttcttcgccggaggctgtggccagcgcctggtacttgacactgccgctaccgcgtccgcgaaagtagcggacggcgcgacacgtcgtaaacatggcccatatgaaaaagagcatgccgaacgaccagctgatgccggtgcggtattcgttgctgaggaaggtatcgtactgcacgatggggtagatgaggccgcagagtccaaagaaggcgcccaggtggtagccgaattgcaccttgacgtattgaaaaaagacggcctcgatcagtaaaaagtagatgatggagatgatagcgtagaccacgaagacggctaacaccatgtggcctgtacgcacgaaaaagttgtttccgaagccgtagcacagggccatggctaccacggtggtgttgaaaccaagcgctacctctaccaggttgacgatgagcgtgcggaactgcaccgtacctttgagcttggggtgcagacgcgagaagaaaaagagtgagcgtttgtagctgcggtactgcgtgaccatgctcacgttgaaaatggtcaggcagaaaaagtgcacggcggccatgaaggcgatcatgctgggcagccgaaatgacatggtcagtgtgaatagttggaacgtgtccatgctgagaatgaagaggaaggctgtgaggctgtcgcccatgtacgaaatgtcgcgtgtcgactggtttaggctcatgcctttgtccttgcgcatgctgatcttgatccagcataccaggtagtagatggtcacggctaaaaagacgagctgcatgaacacggcgtagcacaccaactgcaccgagtctaagaaaagcataggcgtgtgcaggtgcattacgttgtaggccgacatgttgagcctttcaaagtccacgacgtgatagtagacgcaggggtagcccaggtgcggaaaattgctcagcactagatgcacgctgacgttgacaaaagtcagcaccatgaaaacgatagaagcgctccatgtccgtgtattcaccttatccacgtgcgagggggccatggcgatagcggcggcccgctcgctcgggaggcgatgggggcgcgccgatgacgacaggctcgcgggtcgttaaatactacgatgggagccgccgcggctcacgacgcggtttgagcacgtccgggcggtcggtgaaaaaagaccccgcgggccttcgcgactctcttctgtccgaggatgaccgctcagccgccgctgcaccaccgccaccacccgtacaccctgttcgggaccagctgtcatctcagctggtacggccttctagaggcctcggtgcctatcgtacaatgtctgtttttggatctgggtggcggccgtgccgagccgcggcttcacacgttcgtggtgcgcggtgaccgtctaccgccggctgaggtgcgtgctgtgcatcgcgccagctacgctgcgctggcctcggccgtgactacggacgccgatgagcgtcggcgcggcctagagcagcgtagcgccgtgttggcgcgcgtgttgctagaaggcagcgcgttaatccgcgtgttggcgcgcaccttcacgccggtgcagattcagacggacgctagtggcgtggagattttggaggccgcaccggcactgggcgtggaaaccgcagcgctgtcgaacgcgcttagtcttttccacgtagccaagctagtggtcatcggctcgtatcccgaagtgcacgagccgcgtgtggtcacgcataccgcggaacgcgtctccgaagagtatggcacccacgcgcacaaaaaattgcgtcgcggttactacgcctacgatttggccatgtcgtttcgcgtcggcactcacaagtatgtgctggagcgcgacgacgaggccgtcctggcacgcctctttgaggtgcgcgaggtgtgttttttgcgcacctgtctgcgtctggtcacgcctgtcggtttcgtggccgtggcagtgaccgacgagcagtgttgtttattgctgcagtcggcctggactcacctttacgacgtgcttttccgtggtttcgctgggcagccgccgctacgcgactacctggggccggacctctttgagacgggcgccgcccgttctttcttttttcccggtttcccgcccgtgcccgtctacgcggtccacggtctgcacacgttaatgcgcgagacggcgttggacgcggcggctgaggtgctctcgtggtgcggcctgcccgacatcgtgggctcggccggcaagctggaggtggaaccctgcgcgctctcgctcggcgtgcccgaggatgagtggcaggtcttcggtaccgaggccggcggcggcgccgtgcgtctcaatgccacggcttttcgcgagcgaccggccggcggcgatcgtcgctggctgttgccgccgctgccacgtgacgacggcgacggtgaaaacaacgtcgtggaagtcagcagcagcaccggcggtgcgcacccgccgagcgacgacgccactttcaccgtgcacgttcgcgacgccacgctacatcgagtgctcatcgtggatttggtcgagcgcgtgctggccaagtgtgtacgcgcgcgcgacttcaatccctacgtgcgttatagtcatcgactccacacttatgcggtttgtgaaaagtttattgagaatctgcgttttcgctcgcgacgcgctttctggcagatccagagtctgctgggctacatctccgagcacgttacgtcagcctgcgcttcggccggccttttgtgggttctgtcgcgcggccaccgcgagttttatgtctacgacggctattcgggtcacggacccgtctcggccgaagtgtgcgtgcggactgtggtcgactgttattggcgcaaactttttggcggcgacgatccgggtcccacctgtcgtgttcaagagagcgcgcccggcgtgctgttggtctggggcgacgagcggttggtgggtcccttcaacttcttctacggcaacggcggcgccggtggtagtccgctccacggggtggtgggtggtttcgcggcgggacattgcggtggcgcttgttgcgcgggctgcgtcgtcactcaccgccattctagcggcggcggtggtagtggcgtgggcgacgcggaccacgcgagtggcggcggtctagatgccgctgccgggagtggtcataacggcggtagtgatcgggtttctccctccacgccgcccgcggcgttaggtggctgttgctgcgcagccggtggcgactggctctcggccgtgggtcatgtcctgggccggctgccggcgctgttacgggagcgcgtgagcgtgtccgagctggaagccgtgtaccgcgagatcctctttcgtttcgtggctcgccgcaacgacgtggacttttggttactgcgcttccagcccggtgaaaacgaagtaaggccgcacgctggggtgattgactgcgcgcccttccacggcgtgtgggccgagcagggccagatcatcgtacagtcacgcgatacggcgttggcggccgatatcggctacggcgtctatgtggacaaggcctttgccatgctcacggcttgcgtggaggtctgggcgcgagagttattgtcgtcctccaccgcttccaccaccgcttgttcttcttcttccgttctctcctccgccttgccgtccgtcacttcgtcctcttcgggcacggcgacggtgtctcctccgtcttgttcttcttcgtcggcgacttggctcgaggagcgcgacgagtgggtgcgctcgctggcggttgacgcgcaacacgctgctaagcgggtggcttccgagggcctgcggtttttccggctcaacgcttaacgagtcacgtaggggaactacgtgggtaagtgacgtggatactagtaaaaaaagtgcgtcaaagctcttagcgtgtgacgtggatactagtaaaagggacgtcaaagctcactacgtgttgcgtgttttttttttttctatgatatgcgtgtctagttcgcttctcactcttcctctcctcgttcccagcgcggcggcagcttggggggtgagggcaaattggggtagttggcgttgagcacgtctagcaggcccaggcccacgggccaaccgtccacggtcttgcgctcggtcagcttgaggctgaacgagtgtgcctcgtcctgaccggtaaggcggaaaaagaagcgtgctaccagctgcaggcaggtatgccgcgtctgctggaagagcacgaaggtagcgggcacgtactgcacaatgtgcggctctttttcctcaaagagcaggtagagcgcgctgcagatcagccgcctggcgctgtggtgcagcagccggccgaagctttcgcgcacgttcaccgcgtccaggtactggagcaggtcgtgcaggcacttgcgcgttaagttgcaattttccacgcacgaaataacggtacagagcgcgaagtgcagcaggttgtcggctttgacgatgccgcagcggtgtttgagccgcagatccgagagcctcacctgcgtgacggcgtcttcggtctcgagcaaaaacacggcggagtagcctagaaaggccgaggtgcacagcaactcgctgcggtactcggccatggagaccagcagcccgtgctccgtgtgcagccacagcttgtcgccgcgcaccgtaaagtcgagcacttgcggctccatgatcatcacattctgtctagtgaaatccgtatggacctccagcacgccgcggatcatcagggcctccatttcgaaatcggccgacacgctctgggccgcgccgctcctcgtctgccgtgatcaagcggcgcggcgcggacctttcaagtgttcctgggccgccgctcgaggcagttcccctttctggcactccgcccgccgcttcgcggctcatttggcgccgacgcgccttctcgcggctgcaaatcagctccacgtatcggcaaaacttgctgtcgtcgtaggcggcggccacgatctcgccgaaggagagctgcaggtaggcctcgggtacggggtccagcgtgcccagcgccaggatgtgacacagatagggcagggtcacgcgctctaccgtgtaattggagtagacgatggcctcttcggccccttgatgcgtgaccagacgccgtaggcgaaaggtacggaaatactcgttttcccacaactgcgtgaggaagcgttccagcgactcggtgccgggcacgaactgcgagaagaagctgttggccaccaggcggttgtcttccaccgccagcggacggaagggcgccgcgtcgcgcgccttgcgcacggcctccaacacgggcaggtggtagagttcggcgtcgcgcgcgcccaggctcatggagtcctcgcgccgcgaggcgtagcgcgtgagcaggtcgcgcagttcgcgcacgcgattctcccaggtctggttaagcgtgcgcaggtcctggatctcgtccacctgcgactggatctgctcctccaggcacttgataacctgcttcttaaacaggtcgcggatgtcccgctcgggcgccgccgggccgggtggcggcggcagcagcccgacgtggcccgcgggtcctcccaccacggcgccgccgggtcccaccacgccgggtccgcccggaccacgcgcgggtagtagacggttttggtccaccagcgagggggtcaggtcctgcagaaaggactcgacgctgtcctcgatgccgatgcgcgatttgctgtccgagacgttaagcaaaaacttcataatggactttttggcgtcgctgccccggtcgtgctgctccatcatctccaccagcttcttgcagttgagctcgtggcggctggcggtcaccactttcacaggaaaggtattgagcaactggcagatcttttggtggcggcagagcccgtcgtagcgcagaatctcctcgtgcaggtgtgccaccggcgtggtgaacagcagcttgtcgcgctcataagccagcggttcggccgccacgtacaagcggatgtgcttgccgcgcagctgcgcctccagccgctccgagcgcaccttcttgaagacgcgtacctcgggcgcgttggctacgcgcacggcgcccaggcgctcggccacctgcagcagcagcgccaggttagcctgcagcaggtcctgcgccagcgggtgtgtctcggtggcccgctgcacggccgcgcgtacaaattgcgcccgctcggccgcctcgctcggcttggtcttcacgtccagcagcggtaccagtcccaccgttacgcaccaatccacgtagagaccatagtcgtcgttatcggcgtactgatataaaatgtcgcggagcgcgcccagcacgcccgtttgcacgctctggcgcaacgaggcgctccacaccaacagatactgctccaggtcctcttcgtccagcgcgcggtagggaaatagcgccgcgtgcaacttccactcctcggccacgcgccgcaccgtgatggtgtcaaagagcgttttgcacactccgtagagcagctgcttgcgcagcacgcacgggtcgcgcagcacctggtgcatgctttggccgcgacacgtccccagaaagccgtgcagcaaccgcaggaagctcatcgtctgccccgtggggaaaatgtcgatgacggcctcgtcatccacgccgcggcccacgcccaagtacgacgacgccttgatcctcaacctctcgtcggccgccaagatcgaacggatcgtcgacaaggtcaagtccctctcgcgcgagcgctttgcgcccgaggatttttcgttccagtggtttcgctccatcagtcgcgttgaacgaacgacagataacaacccctctgccgcaactaccgccgcggcaacgacgaccgttcactcctccgcctcctcttctgccgccgctgccgcttcgtccgaggccggcggcacgcgcgtgccctgcgtcgaccgttggcccttctttcccttccgcgcgctgctcgtcaccggcacggcgggcgccggcaagacttccagcatccaggtgctggcggccaatctagattgcgtgatcaccggtaccacggtgatcgccgcgcagaacctcagcgcgatcctcaaccgcactcgctcggcgcaggtcaagaccatctaccgcgtcttcggcttcgtcagcaagcacgtgccgctggctgacagcgccgttagccacgagacgctggaacgctaccgcgtgtgcgagccgcacgaggagaccaccatccagcgcctgcagatcaacgatctgctcgcctactggccggtcatcgccgacatcgtggacaaatgcttaaatatgtgggagcgcaaggccgcttcggcctccgccgcggccgcagccgccgcctgcgaggacctctcggagctgtgcgagagcaatatcatcgtcatcgacgagtgcggccttatgctgcgctacatgctgcaggtggtggtgtttttttactacttttacaacgccctgggcgacacgcgactttaccgcgaacgccgcgtgccctgcatcatctgcgtcggttcgcccacgcagaccgaggcgctggagagccgctacgaccactacacgcaaaacaagagcgtgcgcaagggcgttgacgtgctctcggcgctgattcagaacgaggtgctcatcaactactgcgacatcgccgacaactgggtcatgtttattcacaacaagcgttgcaccgacctggactttggcgacctgctcaagtacatggagttcggtatcccgctcaaggaggagcacgtggcctacgtggatcgcttcgtgcggccgcccagctccatccgcaacccctcgtacgccgccgagatgacgcggctttttctctcacacgtcgaggtgcaggcttacttcaagcggctgcacgagcagatccgcctgagcgagcgccaccgtctctttgatctgcccgtctactgcgtggtcaacaaccgcgcgtaccaggagctctgcgagctggccgacccgctgggcgactcgccgcagcccgtcgagctctggttccgccagaacttggcgcgcatcattaactactcgcagtttgtcgaccacaacctctccagcgagatcaccaaggaggcgctgcgccccgcggccgacgtcgttgccaccaacaactcctccgtccaggctcacggagggggaggatctgtaatcgggagcaccggcggcaacgacgagacggcgtttttccaggacgatgataccaccactgcgcccgatagccgtgagacgctgctcaccttgcgcattacctacatcaagggcagttcggtgggagtcaactctaaggtgcgggcctgtgttatcggataccagggcacggtcgaacgtttcgtggacatcttgcaaaaggacacgtttatcgaacgcacgccctgcgagcaggcggcctacgcctactcgttagtttcgggcctgctcttctcggccatgtactacttctacgtgtcgccctacacgaccgaggagatgttgcgtgagctggcgcgcgttgagctgcccgacgtgagttcgctctgcgccgctgccgccgccacggccgccgctcccgcttggagcgggggagagaatccgataaataatcacgtcgacgcggattcttctcagggcggccagagcgtgccggtatctcaacggatggaacatggccaagaggagacccacgacatcccctgcctgtccaaccaccatgacgactcggacgccatcacggacgccgaactcatggatcacaccagtctgtacgcggatcccttttttctcaaatacgtcaagccacctagcctggcgctgctttctttcgaggagacggtgcacatgtacactaccttccgcgacatttttctcaagcgctaccagctcatgcagcgtctcacgggcggtcgcttcgccacgttgccgctcgttacctacaatcgccgtaacgtggtgttcaaggccaactgtcagatcagctcgcagaccggctccttcgtgggcatgctttcgcatgtgtcgccggcgcagacgtacacgctcgagggctacaccagcgacaacgtgctcagtctgcccagtgaccgccaccgcatccaccccgaggtggtgcagcgcggcctttcgcggctggtgctacgcgatgcgcttgggttcctctttgtgctcgacgttaacgtttcgcgcttcgtcgagtcggcgcagggcaagagtctgcacgtgtgcaccaccgtggactacggcctcacttcgcgcacggccatgaccatcgccaagagtcagggcctgtcgctcgagaaggtggccgtggactttggggaccatcccaagaacctcaagatgagccacatctacgtggccatgtcgcgagtcacggaccccgaacacctcatgatgaacgttaacccgttgcgactgccctatgagaagaacaccgctatcaccccctatatctgtcgcgcgctcaaagacaaacgcaccacgcttattttttgacacaacaccgtgtaaggaaaacgtgactttattgagcagggtaaaaaccacgtacaagaaccacgttgtctatccccaaaaaaacacacaccgtcagggaacacatcgcctatagatagcggcactttacataaaaccaccgtacctgcatcacggtggctcgatacactggaaattcaataaaaaccaccgtgtctccgtgacggtacttatcgggtcagcgtcttttgagatttctgttcgtaaacttatccgtttccccggtccgcggtgtctcctcgcgaggctgacagtcgacgggtggtacctgcaagagaagaaacccgggtgggagcgacgccgtcgctgggtatcaaccccgcggctgaccgtcgtccggtaaaggaacaacccgtcgtcgcaagccgggttcgaccaagagaaaaaacccgggtgcggggggagacgggtcgtcctttggttgttcgcggacggcgtacatgccgcgtgggtcagtcgacggcgtcgctccgtgcggtcggtcatcattctgcttcacatatatgggttgtttgtgtttttttttataatgaatacgcactgatcctatccgtgactgcgcgtgtggcagagaggatgccttataacatgtattttgaaaaattgccaacagctataatttctctcatgtagcagaatagagaccttttgtcgtctttttgtttgtcattacttgttttccagggaattagagagagggaaccgcgcctccggcggcggtgcccgcggaccccggccccttctcgcgtgcgcggtgtgactggttgagcgaatgagcagctaggcttggtggtgctccgcgtgcgggggagaagacgattaacaacaaaaaataagtggaagtggccggtgggtctttgtccgcgtgcgcgcccatccgtcgccgggaccgagcagaaagtgatgtggtggtacattgattttttccttgacaggaaagaaaaaaaagagttttgttttcctatgtgagaggagaaaggtatgtgaggagatgttcgatgatcgtatgttacagttatgctgtaaggaagcttttatcgtgcgtcctgtttttcatttgatgtatatgacacaattgaaacctatcgataggcgtatatcgaggattcatcaattcttagaatcgtcgtctttttggctaattggactttgcccatgttggttgtcattcgtggcctgaggtcatcgtcgtccacgacgacgtgtctatagcgtgcggtgtgatcattgtgtcgagccagagaaagcgcgcctcgcacgacgtttgcggatcggctcgcgggtgtgtggaattcctaagaacataatcagctggtcgtctttctttgatgtgttgttgtcgtcgaggtcttgcttcgttttcttttttctttttagtcgatggaacttttcttcggtacgggttcttgttatggaagcttgtgttttcgaacatgaattcgaaaaaataaaaaggcctatcttcgtttcaaaaaaaggacagatatcaatcttcttaacttatatcatggtaaattcagaatcctatggtgtcttattatctctaaagtagtcaacattatggtctaacttgtatttccctgacgagatatatatgatccttataacctggctactatcatgaacaacaatatccttacttacagtcatcttcgtgagttaatgaagtataatatcggtcatctatcaacttatctgctatgtaacgtacccttttaggtattttgcgtttcttaacgagtgtacccgcctgtgtgaggcgaaactctgagaagtctaccgagtcgagttacaagtcactaaaacacttacacgagttatctatactaaaatcactatctatgttgtttgcttacctaattattatcctacatgacgaagctacctcccaacgtaaggtagggggagaggagacagaacaataaaaagtaactaatgtttcttagaacttacccgctaaggacttaccaaactatattcaccaaaaaacaacagctacgtgtttcatttgttttaatctaccgaagtaaaaaaaaaaagatgattagctatccagaacctacttacttcttaatgttttaactaaggatgcctatgggattggaaaaaaaatcacagcaacttgctactaatcagttgacagcgaagagactcataacaaagatttctgggtaatacggttataataatgcttatggactaaaggatacttggaaaaaaagaacgggctatgactatagagattcgtcgagatatcaaacttcaaataggcggctatcattcatggttgtggtgactatatcgtggagaaaaaatgtgatcgttagttagctaggtgagacttacagctatccatccgtctagtttttcgttgtaatgatgatagtacgtctatggtggtgatcgattttggttaacaatttgttcgtttaaaggcttaatgtacttatgctacatgatgtattattctttgattcatcgttcctcctaagggggtgtatgtatgtatgtactagtcgtatagtgttcctaacatcatgactattcagactatggcttcatctatcgtgtctaaagttcacttattctactattactatatatatgcactactatgtaactaggatatggtcctataaggtgtcttctatcacggtggcttgtttatcgcttggcggttacgagcaagagttcatcacggaccagccgtgaggcagggcacacgcgggtcggcggcgatgatgtcccccgcgaaggggacaacgaaaacaagaggccgccggccgcggccacggatgcgtagcggttacacaatgtttggttgagcgttttgtttcatcgtcgtggtggttttgttgttctctgtatatatcgtgtggtggctttatcgtcatcattattatcatcattcttgtttccatcatcacgatgagttttctccgttttcctctcctccagtggtagtcgtgtatcatcatcaatcatcgtagtgacgtcgttgctgctgctgctcttgccttcatggcggtatttctcttcctcccccctaaccccatattaactcgtgagtgtgatggttagagtggctgcttgttttttttttcttttctctttggaacaacaaaagaggataaagatggtcggtgaatgtattattattatcatcattatgatacggtcgcggtcttcttctccgatgacgaaacctgcgcacatcgaagaaaagacgagcgcgcgaaccgatagccgtccgtctgggacgaaggagaagatgatggggagaggaggagagccccagaagccagagcgagaagggagacgacagacatacgtcgtcaccgtcctctggaggaggcacggcggcgctgtttgttgtttggatgcttgattatatcctgttctatggggtagattattatcaataggcttggttttcaaaggtcagcctgtgtattgtcgtgtctttttttttcgttctcatgatcgcggagaccacacagacgtgcgcgtctcccaatggctaggcgttctttttaggtagtaattttttgatcttttttttttcttaacaagtctggcttgatttcttttatctatgatcgattcttctttttctcgggggttgcatcttccgtgaaagtaaagtgacactactctaaatggtaaccatattatctgttgattaggagaaaaaataattttttcgcacgaaatcgatcctaagtgaggtgatttacttgctatcacacgaaatgattatcttttgctgctaacgtactgaattttttaacagaattgcttctccgtaactatttccgcagattcagacagattgtcaaaaaagaatacggcacagaaatagtgggtctgtggcttttggttcgtgtacattcgcgtttgcgtgtcgagatttctacggtatgtttattcttcctgcgatgatgtagggtccttggtgtaagtaggatttcgagtatctctcttagagcgaacaaaataatcaaaaaacaacagctaggaaatcgagggttactctacgataaagtgtctctacaaagtgaagaatgttacgttgtggtggaataataagactcgcgtgatcgatgagtgatcgagagcggctcgaaccttctttaagagctttgtttagtgcaactttaaattacaaggagtagaaagctgaaatgaatctatgaaggtgctattctttgaatatcttactttgtacgcttcacattcgttatttggatagagagttgtctagagaaaatctgtgattctctatgagtgttatttttattatccttttggggactacgatttttcttcttgttctacataccactactactcgtaatcacatacatggacgaaaaaaaaattcgtcaggcagtagataccagattctccgacgttacggcgtcttttttttcttttgagagagtatctgctgagattgtccgtggtgtatctagtcgctatttttgttgttactagtagttttgcacacagtttattcagtatagtttttcttcttgccatgatcaattaagcccaccacctttttttttagagaggaggaatttcgtcttgatctccagccggagacaacggcggtggtggtggtggcgggagagacttcaaggcaatgaaaaaaaaaatttcgttttgccatcaagtggtgacgataacccgtcagattgataattggttcctacagaaactattctaaccgcggaagaaagaaattgaaaaaaaaaattgacaaaaacatcataacataaaggaccacctacctgggacgcgcagttgggcggcggactgggacggcatgctgcggcgatgctgtcggtgatggtctcttcctctctggtcctgatcgtcttttttctaggcgcttccgaggaggcgaagccggcgacgacgacgataaagaatacaaagccgcagtgtcgtccagaggattacgcgaccagattgcaagatctccgcgtcacctttcatcgagtaaaacctacgttggtaggtcacgtaggtacggtttattgcgacggtctttcttttccgcgtgtcgggtgacgtagttttcctcttgtagcaacgtgaggacgactactccgtgtggctcgacggtacggtggtcaaaggctgttggggatgcagcgtcatggactggttgttgaggcggtatctggagatcgtgtttcccgcaggcgaccacgtctatcccggactcaagacggaattgcatagtatgcgctcgacgctagaatccatctacaaagacatgcggcaatgtgtaagtgtctctgtggcggcgctgtccgcacagaggtaacaacgtgttcatagcacgctgttttacttttgtcgggctcccagcctctgttaggttgcggagataagtccgtgattagtcggctgtctcaggaggcggaaaggaaatcggataacggcacgcggaaaggtctcagcgagttggacacgttgtttagccgtctcgaagagtatctgcactcgagaaagtagcgttgcgatttgcagtccgctccggtgtcgttcacccagttactttaataaacgtactgtttaaccacgttgcgtcgtgacgttgtttgtgggtgttgctaggcgggctggaaagatgatgtataaatagagtctgcgacggggttcggcgctctgccggctgcggcggcactcgctccacggcctccgacgagcgttgcgctcgcgctttgcgccgccgcgtcatggatctccctactaccgtcgtgcgaaaatactggacttttgcgaatcctaatcgcatcctgcatcaaagcgtcaatcagactttcgacgtgcgccagttcgtcttcgataccgcgcgtctggtcaactgcgtggacggcgatggcaaggtgctgcacctcaacaagggctggctctgcgctaccattatgcagcacggcgaggcttcggccggcgccaagacgcagcagggcttcatgtctattgacattacgggcgacggggagctgcaggagcacctctttgtacgcggcggtatcgtcttcaacaaatccgtctcctcggtggtgggctccagcggacccaatgagagcgcgctgctcaccatgatttccgagaacggtaatttgcaagtgacttacgtgcggcattacctgaaaaaccacggcgaatcctccagcggaggcggtggttgcggcgccgcgtctaccgcttccgccgtctgcgtgtcctcgctgggtggcagcggcgggactcgcgacggcccttctgcggaggaacagcaacggcgaaggcaggaacagcgtcacgaagaacggcgcaaaaagtcgtcctcgtctgccggtggtggtggaggcggcggcgctggtggtggcggtggcggcggcgggagcggcggtcagcactcctcggactccgccaacggactgctgcgggatccccggttgatgaaccggcagaaggagcggcggccgcctccctcctccgagaacgacggtgagtcccggccctcctcgcgtcacggtgctttccgagtggactcgtgagcctcccgtagcgcacgagcgagcaggcgagcggtgttggtgcgctggtggttgtgtggatgataaccatgtgctttttcgtgcgctatgtgtcgtcccgtctgtaggctctcctcccctccgggaggcgaagagacaaaagaccaccgcacagcacgaaggccatggcggcggcggcaagaacgagacggagcagcagtccggtggtgctggcggtggtggtggcggcggcagcggccgcatgtcgctgccgctggacacgtctgaagcggtggcctttctcaattactcgtcctcatcctccgcggtctcttcttcctccaacaaccaccaccaccatcatcaccaccataacgccgtgacggacgtggccgccggcaccgacggtgcgttacttctacccattgagcgcggagcggtggtttcgtcgccgtcgtcgacgtcgccgtcgtcacttctttcgctccctcgacccagcagcgcccacagcgcgggcgagacggtgcaggagtccgaggcggcggcgacggcggcggctgcggggttaatgatgatgaggaggatgaggagggctccggctgaggcggcggaggcaccaccgcagtcggaggaggagaatgattccaccactccagtctctaactgccgtgttcctccgaattcgcaggaatccgcggcgcctcagcctcctcgcagtccgcgttttgatgacattatacagtcattgaccaaaatgctcaatgattgtaaggagaaaagattgtgcgatctccccctggtttccagcagactcttgccagagacgtcgggcgggactgtcgtcgtcaaccacagcagcgtcgcgaggaccgccgcagctgtctccgcagccggcgttggccccccagcagccgcatgtccgccactcgtcaccaccggtgttgtaccctcaggttccgtcgccggtgtcgcgcccgttgccgccgcaatcgaaacaccagctgctcctccccggcccgtgtgtgaaatcaagccctacgtggtaaaccccgttgtcgccaccgccgcggctgccagtaactcttcctcgtcttcttcggctccactgccgccgccgccaccaccgtcgggcggacgtcggggtcgggcccggaacaatactcgaggaggcggcggtggtggcggtggtagaaacagccggcggcaggctgcatcgtcgtcgtcctcctcctctcggagatcgcgacggagaaacaaccgccacgaggacgaggaggacaacgaccctctgctccggttgtcgcaagttgccggcaacggccgccggcgagggccctcgttcctcgaggacggactcgaaattatcgatcccagcgaggaggctgcgatcgccgccgcctcgatcgcggcgtttttcgacgattaaaaaaccgagccgagaccggaaaaaatatgaaacaggacgcgcttggacatttgggtttccaccccttttggtgtgtgtctatatatattggtcactgattttttttacaataaagagatagacatcacagttcaccaccttgtctccccggtgtgtctattatcatcaatcacccacagagtcgccagtccatggtctctcggtaatgcgtgtccagatacgcgttggccagtataaaatggtcgttgcccacgaaggcgcgggtggtgttgcgcggcgacgggtggcaggacttgagtaccaagtgccgccgtcggtcgatcaggtactcgcaggtgtgcgcgtcggcgccccacagcatgaacaccagatgctcccggcgctctgacagcctccggatcacatggttactcagcgtctgccagcctaagtgacggtgagatccaggctgtccgtgcaccacggtgaacacggtgttgagcagcagcacgccgcgtcgcgcccaggcgtccaggcaacccgaggccggacgctgaaacccgtccaccgtacgcgccagttcgcgaaacacgttgttgagggagggcggcggcggtcggcccgccagcgtgccgaaggccaggccgctggcgctgccgtcgcagtacgggtcctggcccacgatcaccacgcgcacctgctcgggcggacacagatagctccagcggtgtacgtgctcgggtgccgggtacaccatctcgagttgccgcgcgccctccaccgccgccaccgtgtcgcgcagcagcaccgtgtcgtggtcgggcaagctgaggaagcggatccagtcggcgctcagacaaaacacgcgagcctgctcgtcgggggttaacagagagcctttattatcagcaatgttagcgagcatccactgcttgagggccatagcgcgagtgagccggcaggttgacgcgcgtctgcttcagctcgggcggcagtccggcgtagtatttatctaggtggcgtagtagcggcgggtccagctggtgacgcaggcagaattccttcactgcgttgtacaggccgtaaaagagtgtgatgccctcgggcgcggcagcggtgctcacgggcagacgcacggcgcggttggtacgcgtggcttcgttgcgtatggccaccaccacgttaaagagagacggtggcaccagctcgaagcctaacacgtgttccgtgaagatgctgcgcccgtatgacagtcgcgtgaggtcgtagccgcggcacaggtcgtccacgcacgtgtacacggccggcgagccatcgccgcactcgctgtagccgcgcatcaccgtcatccagcgcggcgctgtgtccgagctcaacagcgtcagcagggcccgcaattgatccggattgttgtacagcagggccagagtgtccaggaaagcatcgtccaacagcacggagttggcggcctccggcgtaacgggacggtaacgaataagttgcgatagcgggccatcgcgtctggtaacattcaccaacgggcgcagccaactttcatacttgtcaccctgaaacacctcacccaacaggcatcgacgcgttagttcggggcactccgcggggactttctcggcggcggtaggagcgacgctgacggcgactgaggaaacaatgggcagcagaaggcaacaccacagcagtaccaccggtccaggtgagaaagagaagccgcaatccgggcggcggcacatcaagtctgcggcacgatgagagtgtgacggtaaggagccagttggcgccgaaagttggcgctcaggtcttcgatccctaaaacgttatatattgcatccagcaggtgagccaggctaaacggattcacgtaccaggtttggttacccgcgacgatgacggccagaccgtgggcgctacagttggagaggttcctgggtacgaaggtaactgagtcgatgtcgcgccacggggggaatgagacagacgactggcgcacgctgtaatcacaactgtgattgacgtgtagcgtgtaatttcggttgcactcagcctcgaagtagagggggaaccacagttcgtcgtactcgtcgtcgtcctccagttctggctcttcttcatccaccgcaatgtctacgctgctctgagattcctcttcgtacaggatgattgacaggttatggctacacaggtcctgggcgggaggacgcgtgggagcgcgggtggtggtaatgttttccagatcgtcaaaagtcggagtgtagtctgacgccgtgacgacaccgtcgacggagatggtagaagttgcggccggtgtcacggtggtaagtatggatacagaaggggagggggaagtagcgttcgtaccgatggttgtggtattattattccctgtgtttcttgttccagaaaccgttgacgttgagatgggaatcgacgtggtgctggacgtcagattgctgaccgaggaaaccgtggtgggagtggtgacggtgttactcgtggttgaagtgacgttaggggaggtagtagtggtaccggtggtggcgacggtagtgtttgtcgtggcggcggcagcggtggtactggtaacggtggtcgcgttggtttccaccgcttcacacagtaagcaaaagcacagggccgggaaaagcaaccagccccgccatcgccgccgccgcttcatgaggtgggcaggcgaaagctggtgaattcgttgtacagcggcaagtggggcgccgcgatcgaagggtacgtcaacaagctgacgttgatattaaatacgtctggctgcttttctacgatggaagcgcacagggttacggcgtcaaacaggtctttcttggtggcgcccgagacccacatctggtatacacccgtctcgtggtacgaagtagagcgcggcaccaccggacggatgcagtccagaacgcggttgggatcctggtgaaagaatttgaacgtggctacggcctgtggcgtgtgcggcatcgtctgcgtgatgagctgctggcccgctaacacggtgacgttgtgcaacttgagcagggcactcttgagggcctggaaagcgttgccgcacgaggcgctgatctgcagctgcacggccgtggagtcgtgcagccgcatgagacgtgatacctcttcgaagacgtacttgtatttgctggcaaaaagtggcgcgtaccgacagtcggccggcaaaatgtaggtggcgttaccgccgttggtggccacggcgggcgcagcggccgcggaggccggcgtaaacagcgtcagcggccggtggtggctggtaaggtcgatcatgggcggcgtggtgaccgtggcggtggcgggcatgacggggtttgcggcgacgggcactccggccacagcggcggccgcggcggccacggcggcacttgccgagcccacacccgccggcagtcctccgccacccatgacgccgccgggcagagcgtcgcccagacagacttccgcagtggcgggcgcgctctcagcggtcagtacggtttgccgatcgacctcgcgacgaaagctggtgaggaactcactgtgatccatggccgcagggcccgagatcccgggattctgcgggtgctgaccgagtgcggggcgagttatatggaagacgattagcttggagcggagttttgcgtccctagctgacctgcggatcagcgacgtgccatagggatagactgtgagcggcggccgcaacggcggggtcggccgccgctcgtcgtcacggggcggcgcgagggaggaggaggtggtgggtacgatcttgacgtggttgacgtcctgcccgtccgggggaatacgcaaaaaaccccgtcgcggcgctaccacgatggtgcgatgggtctttctcttgttggccggggccagggacttgcagatgcgtgtggagccgtagacgatctggacgtggtcctgggagaacatgaccatcgccgccaacgctcagcggggggacgtgttgggaacacagaggctgagggaaaactccgtagaagtcagcgaaataaagacaacacagcagccactcctctcgtctcgggccctaccactgcttgaagtagggcaccgggtgtttcttttcctcaacgggctcctccagtctcttataggaccagtcccgccggcgcgccagcatgtaggtcacgtacaaaagaataatcaccatgaacaccaggaaagccagcacgccgtaggccagcagccggtcctcgaacagcgggtcgctcttgataaacacgtaggtggtggtaaaacttcggcccgcaatctgaacgtggagacgcacgacagtatacgtgccgttgaggtagaagacaaactcgcgtaaccgttgtccgttatacgtcacgttactaatattccacggcggaatgagctggttgccctgatgcagatgcacggtgctgttggggtgatagaggctgctaccgttgagcaagcagtgttcgtgttcctgaagcagcacgcggacccgcatcgtggtggcgttcaggcgagtcccgtacacggcgtagatgggataggtgaaaaggtcccaagtggcgttgtgatggcggccccagctgaagaaagagcacgtgtactcagtggtctcctgcggcctgagtcccgagataagcagctcttgagcagtagcgttgtaggagagatgtagttttcctgtggataaaattcataagttgtttattttgttggcaggttggcgggggaggaaaaggggttgaacagaaaggtaggtgctacttaccttcattatcgggggggaaggcgctaagataccccacctgagtgaagggacccttgcagtctgtccgtgcataacaagtaactgataaaatgtctggatttttggtgttattcaacaggataactttgcaggtggcgtttagagacacttggtcgtggctgtagctggcttcgcaattcacagtatacaggtgcccctctttctgcgtcgtggctatcacggaagtggaggcggacgaggtagaggtttgtaccgtggtggtgacagcagaagtgacgttgttagaggtacttattgacgtagtagacgtgacggtggtattactaggggaagtgacggcgcttgtggtgctacttttcacccccgggtgcatgtcgcccaagagcgcaactacgagcgcgatcgccagtacggaacacatgttgccgtgtgacgagacggcgtgtggacgagctatatgtggcaggaggtcgcgtcacctcttgtgacgcctaaacgtccagctccagataaaagaggcgttaataatgaagaccacaaaaaccacttgcgtcagtatgacaatcataaaggctcggtgattgctacgcctaaagtacgcgggattatccaccagttcatcctgctgaacaaagtggatgattgacgtattggtgttactatccgtgttgttgaccatggatttgactaagaaagtcttggcgccaaaagtcccgttagagccccagcaggtgacgctgctattcacataagttcccggtgcccccgctagcatgtatttcagttggtgggtataattttttctgtcgttatccatgtcattgctgtagttgaccttgctggtgagaaagcgtgttttcaacggggcacttatcatcatccctgaggccaaaaagggcgaattgcaagctgtagtgttacaaaaaatagtcaagttagtgtcattgtattgataaatgtaagccatgcttacttcaggctcataccacccgattccaatcgcggccgccatcgttaccacgtcccatcttcccagacttaccaccgccaccactaacagcgtcacccccgcacggtacatagttaccctctcgacgtcgccggctgtcaatgacgtgcctgcgtcagtggctatgatttatagcttttgggcccaaccgcaacggatctgtcgtaatctaccttccacagggccgccgcgacgatgctgaacgacaggatcagacagacggcgtacaaaagtcctaggtcggcgtcgacgcggcaggtgcggatgtctcgcagggtgggtagatgggcgatgcacaactctttctccccccgcccgtacatcccatcttgtatcagcagccgtagcgtggcattgatggtcagcggggtaaccaaagaaatcacatagggatgtgtacaggaagtgcagtgacgggtatccgtgagatgtaagtcaccaccctcctcaccgtcatcatgaaagaccaggactcgggtgagacgacccgatgaatactggatctcccaccacagtctttggtccaacaccgagagggcgcaagagattctaagtctccctgggttgggggagcagatgtaagtcccgtatgtgcctctcgccatcagggccatacacatgagggggagaaggacaattatccgggaccacccgcacccccacatcacgagaccagagacggagatgtataaaaaaagctacttttattaaacagcattctcaccacacgttaatactgtcacggggaatcactatgtacaagagtccatgtctctctttccagtttttcacttactgagacttgttcctcaggtcctggatggctgcctcgatggccaggctcagggtgtccaggtcttcgggaggggtctcggtgggctgctcaaactgccccacggcgtaggccttcgcggccgtctcgtagataggcagcatgaacccaccctggttggtggagaagatgcgcaccatgacctgtttgggaaacttttgcatcaggggcaggcacaggttgagagcgcccaacaggtccacgggggtggcagcgtggatgatcatgttgcggtaatcggaggaacgggggcataattggtgggtgtgcaattctttgaggctccacgcggccttgacgccttcgttacaagcatcggctgtgcgctgcgccacttcgggtggatgtgtcacgggcatggtgtgctccatgaggaagggagtggagagggccaggttgcacatggtgcccaggcgacaccgcaccgcatccacctcactcttcacctcatgattgcgggtgtagataatctggatgcccttgttgttcacctgcatggttttgcaggctttgatggcctcatctaacacctggtgcatactgggaatcgtgaagggcaggttcttgtactcaagagagcgattggtgttgcggaacatgcggctcacctcgtcaatcttgacgcgaccccgccgagtctgcacgttgggtgtgcagaagggggtgttcttatctttcatgatattgcgcaccttctcgttgtccaactcggagatgcgtttgctcttcttcttgcggggtccggtgctcgccccgccgctgctctgatggccgcagctcagcagagaggaggaggccgcgccaccaaaaccgccgcgcccatggtggctcgaggtcacggatgctcctccgccactgctgcatttcatctcctcggactcactctccgagtccgaagccgaactgcaggaggaggaagacgaagaggaactatcttcatcgggccggcccaagggatcgggaagaggagggtggttcatctgggagagcgggtgcgtgggagaggtcactcgcggcgtgccgctgccggtggaaggggaagacgcggtagcaccgcgggtttcgacttcttcaccctgttcttcctcgctatcagagatcacgatacagccggcggtatcgataatcttgttgcggtactggatggtaaagtcgggctcgggcttgatgtcttcctgtttgatgaggggcagcatgataggcgcgggaggcacgggcggtttaataatcaccttgaaaggacgcgtggttttgcgcggtttcttacgcgggctgagctcgggagtagcggatgccccggggagaggagtgttagtaaccgcgacgctggtgggggtcggcttgttaagaggggcgctgctaacgctgcaagagtgggttgtcagcgtggggccggtgctactggaatcgataccggcatgattgacagcctgggcgaggatgtcacctgatggtgataagaagacacgggagacttagtacggtttcacaggcgtgacacgtttattgagtaggattacagagtataacatagagtataatatagagtatacaatagtgacgtgggatccataacagtaactgatatatatatacaatagtttactggtcagccttgcttctagtcaccatagggtgggtgctcttgcctccagaggcggtgggttcctcagcaccatcctcctcttcctctggggcaacttcctctatctcagacactggctcagacttgacagacacagtgtcctcccgctcctcctgagcaccctcctcctcttcctcatcactctgctcactttcttcctgatcactgttctcagccacaattactgaggacagagggatagtcgcgggtacaggggactctgggggtgacaccagagaatcagaggagctgacaccagcggtggccaaagtgtaggctacaatagcctcttcctcatctgactcctcggcgatggcccgtaggtcatccacactaggagagcagactctcagaggatcggcccccagaatgtactgggcaaagaccttcatgcagatctcctcaatgcggcgcttcattacactgataacctcaggcttggttatcagaggccgcttggccagcatcacactagtctcctctaagacatagcagcacagcacccgacagaactcacttaagagagagatgcccccgtacatggtcatcatacaagcgtcactagtgaccttgtactcattacacattgtttccacacatgtagtgaggatatccataaatatgtgatcaatgtgcgtgagcaccttgtctctctcctcatccaaaatcttaaatattttctgggcataagccataatctcatcaggggagcactgaggcaagttctgcagtgccgccatggcctgactgcagccattggtggtcttagggaaggctgagttcttggtaaagaactctatattcctgtagcacatatacatcatctttctcctaagttcatcctttttagcacgggccttagcctgcagtgcaccccccaacttgttagcggcgcccttgctcacatcatgcagctccttaatacaagccatccacatctcccgcttatcctcaggtacaatgtagttctcatacatgctctgcatagttagcccaatacacttcatctcctcgaaaggctcatgaaccttatctaagatatctaaggcattctgcaaacatcctcccatcatattaaaggcgccagtgaatttctcttccgtctgggtatattttttcagcatgtgctccttgattctatgccgcaccatgtccactcgaaccttaatctgtttgactgtagaggaggataacaacacatataagtatccgtcctcctgactcatttatcgctatctcgatgccccgctcacatgcaagagttaatctttactctatctgacatacacaagtaaatccacgtcccatgcaggttagtatacatcacatacatgtcaacagacttaccgagttctgccaggacatctttctcggggttctcgttgcaatcctcggtcacttgttcaaaagttttgagggattcttcggccaactctggaaacagcgggtctcccagactcagctgactgttaacctccttcctcaacatagtctgcaggaacgtcgtggccttggtcacgggtgtctcgggcctaaacacatgagaaatagagtcataagcacatgggtcacatacaggagatatgtatataacattaatacaattttattaaaaaaaaagggggggcacaaaccccgacacgtaccgtggcaccttggaggaagggccctcgtcaggattatcagggtccatctttctcttggcagaggactcttccggttttagaagctccacatcgaagacgagagtggcatgtggtgggatgatgcctgggtgcccagtggcaccataggcataatctggagatatagtcagtttggctctctgacccacactcatctgggcaaccccttcttcccagcctcggatcacctcctgcttgcctagcataaacttaaagggcttgtttctgtcccgggaggaatcgactttctttccatcttcaagcatcccggtgtagtgcaccacacaggtctggccgcgcttggggaaggtgcgcccgtctcctggggagatggtttccacctgcactcccatcgtgtcaaggacggtgactgcagaaaagacccatggaaaggaacagtctgttagtctgtcagctattatgtctggtggcgcgcgcggcagcaacgagtactgctcagactacactgccctccaccgttaacagcaccgcaacgggagttacctctgactcttatcagaacacaacaactcagctgcctgcatcttcttctgccgctgccttaagtcttccaaatgcgtcagcggtgcaagcccgctccccgagctcattttcagacacataccctaccgccacggccttgtgcggcacactggtggtggtgggcatcgtgctgtgcctaagtctggcctccactgttaggagcaaggagctgccgagcgaccatgagtcgctggaggcatgggagcagggctcggatgtagaagctccgccgctaccggagaagagcccatgtccggaacacgtacccgagattcgcgtggagatcccacgttatgtttaataaaaactgcgggcactggggacggtggtgttgtatatgtgaatttgtaaataataaatgagaccccatcctgtaaaaatacagagtccgtgtcagtctctgaaggacagtgtattggcatatagccaataaagagagttgtggcaaagagccatgttatggattagtaatggaaagtatcgtcaccaataggggagtggtcaataatggtcaataacccacacctataggctaagctataccatcacctataacatgaggaagcgggggtgtatagaccccaagccaaaaacagtatagcatgcataagaagccaagggggtgggcctatagactctataggcggtacttacgtcactcttggcacggggaatccgcgttccaatgcaccgttcccggccgcggaggctggatcggtcccggtgtcttctatggaggtcaaaacagcgtggatggcgtctccaggcgatctgacggttcactaaacgagctctgcttatatagacctcccaccgtacacgcctaccgcccatttgcgtcaatggggcggagttgttacgacattttggaaagtcccgttgattttggtgccaaaacaaactcccattgacgtcaatggggtggagacttggaaatccccgtgagtcaaaccgctatccacgcccattgatgtactgccaaaaccgcatcaccatggtaatagcgatgactaatacgtagatgtactgccaagtaggaaagtcccataaggtcatgtactgggcataatgccaggcgggccatttaccgtcattgacgtcaatagggggcgtacttggcatatgatacacttgatgtactgccaagtgggcagtttaccgtaaatactccacccattgacgtcaatggaaagtccctattggcgttactatgggaacatacgtcattattgacgtcaatgggcgggggtcgttgggcggtcagccaggcgggccatttaccgtaagttatgtaacgcggaactccatatatgggctatgaactaatgaccccgtaattgattactattaataactagtcaataatcaatgtcaacatggcggtaatgttggacatgagccaatataaatgtacatattatgatatggatacaacgtatgcaatggccaatagccaatattgatttatgctatataaccaatgaataatatggctaatggccaatattgattcaatgtatagatcgatatgcattggccatgtgccagcttgatgtcgcctctatcggcgatatagcctcatatcgtctgtcacctatatcgaaactgcgatatttgcgacacacagaatcgcccaagtcaccaaagtcgtctatcgccatcccccgtaaacgatataagcgctatcgccagatatcgcgtatgcccaaaaatcacttttggaaaaatggcgatatcagttacacagaaactcacatcggcgacattttcaatatgccatattttcaaatatcgatttttccaatatcgccatctctatcggcgataaacaccactatcgcgcgacatgaatttagtcggcgacagaaatctcaaaacgcgtatttcggacaaacacacattttattattcactgcagcatatagcccattttagcgcggcacacatccagccgtttgtgttttttaacgctctccaggtactgatccaggcccacgatccgggttatcttgtcgtattccaggttgatccatcgatagggaacgctgccagcggcgcccagcaggtactgcgccttgtcgttcactttgccgcagcgtattcgcccgtcagcttcgaggtataacctacaacacggaggggaagggggggtacaaaacgtgaaattagactttttttttaatgatgttttgtccctctgtcttactttcccataggctgtaaggccctcgaggaagagacttacggattgtagttgcagctcgtcagtttgttgtgtacgacctggcgtgtcaatgaatgggtcatggtggtgacgatcccgcgaatctcagccgttttctcgggactgtagcagacttcgccgtccggacaccgcagcctgtggattcatgaaaatctactctggcattcccgaggatcgtcgatggaacatggctatcagaaacgtcgagagacaaatccagacgcaccacagaacgcagacaatcataaaaatacgtacgcgacggtgaagcgattgcacattttgaaatcgtaacagcgttccggcgggtggttgacgtttatgaattcgcaacattcttctgcgcgcacccgcggcacgcggctgtgacccaatagcagccacaacgtcgtcaagaacggcgtcaggtctttgggactcatgacgcgcggttttcaaaattccctgcgcgcgcgacgggctcaaacgatgagattgggatgggtacagaaggtgtaagtctggttattggcctcggtgaacgtcaatcgcacctgaaaagacacgctgtagtcccggaagacgtgggcccagctctccagcttcatcacacacatctgataacgcgtgccatcgttgacgacgaagcgtagcagcttggtctgcttgggcaccatgtgcgctccaaaaatcttggcgtcttccacgctgatctgcacgtttccgtcgctcggtttcgaagccgtttggggcatccgttggaggatggtctggttgcgaccgctcagataccagatcacctttttcacccaggtggagcttctctccaccaaggtctggccttcccggttgtacagcagatacagggtctcgttgcgacactcgggacccgttgatacctgctggaaccccgagaattgcaagggggaccgtgggggcgagggatagagaaaaggacagtaaaacgtcgccgcgtcatgcggtttggaatacgtcagtttagaccatggcggggacggattctggtttgccgttagcgtcgaccacggagacgccagacagggcgttgcccaaaccgcgcacagaagcaggcagtgaaagtggtgacgaagcagaagccgcagcatattatttcccgtgacgcaggctagttggcaaagagccgcacgctgaactcgaggctccgggcgtgtggcgccagcgaaccggcggcgttgaacgtggtccttttgttggtgccgccgcgacggttctgacgtctaaagtcgctgatgagcaacgacacctcggtcacgttgattctgcaagcacaggttccaaacgtcatttcataccccatgcggttacttagccgttacccgttcgcccttaccttcccgttgtcatgcacctttagcgcgtaccctcacctcttgagcacgtcaaagttgtccaagccgtggctcgcatcgtagtggtagttcaacgtgaggtccacgagctgttccacatacttgtaacgggtttggtcgggcagcgcgcgagagcacgcgtcccagtaatgcggtactcggtaataatcgtttttttccgcggtttcccgctggcactgacccagcaccacggcgcacagacaaacagacagccacacccgacacagccgcatgttgcagactgagaaagaaagctttattatgagacatcatacacatagtataggcgaggtgatggggcggggaaagagttggaaccgaaagacaaaaaaaaaagcctagtcgtactcgggatctctgagcgagacgggttgcatggcaactttcattagtttgggaatctgccagctggtgctgttcgaaggttcttccatttccgaggcggtcagttcatcgtacaccgaaacgtagtacctgatggggtcctcctcattgtccgagaggtgagattcgatggtcaaaggcgagcctctcccataattgggattcacgaacgacgtgtccaagttgccatcctttctgaaatagatgacgttctcaggatcatgtttcatgcgctcgcgggccgcggacgcctcctcctcctcgtcccagtcccgagtttccaaccgctgataagggctcgaggaacaaaatccggcggggatctgagaacctcgtcgggaaccgctgccaaacgggctgctgccgccactgtcgtccgtgtcgtccaacaggttgacggcctcttcgtcggcgaaacgaaagcggcccgggtgcttgcaacacgaggagtaaactaccgcgatcagtaccgctatgaagctgaaaatggaggtgcctgtcacgatgtagaagaggatagccagcactttcatgatttcgtcattgcgcgcgtcgtgaacggaagattcgcgggcagtggtcatgttggtttcggttgtaggttcgctactcgtggtgctctcgacggtatttctgctgctggtgctagtagggacgtttgtgctgctggtcatatttgtagcgtcgctgaagtcgatgtgaagcagcaacccgaacgcgaccaggaccaggaatgttgcgcgaaggagaccccgcggggccggcattcttgagacgtggcgacgtggatttcttgttatgtccgcgaacgacgtgtaacgaggacgtggtttccgcaagcctctaccgacgccgcgacaccaggtaggttatcaaaacgcgagcccatatcgccgccatcattgtaatcagcaatgtgttgaggtactgcacgatgaatctgtctagtgacaccagccaaccctctgcttttgcgggcaagcgcgctttcggtgacagggtgtatcgtacgtagccgcgggtcaggcgcgcgttgtagcggtacacgcagaaatctatccacaggccaacgcccggctgtagcttcggatggtggataatagcgcggtgacgtacgccgcgtggctttagaatctccacctgtaaggccatctcctccaggtagtgggtctgactgcgacgcagcgtccagttcatgtaaaagtcggtctcgccgtgtccggccacgaagaggctgcttactaatccagtctacattgtgccatttctcagtctgattgcattttttagagttatgttgccaccaacgtatcctgttacgttgattacctcgtaactgcggtcgcatcttttatggactgtataattgaaaccatcacaagtaacggtcgtggtggtgttggtacatgtggtagtctcaacgtttgtatttgtcgttgtggatatctgtgtggttgttttcgacggttttgtagaaacggtggttgctggtgcagttgcagtagagcaatttatagattctgaagtgcttttattgctgataactgttgtactgtatgttgatgtggctgtctcagtactagtggaatagttaacggtagtactacagggacattgacaggaacaggtttgattgcagctttctgataacgcggatattagtatcgtccacataaccgtaaatcgccagtccattgcaatattagttctcgctcaatgggcattaatattcctttgaacgctgagccttacagaatgttttagtttattgttcagcttcataagatgtctgcccggaaacgtagctcaatcttcatgttctgtgtgatatcgaacaatgaattctgattcactgacggtgtcttgcaacatatggtactttttgttaaaggctcgtcgtgcaaaaaacagaactatgcaggccatacaaaccaacacgatggtccatacggtgcggcttctttgcgagctatgatagagattacgtttgtggtgatgtgtattgttagtatgttgacttcctttctctctatcttcattttcgatatcggtgttgtatctagggcaaacgaaagtagcattaatagcttcagtatgattttttggtgttactaataggtagaaattttcatcttcgtgatgtcctgtgaagtaattttctttaaaacaacgtctgctgtacctgccggaattggtgatatttagatcgtacagatgtagttctgtgttgttgcacgaacgacataagtcatggtacagtgaaggtctttcatgttgagaatgacatacagtatgagaggtaaggatgcgtaaccaataccaagattgggtatgtgcgttcttacgatgacctagatgatgtccgtgtgtggatcgattgtaatgtcgtatccaggcgactgaaagacaatcccacgtagaattaccttttatggtgacattactcccttctattcctgttgtattagtttctttgaaacgtatgattgttgtctctgtgtgacaagcgttggaagagttagtacggttgtacgtggtgtacgttgtggcgctgcaatttgtaagccatggcgtgcttataagtgcagtattagtggatacgttgtgcgaagtttcatctgacgtgatagttacggtgattgttgtgttataagatgatgtagcgtttgctgttacgttggtaaaagataatatagtgttggtatttgttgaaatcaattctgtagtggcagccgtattggatatattagcatatgatgtattgaatgtagaatatacggttgtgaaagtactcaagtcggaggtaacgttggtgatgttgccaatggttgacgcttgtgaggtgacagatgtgtgtggcgtcgttgatgtgttgttattcggagtagaaaatacgctggtcacaaaggtggtagaagcagtgttgggtgatgtgatggatgcagtattggtagtagtactgttgcatgtaactctatgcagaatatagaatattatgattgtatacgccgtatgcctgtacgtgagatggtgaggtcttcggcaggcgacacgcatcttttactgtaaatccccgtccaccgtcaacaacaaaggttccgtatctaggtccgtccgcagatgttcagcgtcctgttccccgattcgttgcgatcgcaggaagcagatgaccagcgcgccaacaaagatcatcattcccgaaacccaggcgcaatggagtgagaggccggaccactggcgttttaaatccgagataattgcccggtctgcctcttgggaatccgtaaccacaactctccctggtcccggataaaagcatcgacgcgtttccaaggctcggcagaagctacgtgggtggatgatgaggtagaaagcctcgacatcgccggtatactgatcctgcaggaggtagactcccgtatctttaaccgtgagattgtacagcgtcagattttggcgcgtgcacgcgaacgccgcaccgccctgacgcgtggtttctttataggcgtctgtaatgatacaaagtggcggcatacgacgcatgtatctgctgtagatatcataacgctgccagactacgctgtgatggctagtgttaagcctggtaaccagcgtgcgtgtacggtcctcgcaggtggcacggtagttggcgagctttaggggttttttggttggttcgacggcgttcgatgaacttccctgagttgtgaacaaaaacagcgacgtgactatgacaagcgtgaggggggtgctgtaggtctgcatggtgcaaaacacgttctcgccttccttatcagacgttgtcgtcctcgtcctcttcgtcgtctgtgcccgtcggttcgatcaacggggagttatctttctgtctggagggtcggtatggaatccgttcgtagatgttctgctttttagccgcgtgttgttccagctttttgcgtgtcaggctccgataggccagacattgatctacctcggtgcccgtgttgtttttctcctcctcgcgcgcgtaaattacaaagaagaccaccagcaggactatcagcgtagccacgaacgagcccgcgccccaggccgagtatgcgcctagcatggtaatgggttctgtgatccggcatttgcacatcgcgtggcacttgctgccattgccggtattagatgatgtgttattcggactgcacttgcacgtcaaatgggtattttctgatttcacgagacagttggtggcgactttggtttcggcgcagacggccacatagcttaccaagctgagtgccagaaagcacaccgcgtgcattacacgcggatacatattaaaacaccgtgttccacaagcaccgcacacgtcaatcctccccgcacggtcttcagcccgcccatgacatgatctccctcacgttacccttcaacaccctgtagtactctgtctcggcttccggtccccatgtcctaattataacaaaacaccgtgacactgtccatctccctgtctttttgcgccgccggtcccccccaaatcatgtctctagatgccgccggccaccaaccggaggcacggcggctattggattcggcattggtgcgccgcgtcttggcctgcatgatcatcgtcatcatgattgccattagcatctggatcctgacctacgtgctgtttctctaataagaaccccggcccctgacggtaattttcctttcttctccgtttctcctcagctgccgtacgtgatgcctcacggccatctccgacaggccctctccccgacctcctggacatgtgagggcttgttgctcctcctgggattgctggtgctcttctttcaccaccacaaccagtcggccgtggagaggcgtcgccgcgtctcgttcgtcgaggccgatcgactgccgcatgagagcgggtggtattcttccgatgacgacggagaccgggacggtgatgaggaaactggagagagccacaacagaaacagcgtgggactgtccgctgtttttagctgactggcgtgcgacctgtaaaccgttactcgggtctcaagatggtttggaagttgtgactcatcttcctgtgggtgatacccaaccggacgcgagtgttccataaaagccgggcgctccggcgagaccatgccatcctcgccttcggacgccccgctcctcttctctctcctctcctccccgctgccgcggccattgccgccgccgcccataccatcggcatgtcggccgacaaatcgcagctgtcttcgccgccgcagctgtagcagttaacgtcgccggcctccaggaggagatggcgctgtgcgtcgtctcttcgtcccgtctccctctgtggtcgtgggtggtgcgagagtacacgatgggtggctctcgtctcgggggaccacagggggaggggggtaatttattattcgtattactgtaattttgtatcgcttaatttgtttagagccgcacgcttgacaacgccttgtatagccttatttatcccgatgacttttttctccgtacaagaaatggacgtcacttgagcagacacagtttcatcgaccacgacagtctcatgatctgactacctctgacccgccaacgagaaaaccgaaaagtaaaagatgaccgcgccctcggagtccttttttccttttcaatcatgaaagcaagaggcagccgagagaatgccagtaagagacgaccatcgcagacacagtacgatactcatcttagaacgaaccagcgaataaccatcacacgtacagcagaatctcatgaactagtcaaccaacgtcataaaatcttcacacaatcgtttttgcgaacttttaggaaccagcaagtcaacaaaagactaacaaagaaaaaccatcttggaattaaaaaaagtagcatcgttaccttatgaaccagcagcattcagtatatacaccagatataatatatttattaatgtatcctctctttctcctgatgtaattttgtttttgtaaattcaattgttgaaagtctctccctgggggaattgcatatcttattgatgaagaagaaatccctgccatatgtgttgtcaaactatcattatttctctatatgggtattttttttctaagaagcaaaagactagcagcagccaaaataaacctgatgaaatctttaactgaactcccagtggtctgtgtgtatatttctgttggtggtcggttgtctgaacccgggtgggttgttcggaaacggcgggacggggaaacggatggaaacagcgtcgctatatacgtgacttttgatctaaacggacgtcgctaggctgacagtttacgaattgctaaacaagataggaacaaaacaagcggggctttgcctggtaggatttcctgtggaaacaataaccggatgtgattgtggctggtacataagctggttctggctgcaagcgcttttcactgcattaggtttggcgtttgcttttgcctgggaacgctatggctataacgggaaagaaccggtttggcaacattccattgtggggggggggtacttatagcgtgcctagctatgacgttgatatatgtggatgcggataatactcgtaatgagctaaaagcgacgactggtagtaattttaccattacgcataggaaagatccgttgacaactaagtggaaaaccgtttttggtaacaatggtgatcagtggttgtgcaacgttacgggtataggtaatgctactgtgaatagtaacgcaactatttgtgtgtcgagctgtggtcataatacgttggatttatgtaatttaaagtcgggagattctggcttcttcgatctgtctcgttggttcggtgaaaacatggatgaatacagtggtgatgtgtggcacttggaagtcagctaaatgttgtatcgcttagtgaattggtgttcttacagttttcatgtaataaactacgtgtaattcgttaaatttgtgtgtttttttgttagtattctgcgtaacggtggaataaaattgcgttgacctagttagatttcctgtgtagaacaatgaccggacgtgcttggactggtacatacgcaggggctggacgtggttaccggtcactggactcggtttcgctgtagctgtggttcaacctgaacatggctcccagagctgctaggaaccggtccagtcacattttttggtgggtggggggtactaaaaaagtgtttaatatttgggtttaatgataaaatccaggttatggatatgaggaaactgaatacctcgcagggtcgaaatcttaccacagttgatgatagaagacggttttccatcgggtgggaaacatgggataacggtggtgactaataatggtacaacggtcgtcaatacaacagcctgtgtttcaagttgttcgcatacgtcgcttgtgctttgcaatatgacgcagcagactgattcgttgtacggagtgggtcatcggttgaatgacgaagaagatggtgaactgtggagagtttcggtttcttaataatcccatacgacatgtgttcatttatatctgaattttaggatgatgactatagtataactctggggaacaaatatcatacgttaatcactttaagttacgccgttaggaaaagaaaatcagtccgaatgaagcatagtcagccgaatgatacagcaatagcttgtttacaacgtgttcttttttacattatgaacgtgccttgctttttatacacacatggagacagaggtccctcagcccttgtcacgacaactccctttttctaaaccgtatgtgctccaaaccgtatctcctcatcgtcacgtgaaataccatgggaccccttttcgtcacacacgtctttccgcttacccaacgcgtcagcccgcgctcggcagagctaccatataaaaacgcaggggtttagcagcttccccagatcgctgctgccccggcgttctccagaagccccggcgggcgaatcggccggctggtcggtcggcgctcggacggatggggagaacggcggtgacttagccgcccgtggccgggagaagacggaggagccgagatgacaacagcagtcgtggaagggtcgccaagccccggtccttctcttctgtctggtcgaatcttgttttcttttttcaaccgctctttttgtcacctttttatgtgagtttctcttccgcgtctcccggccgtaccatccacccatgcagcatgcacgcgtgtatgtatgcatcgcctctcctccgtcccgactaccatcagcagtaccactgccgccacccccagcgccaccaccgctgccgtcgccaccgcgttatccgttcctcgtaggctggtcctggggaacgggtcggcggccggtcggcttctgttttattatttttttttattttttatcttctcctttccttaatctcggattatcatttccctctcctacctaccacgaatcgcagatgataaacaagagggtaaaaagaaaaaagctacagacatttgggtacctcagctttccgataactcgaagaattcaaagtcgacgattcccaacaagagaaaacagaacaaaaacaaggtcatttttatttatcctcatcgtcaacaacaactaccgacaacaacgaaacaccaccaagaatgtcaatccgcaagggtgttcctgccccctcgacgcgcctgtcgcgatcctcatggcgaggaccgcgatctccgtataggtagatgaaattatcccgtgtccggtcctgattccccgcatgccctgcacatcctgacgcgtcggtcagcagccaaacaatcataggaaatgaaccagaagaacaaaaagatcatctctctcggtgtatagcaacaccaacaacaaccgcatcgcaacatcttcatccgcaagacggaaagaaaacaacaataatgagaatgaaatcaccacaaccaagccagatttcacgtccatgagtttttattatattattatcaaaacgaaaaacagaaaaactgtcatagataaatataaaaaaaaatagaaaccacaaacgactactagtactccaatcttagatgtatatgctcctagataagatttagtattaccataatcatcgaagaatgaaagacgacgatgattccttaccgctcctgccacccggtctgtatgtagagagagaagagagaaaacggtgaatccaagatccccgggtcggcgtcggcatgccgctgatcgcagtggccccacctcggcatgccggcgccgggcgaggaattgctcatgaaaaaaagtatctttctgtaaaaaaagaaaacaatacatgattaaccgaaaagaaaccaacaaaaagaacccgagatcagtcgatttcgatcactacgataaacacatggaagatttcttgaaaaaagaaaagagaaagagaccaccttcccggcggcggacacgctcctctccgtcgccgttctgcaccatgattcgatcaataacaacatcatcatcggagaccatcttttaatcaatcagcgttgcagtagtcgactccctggacacgaaggagtcatccatttttatcctcgcacttcttcgctctcaaagccgcctttaaagttgaaatgaaaggatggaaacatggaatacagttttaattgcacgtatcaccattttactacaaaaagaaaaaaaaacaacttacacatagtattaccttaggtttacggataagtagagtgtaggcgtttttgaaacagttcagccaatgcaatcttgtctcggcataatcactctttctgcatataatagtagtagtagatttattcacatcaacacagcgaaaaactccagcatcaaagtacacctagagacagcccttaaaatatagtttgcagcttttagatgtacttacaccaaagaagattaccgtccttacgagaaaacagatactcggatataggaatcaagacagctctgcactgaaaacacactctcctgtcacgacaccgcgccacaccagaggcgtacgcgtgacttcatcgcaacgatccatcgtgatgtccctcgcagaacctaaaaagaccaaaaaaaaatcttggaccacagttgtcgatacttgaagacaatattctcgtgagaactttgagattcgcacttgaaacctcttaggatccacaaaaacaacaacctctgtatggaaaatgcgctattttatctcagcttttctcccaaacctcggtttcttcctattcttatgttttccctagtatatttgcctccttataagaaaagaagcacaagctcggtcgcacggattattccttctgctaatctattattttgttccttttttttttctttgccttcaccctcttcactccctgtagcaacacagagtagtagacacaataaatgagaagtttgcatgcatttgtcgtgtccgtggtttgttatggcgtgtggagtgctcgggatgggtggacgtggggacggattcttgaggctacaaagatacgcggagacgtcgtggcgaggggatgggtttattggatatcggtgaagcagcgtggcggcgaaagacgcgatccctgggctggtagatccccctaccccgtctaccagggacgtttatcctttggacacgtaaatgtctcggccggcatccacgcgccacgttcaccgcgttgtgcccagcgccatgtgcgggtcgtttcggcgtgaagttggacggcgtagtttcggggattgtgaaccgtggctgagggtgtagatgggacaggaaaaagcgtgtgatctgaccgaggcgaagcatgtgggtggtgcgatgcggtggatgtggcggggtgcggcggtttccgacgtggagatgtggagatgggggtgatccggatgcgtggcaagaggcctcgagcttgggcttctcccgcggatggacgttctaactgtacacggcggccgtggcctccgagtaaaaaaaccaggtgctgacgccagacagagacgccgtcctcggaatcgtgtgcgcgaaagcctgtgccgcggcagcgtacgacgttccagtcagcgaggccgtcgcgttggcgcgccaacagtaaggtgacgacaggttggcggcccatggttccgaagcgtccccacatgcaccagcagtcggcgtcaaagtcgcttgcgctgtcggcccagtcgccaccgccgcggcggatttccgcgcgggggacggggtagccgagtgctgcgccctcgccaatgttgtgaagtggatgcgtgagttgatgttgattctctgtgggaaaatgagcgctgtcctgtgggttggtgttggggtatgcgagtagtaggggttgtgtttgatcgtagaggtgttggcgggcctgtgcgcaagcagcgtagtctgcggcgtcgagctccatctgtgtgcggtgttcttcgtcggcgtgtttgtccgaggtttggacatgcggttgtgtgttgctgtggtgtaagggtaacgtgtgttgggcgtctgggtgaagcggcgtggtgtgggtgctgtttgtgtctgtggctggcatgattgtgcggcatgtgtgtgttgtagtgggtggaggttaaataggtgaggtgggttccctggtccgcgccgcaaactgtccccgtccccaacgtaacctcccctacgcggcgcgaacagccccggccccagcgcaacccccgtccccggccccaacaccgtcccgcacaccccccgtctccgcaacaccccggcatcgccggcggccagaacgctcgaaaacccccgacaagcgcagcgccgaaacgacacaggcaaggaccgtggaacgcaccggcagcgcgccgaaacaccgtcccgaagcccggtgccgacaacaaataccgtgggacgacacgcaccggcagtgcgcaggcagcgtcggacacaacacgcttacggccctcaacactccctcgaggacccaccacgcggccccgcaccggcggtgttttgggtgtgtcggggcgcggccgggtgggtgtgtgccgggtgtgtcgcgggcgtgtgttgggtgtgtcgggggtgtgttggcagggtgtgtcagggtgtgtcgcgggcgtgtgccgggtgtgtcgtgccgggtgtgtcgcgggcgtgtggcgggtgtgccggcggggtgtggtggcggggtgtgtcggcggtgtgcgcggcctcggggtgtgcggcttcgcaggaacgagtgtgtggcctcgcggccgttatttcccccgcggtccccagggccgtcgtccctcgcccccgggcgttgcttttcgtgtgtccccagggacccatgctgccgtcccccgggaacttcctcttttccccggggaatcacacagacacagacacgcgtcttcttttcgccgtgcgcgccgcacgtcgcttttattcgccgtcgccgtcctccgcaccacacgcaactagtcgccgtccacacacgcaactccaagtttcacccccccgctaaaaacacccccccgcccctcgaggacccaccacgcggcccggaatggatgtcgggcgtccacctagatgggtgcgcgcccgggaggcggctgtgcgctccagtggtacgcgcctgccgcgcgtcttccttcgggtagctgcctttcccagtccacggccttccagactgcgtggcgccaaggcggcgccagcacgcgccgtgcacgtcgctgcctataaaagccagctgcgtgtcgcccgcggcacacgggcgacgaaggcgtccgcgtgtctaaaccgcgtgctcgctgacgcgggtttgcttcctatatagtggacgtcggaggtgtccggcgcccatggcccagcgcaacggcatgtcgccgcgccccccgccccttggtcgcggccgcggggccggagggccttcgggggttggttcctctcctccttcttcttgtgtgccgatgggagcgccgtcaacagcgggcactggtgcgagtgctgcggctacgacgacgccgggccacggcgtccaccgggtagaaccccgcgggccgccgggcgcccctccgagtagcggcaacaatagcaacttttggcacggcccggagcgcctgttgctgtctcagattccggtggagcgccaggcgctgacggagctggaataccaggccatgggcgccgtgtggcgcgcggcgtttttggccaacagcacgggccgcgccatgcgcaagtggtcgcagcgcgacgcgggcacgctgctgccgctcggacggccgtacggattctacgcgcgggtgacgccgcgcagccagatgaacggcgtgggcgcgacggacctgcgtcaactgtcgccgcgggacgcgtggatcgtactggtggctaccgtggtgcacgaggtggaccccgcagccgacccgacggtgggcgacaaggccggccatcccgagggtctgtgcgcgcaggacggactgtacctggcgctgggcgccgggttccgcgtgttcgtgtacgacctggcaaacaacacgctgatcctagcggcgcgcgacgcggacgagtggtttcggcacggcgcgggcgaggtggtgcggctgtaccgctgcaaccggctgggcgtgggcaccccgcgcgcgacgctgctgcctcagccggcgctccgacagacgttgctgcgcgccgaggaggcgacggcgctcggacgggagctgcgccggcggtgggccggcacgacggtggcgctgcagacgccgggcaggcgactgcagccgatggtactgctgggcgcgtggcaggagctggcgcagtacgagccgttcgcgtcggcgccgcaccccgcgtcgctgctgacggccgtgcgtcggcacctgaaccagcgtctgtgctgcggctggctggcgctgggcgcggtgctgcccgcgcggtggctgggctgcgcggcggggccggcgacggggacggcggcggggacgacgtcgccgccagcggcgagcggcacggagacggaggccgccggcggggacgcgccgtgcgcgatagcgggagccgtggggtccgctgtacctgtgcctccgcagccgtacggcgccgccggcgggggcgcgatttgcgtgcctaacgcggacgcgcacgcggtggtcggggcggacgcggcagcagcagcggcgccgacggtgatggtgggttcgacagcgatggcgggtccggcggcgtcggggaccgtgccgcgcgccatgctggtggtgctgctggacgagctgggcgccgtgttcgggtactgcccgctggacgggcacgtgtacccgctggcggcggagctgtcgcactttctgcgcgcgggcgtgctgggcgcgctggcgctgggacgcgagtcggcgcccgccgccgaggccgcgcggcggctgctgcccgagctggaccgcgagcagtgggagcggccgcgctgggacgcgctgcacctgcacccgcgcgccgcgctgtgggcgcgcgagccgcacgggcagtgggagttcatgtttcgcgaacaacgcggtgaccccataaatgatcccctcgcatttcgtctttcggacgctcgaactctcggtctcgacctcaccaccgtcatgacagagcgtcaaagtcaattgcccgaaaagtatatcggtttctatcagattaggaaacctccttggctcatggaacaacctccacccccatctcgccaaaccaaaccggacgctgcaacgatgcccccaccgctcagtgctcaggcaagcgtcagctacgcgctccgatacgatgacgagtcctggcgcccgctcagcacagttgacgaccacaaagcctggttggatctcgacgaatcacattgggtcctcggggacagccgacccgacgatataaaacaacgcagactgctgaaggccactcaacgacgaggcgccgaaatcgacagacccatgcctgtcgtgcctgaagaatgttacgaccaacgcttcactaccgaaggccaccaggtcatcccgttgtgcgcgtccgaacccgaggatgacgacgaagatcctacctacgacgaattgccgtcgcgcccaccccagaaacataagccgccagacaaacctccgcgcttatgcaaaacgggccccggcccacctccgctgccgccaaagcaacggcacggttccaccgacggaaaagtttctgcgccccgacagtcggagcatcataaaagacagacccgaccgccaaggccgccaccgcccaaattcggggatagaaccgcggcccatctctcgcaaaatatgcgggacatgtacctcgatatgtgtacatcttcgggccacaggccacggccgccagcacctccgcggccgaaaaaatgtcaaacacacgcccctcaccacgttcatcattgaaagtctctccagtccatatgttgtcaggacgtgctgtcgttctccgcttgctgcgaagcccgttcttccgagtcgtgtcgctgcgtccagcgtcgcgcccaagatgggaatttgggtcttttcacgcgtagcctcctccaccacggctgctgatcgccgtcactaaggaccgacacggaggatgacgaggagcttctccccgactccgcggtccgcgaccggctacgtagcgcgtgtccctgccagtctccgcagttacaccacacgtcgtgagcagcgtgcacctgctgccgccactgggcctcggcgtgctcaggccacccgccggagcccggtctgagctccgacgcaggatgcgcgtactcaacgtgcgccttccagtccatacagcaacaccataggtcgtgcgagtcgtcggctacccgccgccaggccagttcccgcatgggaaggctggacacgccgaccgagaggtcaccgagcccggacgccatctcttcttcctctccgtcgctgtcattaagcagccaggtcacctcctccgctccgcggtccgccggtctcgacggaccgcgccgccgtcggcaacacggaaaacagcacgccagcccgagccgctaaggccgcatgcccctgccgcccaactgaacacgcataccccgctcaactgcgttttgccacccctgtcagtgctctcgctcgagcaccaccccgcatctcccaacctttttccaataaacgaaaccgacatgacacacgtaatgggtactcgtggctagatttattgaaataaaccgcgatcccgggcgtctcagcacacgaaaaaccgcatccacatcatagacaagttacagtccacagtcacatacacgataaacaataccaacagggtaatgtttatggagtaaaacactattgtccaggccacatgcgtgtatgacttccgcaccatcccgtactgcatgttccacatgtacgcgctagacgtgtaatccactcgcagttcggggacgcaacgcagccagatcacatccccttgcagtaccagacgcagggctagcgtctcgaagatcggcatcacatctaagttccgcacgttccactttaacgactccccgggaacgaactccacgtcgtcggcgtgtacgtacaggttctctcccacgccgccataatcggccttcggatcgaagacgaaccgactcatgttgcccacgatgctcccccgagcaaacaacttgccgttgtcaatgtagcaccggttgtcctcgatttgaaaccagggatgcttggccgtggacttccagggccggagcgcgtcttccccggctttagtgattccatcgggcaggcggatcaagggacccatggaggtccaaagacccacccaggctttccagagattgttcatggtgaaacagcgtgtggactgtacgctctttcccaatttatatcccagagtagtgacgtgagcccagccacctcccagattcctgacgttttggttgtctttcctgccaattcctcccgtaaacttatgattatcctagcccattcccgataaaaatacacggagacagtagatagagttacgaataaaccggtttatttattcaagtgtctcaggagattattgaacgagcgtggataccacgccgtcgtcagttcatggtggcattgagcagccatagcaccagagtcccggcgcccggtatcagacacgctgacctaccgggcgccttcgagtccgtaccccgcggcctgggtgttagagtccgtaccttgcagcccaggtaggtttcaggtaccagctggttcgtacctgttaaataaatcgcagacgggcgctcacccctacggtcaggagcacaagaacaaccagagagaacagatatacgagcagggttctgaacagcagaccccaattgtcgtctctcatgcttcgctgaaggtaccagttgatggtctgagagctatagtccatcctcacctgaggaacacacgcggcatatttcttggggtctccccacctcgtagacaacgtgatgtccaccatatccacggtgtgcgtcaccgggtgcccaccgatgttccactcgaaataggctccgcgctcatcatggtggtactgctcaccggacacctgcagtctgtccatgtaagattgagagacgatacccacgttcacaaagtgtttctcggtgaagttgcccgacatcctccccttgaagtacagcatgcccatatggaaccagcattggttctcctccactcgaaagtgggccgatctgatctccgataccaccacatccaggggccggggcaccgagtccgcgagtctcaggaacaagacggccaggatcgcgagcaccaacaccggcttcatggctccgaaggtccgctgctcggctccgctcaccgctccggtctggctgcagcagtgcttcgctgagaagtagcgtgtggactgaacggtgtttttgaatatatagcgtttcttggtgacgttgtttcccctacgtagtaggcaactacgtgccaaaagaggcgttacggtactttccgtactgggatttccaaaccgggactttccacacggcggtttcaacaccgggacttttcacacggtgatttcggcaccgggactttccgcacggcggtttcgccaccgctgacgttctcatcgccgcccacgtcaacggtggcgacaccgtactttcccatgcggtttataaacgtcaagagtcacgtcagtcgcccacccccattacacggcgatatcccgatagggcatgaggggacccgggtgtcgcgacatgtcgacgacaggtgcggattagtggtcgtgtcgcgacatggacgtgcagggggatgtctgtcgcgatagagttgatgtgacagcccgctacacctctctgtcgcgacatgcatacacaacgggccggcttgtcggcgattgtcgcgacatatcgttatcagttagcgaccggagttgtctatcgcgacatatcgtcgactatcgcgacagaaaaaataccgttcgtagagaatgccgtgttgaaggaacgcgcttttattgagacgataaaacagcatcaggagccacaacgtcgaatcccacgtccagtcgattcgtatgttatgctgcacagcaatgctagaataacaaccagcagggtaatcccgcaacataaatacaaagtcacagcgaagaatccgtgtcgttctatcaagcgaaacgcgttccaaacggccccgtcacagacgcagttattcataagcgttaacaaccggtggctaggatgaatatccaaatcacagggcagtagccgacggactcgttgacaggtcagcctaccctcaaggttcctatcgttcggacgggatttgtgcgttttaggcctctttttcgccgcctgcaagcattggtgcgcaaagtcctcacccagctgtttccagctatcatctgcatctgtgcagtcccctgtatcgttgtaacaaacgggtctgtgcgacttcgttctcggaacacaagcttgttgtcgcggagacagagagagaagggttttcgggtcacgcgaagaccgctcaccgggggtcggcaacgcacacatcaacagaaaaccgagacgaatcaagagatccatagtgaaggagtgatatcgacgtgcttacgaaacggcgattatatatgttctcaacaataccgccctacgttgtatgatgtaacgtgtgacgtgagtctgatccaacactgaacgctttcgtcgtgtttttcatgcagcttttacagaccatgacaagcctgacgagagcgttcatcggggcatgaagtacgcattacacaaactccatatatttgttacgatagaatacggaacggaggaggctttcgccacacctatcctgaaagcgttgcattctttatgataggtgtgacgatgtctttaccattcccacggctgctttgcgtgatgatgacattcatcatgtatttccattcacacataccttttgtgcatacggtttatatatgaccatccacgcttataacgaacctaacagtttattagcccttgacaggataggtcaaaagattatatgtaggttttccggtaaaccgaattgtgatatttctctgcaggaaatagaacagcctggtacctataaaacggacaatgcagtactgtagcagcgtaaccaagtaggtccacatgaacacgtacaaaattatggtaagccatcgtttttcataccacagcctgtagctgtcgtacatgaatgaggacggtcgaggaacccagggtagttgtaattgggggcgacattcgtactgtccagaagacaattgcacgggtttcagtgagatgagtactttagcgatgtcggcgggggcgctacgtttcaccgtgacggtgagaacttgaccgtcgttttgtatttcatgaggcacgttatacaagccactggtatcatgaaggatgacctctgatgcgatgtgaggattaaattgtccctcaaaccgccaaacgctggtcatgtttccaccgtcaattacgcagctgacggtgtgagataccacgatgttggacttaggtttgggggctaattgcctttttacaaattcccttctgtattgcaggtcctgctgccactgcttttccgtgcggaaagtcgccatgtcttccacacgtgtggcgacgatagacgccaccaaggtagctaccagaagcagctggatccgcatggcattaccgtatgtcaattagaaagttgagcggacacggttatcgttcctggcggatataagtatataaacgcgagttagcctttcccgtccgttttgtacacccgttccccacacaaatgacgaatacgacctttttttttataaaaataaaccacgtgtattatataaaaacatttacatagaaaagagacacacggatcaacataaggacttttcacacttttggggtacacaggcgtgccaccgcagatagtaagcgctggatacacggtacacagtcctggccagcacgtatcccaacagcagcaccatcgccatacagatggcgatcacgaccccgagctctaagtgtctgtattcatagtgtagtcgccgcaggttatccactgaattcccgtaactgaaataacgtatatggtaccgaggctggcaccacatgggtttgcatttggtgcacggcaccaaatgcagagtgagatggtccaagtccgtgggcacccactggcgcaaacggaatacggcttcggtggtctccacgaggcactccggggcgtgcagacggccccactttcgtccgcgacggcccgaccagccgacccgagccactatccctttctcgggatagaacgtaccctgtacacgccacacagcgtccaacacgccgtccttgacgacgcagctggcctgatagctggacacgttgttaagcggcggaaagcgaaactgacgtgccggcggagccacatagttcggttcaccgtgttgtcgcggttcgtcctccctatagtaatagtagtcgtcgtcctcataggggttgccggcgtgagccagcgttacccaacagcagcccaggccgacgaggaggcgcagccaccgcctcatggcggcttcgccagtcaatcgtctttagcctcttcttcccgtgaggtccttccggtggcgcggtgccgacctcggacccagggacgtatccacctcaggtacacacagcaggctacctggacaccgaagctgaacaaggctacgtgtttcacaaactgcaccagtaccacatagaggaatgtcaggtagcgtctctccgcaaacagccgttccaagtctgagggcgttacccgcagcggcaaccagggcagcctggacgccggccggcaatggagcacgctccggttacaggcactgcaggggtaaacggttaacatcacgtaagagagtcgtgcgtccacctgtgggagctcagtttcgtaacgtagagccccgtcattttccagctggggtgcgccgaccttgaaatgggtcgcgctccgctcgttaccccaggtgccgtaggctctcggggccgtatcggagaagttgccacgcacaagccaggcggccacgagtaccccgtgctggacgtaacattcggacacggaactggagacacggtagccggacacgtccccaaacccgcgagggtactggggcagacggacggacttgctatttgacaacggacagatacgagacgacgaggacgcagacgactcgtcgctggaccacgacaaccggagcgactccttggagcggctcgagagtacacttactgcgatcagacaccagtgccagaagaaggaacaggtggacggggaccacaggatcatagccgccggcaccgcggccggccgcaggaagccgcccggcgcgtcgtctgtgtgcgggagccgaaacaccgtgcctctttatatcgtcccgacgtgacgcgagtattacgtgtcaggggaaacccccgtcacgacgaacgtgatttgtaagtgacgcggggtgctgacggggttcggcccgagaggtgacggagcgcctcacgtcagtatgatgtccgatccgcgtcagccccgacgtggttgtggtcaccgaaacccacgtttatatggacgttgagagcagcgcctgaccacatgattcatcataccatttctcggaatcgggcccatgccgggaaagcacattccttttcagtaaacaacaatgacatcataacaaatcattttattcgcgaggtggataataaccgcatatcaggaggagggatcgggtgatgacgcaggccccgcagaacagtccgaaataaatttttagtattgccccatagtcgcctagataccagaggtacgttaagttcatcaaaacgcccatcggcgtcccggaatcgtataccgggcacacgaagcgttcataacaatcccgggaggcgagtgttagggtagcagagtagtttcggggtcggtttccttccggcgacgacagttccgtgggcagcagaatgtacagcgcctcggtagctgtcgcggtgccttccacgaggatgggctgccggtgcctttcgtgattttccccgtcgtgtagccaagccgaggcccgcaaagtcttaggcgaggggaattgtccatagagtttcaccgcacccttcagtacatggttctgaataacacagccgcacgtgaagtaggtaggttctctcgtctcctccgtggctgccgccaccactcccagccaccacaacaggcagatcgccagagggttccggaggcttccccggcgtagcatggttttgggttaaagcaaaaagtctggtgagtcgtttccgagcgactcgagatgcactccgcttcagtctatatatcaccactggtccgaaaacatccagggaaaatgtcggtgcagccaacctttcacatacagcccccaaaacacttgaatcactgccaccatcatcagcgtatactgcgccgacttaatcgtgagcgcgtagtacgccattagacggcgatcttcgaacaatagtcgttcgatgtcctctaacgagctccacaggggaacccaaggcacgaggcaccggggttcgcactctacataataagtttggcattggtggcagggggaaaagtagaacaacacgagttttgtgcgttggggaacacgatagtcccggagccagtagcgttttgcgacgaggctttcggagacgtcctccaccggcgtcggcactcgatccgcgtagccctccagcgtctggtagtacacccggggtgtcggcgtgggcacggacaggttcccgcgcagggtccacagagcctccagtcgaccgcccgatcggagcacgcagcgcgcctcggaatactctactcggtactccgaaacatcggacagaggcggtaacggctccgtctccaccaagggcggaggttcatcgaaaagagtcaaggataattcaggcatactacccgcgaccggggcccagagggctagaataagcattacaaggttcattctgtcttacaagggaaggctgttaccctgtctagactcaaaagctgtaaggctgtcttatagcatgtagtcttgcacgtcacggggaacagggtggtgatctagtgacgtcgggagaacacggtgttttagggtgcgggggacaaaggacagtacgacagattaggtgatagaaacgtttttttttatttatgaaaaagccagtgtgccgtgcggcctagggccccggcgtagtttggataccagatgggggccgtcaggggtactaccacgagcagaaacataatgacttggtccatgtatagcagcatagcggtgcgcagcaggtcgccgtccgtgtagcaatttgacggtgagcgataaagcaccgttaatgtgtcgcggataagcacgatcttgaggccgtagatgaagctcacagtcagtgctaaaatgatgcgttggtatggttcccaggactgcacggcgatgaagagccagagtatgggaagcatgaagcttagcaaacagaggatggctaaccgtcgttgcatgttccaggccatgagccaggctaggcccgtacaccagacgcagagcatggatgacaggacataggcctggattaccacggtgcgatcgaaacacagcccgatggtggacacggatatcgtagtgagggtggtatataccatgaccagcatcagggtcccgggtcggcgccgacgttccagccagtacgcgtggcaacgcagagcgcagggtagcagtgtgctccagaagggcaatgtatcgcgcaggtagggggccgtcacgcgccacggtatgagcatgaaaaggatggtagtggctatggtggcgctggtctggaacacgacagtgccgtagagacgtaccatccagagaaagtgttgaacgctccgcagggtgtcttcatctttggtgattacggtgactcgacggatcggcggtggtgacggcggcgacacgggtgggggtttctctttcttatggccgagtggctcgccttggtgaaactggatctgtaccatgacgggtgctcgacgaacagtcgtgggggctttaggtacccggcaagttttatagagaaagggggacgatgggtggtggctacgagccaccgccaccttcgcaatacgaggatctgaaggcggcaaagacggtcgtccagggcaggcgccagaggttgggactgagcacgatcagcgtgattttaaacatggtcaccagtcctacgtagatcagcagcgagccgcgtaacgtctgagcagccggcagttcgtcgcggatgtaacgcgtgccgtagaaagtcacggtcatcataaggaagacgatggcgccgtagccgtagagtagaatacgctgatgatggaacacggtctggtcgccgataacccagagcgtgatgaaaaaaacgctggtgagtacccgtgagcatatgagctcccaacgcttagcgcgaaagctgtccccaaccatgacagcgccggtgcaagctatccacagcgtgaggaccagtgtgtagtcgatgaggatggcgggcaggtcggagcaccaggtgtagaaaaccgtggtaacggagaggaggcctacgtagcccatggtcaataccacgtcgtcggggtgcctttcgccctgtatcaagaccaaacaccagagaagggagggggcaaaaaccagcagcagaggggaagattcatgttgacatatgttgtgggaatcggggatacccagccaaatcattccgcagaaagccgtactgatggcgatgtgaaagaccactagggcgtagacccggacgaggacagcaaaacggcgcagccacataaggccgtggtgcagctgcaggagggaagcccattgcggcgaatgtagcgacggtagcggcgggtccatgaggcgggtgatgcgcccgagtgaacgggtgagcgtctcggtggagtcttcttataaaccagcggagctcaggcagccttgctctggaacgtcgcagtggtggtgttgaggatgacgctgagcgtgccgttgtcaatcaggtaatgatgataggtgccgagcttggccaggtagctgaacatttggtcccagcgtgccgaccacaccacgggcgtgagcatcaggagtgtggtgtgatagattagtgtttcggtggcgtaaagtatcagcgagctgcggatgacgtggctcacgggcattttggtggcgatgtagcgcacgtcttggaaaaggacggccaggatgcagcccacgaacacggtgtagagacacagcaaagtcttatgtaaccaggtgtaagtagaagccaggacgctgaccatcaccgtcaaaagtgtggaggtaaaaagcgcgtcacgccacacggagctgagacggtgctcccaagccacgccgttgcaggccacgaacaacgtccacgttaggatgaggctagaaatgccgatgggcgctgtggcgcacaggttgagcccggcggtggtgaacgagagaagcgccacatacagcgcaaacaccaggccgttgctggggtgtctgtgatcggtgagctccagcgcgcccagaaccaatactggtgtgcagctaagcaatagcggcgagggatcgtcgctgcacttgtagcccagcgaggggtaacccagccaaaccagcgcgctaatgagtacgctgaaagcggtttccagcgtcagcaatccgtagacacgcatgacaatcgcggtccgccgtagccaacacacggcatcttcggaaactgtggacgctgtttccgaataccgggaggagatcgtgcttccctcttccaaggatcggaaagtagcgtccgtcgtttccgcggacgcggcttccctggtacgctccgtttccgacgacgcggtttcccgctgcgtggaaactgtctccatgtcgggaccgcagcgcccggcggcgtatccgcaaggtctcgaagctacagcttgtcagaggaaaagtaggtttgcaaaaaggtgcgcagggtcatgattctcagcaccatcagcagagtgaaaaccagactgagaaacaccttgacggccgccaaaagcgcgcgttccagcggcgtctcgtagcgtacagccagggccgcttcgtggaaatgcgagacggctagacaggtaatgagcacgctgaaggacaagacgatcttaaagcaccaggaccaaccacgcctcaagatgaccaccacgattgccgtgaaggtcaacgtgatcaaagcatggacgaccacgatctgacggcggacggtacgttcgggagccaacaacgctacgccggtgcagctgagaaaggccagtaaggtgaacaacgcggccgagatgaccaacgtaccgtccaggcagagacatatcacgatcaacggcggcacgtgaagcagcgtgtaaaagagcagaacgccgatattgctgggatgcgatgtttcgtaacagtgaatgaagatcactgacgtgacgggtatgacaaagacgaggctgggcgaggactccgtgagacacagacgagaatggtgaaaccacgtcgcgggcgccgcgtagcagaaggcgctcaacaacgcggtcaagccggccagctgccaacccacggcgccataggtgtgcagcgccacgcggcaacagtcgacccaagccagactgcgggtcgccagccgggtctcttggatcccggggggcacgtagatgaccgtgccatcggtgggtacttgaaaccctttttctcttctcatggtgcgctgcgttctctggaaacggctgctctgtccgaaaaccagttccgaacgaaaatctagggcgagagggtggacaacggcgtcgacgacgaagcatgggacaggtcgttcggcgttaacgtcatcgcgtcggacgacggtagttctaagagacgtagatcgctcagcaggtcctgacagttgcggattcgcaagatcagaaaaaaaagggaaatgaacgtaataaagagctgtagcgacgtatgcgccacatcgcgtggcataagaacgtgacggacgaaaaggacctgctgcgaaaagtgaccggcgaagataaggcccaccgtgctgtagaagcccaaaagcagccgcaggggccaagtccagggccgcgtgaagacgatgagaacgttgaccagaaagaccacgacccagacgccgttgatgagggtaaattgatcggacagggtgcagttgtcgcgacagatgaagactacttccgcgcagagcaaggtgatgaccaacgtgagcacaaacgacgtcaacacctcgcggggctcctggcaggcacacgtgacacctagcgccgggatgtgcgccaggaggccggcgagtaatagcaccagctgtcggaacggacgacggcagcgcgggtgccggtttcgctgagcgagaaccggtcgctcatagcggaaatacacgaagagcgcggaggccacaggcaccaggaggagcacctcgggcgcccagacaacgtgacaaggaaagcccggacgcgacttgagagtcgctgtagggaagaccagagagaagctacccaagacggccaccgccgcggagatttggaagaggagcaagccggcgattcggacgacaacctcgaagcgatgcacccagcccagcacggccaccacggccgcttcatcatagtcgtcgttgttgccgctgtcgaacagccgccgaaacacgatctgtcgctgggtcgcggtgggaaagcgcagacccatgacagccggaggctatatgaccgcgcgtctaagacgcgagatccgtggggggacttttagatgtttgggcggcccgcggttctaacaggcttgattggtggagacggccggcgcggcgggtgggggaaacgacgagtttttccgttacgccatggttcgcgtgaggtttctctgtacctcccgcaaaaggtcacagcccgaaatggaggccgcgttggtggccccggtggcgcgtgacgataaccaggtcatccaagcgatgagtttgtctaatgagtcctcggtggtgaagaggatgagaatgagcaggtacaggtacaccaggttctcatagagacacaaggtgagcaggtcagcctcggaccacgcgatctcaaacaggcgcgtggtgtcaaagaccgtgacgaccagcatgaagctgagcgccatggcgtaatagcccaaaaaaagtttgtgccccaacggtacgggctgcaggtaaagtgcgatcaagaacgcgataacgccgatcacaaacagcgtgacgatgacctgccatcgacggtgattatggccggctagacccgtgacgcagctgcagaggctaaaaagcacgcaagccaagaggcccgagaaggtcactagcgtagaggaggagcaggcgctggccacgatcaccgaaagcgtcgtgagcacgctataaatggtgagcaggccagggctcggtggcgacgtgaacgatccttcatcgcgtttgccgtgcagcagggccaaacagatggtgggcaccatcaaacttaagggcggcataaagccggtgcaacagagaaagacggtgcctttaagatgcggaaaagccagcaccaggcccagacagagcaagaaggtgcaggtgccctgcacggccacggtgctgtagacccgcatacaaagtaaaaagcgacgtacgtcgttcgtcgacacggaggaaatcataatgactccgcgcgagggtcgcgggggtgggggcgcccaggccgtcccggtggcctctgagttcggagacatgacggcggtggcgatcaaaaggcgcgtatgagaaaccgtttatagagtgtaatagaatcaccgtcattcccacacggcgttcccccataaagtcacgtaacactcgagtaagcgtgaaaaagctttattgttgaataaaaaacacgagtacaacaccgagttgcggtgtcctgtctgtctactgggtggggaaggttcatcgtctgtctctagagggaaggtggggaatgtctaagcgagcgggagcgtgtcatctcccccatctttttacaacaagctgaggagactcacgccgtcgatgcgtccgccgtgtttctcggcgtactgctgcacccagacgtggccgctaaatatggcgacgctcatgtttaggagactcatgacgatggtgtacaacacgacgctgacacagacgctgtttttagacaacgttccacgctggtagatgagatccagggtctcgtaaataagcacggccgaagcggcggtcaccaccaggacgtagagtccgctgtagatcttgctgacccacagcacgggcgaaaagtaaagcaataggtaaaagacgatgacggaccagccgtagccaatcccgatgactttccagcgcgtgggattgttgccggccaggtaggtgagaccgctgcagagaacgaaaaagaccatcaccagggcaaacgacagaccgatgacgcgcctttctccgcaaaagcccgtgcacacggtgatgccggtgttgatcagcaagcacgccaccgtgagatgagcaaaattggtggtgtgtgggcgaaactcggcgaaaccgcgtagcatagccagcgtggacacgggtacgatggaggatagggctggcactatgccgttggcgcactgtccctgcacatcggggaaggcgagccaagccagcaagcagaccgtgagggtacaagccagctgccacacgagcccgtgatagacctccatgagcagcttaaagcgtttcaaccattggaagagctgctgttcggccaccagcgcgtggctgcgatggagcggcacgatggtgaccgtcggcgactcatggtgttcggaaaccgaggcggtgtcgcccatgctgccgcttacgaccgctgtcggtctaaggtaggcgtcgatgaaacagtccgtcttatcagcacccggttaccgcggatttgattgacgtcacgagtgtggtcaaaccgtggcggcaccctgtatccgacccgtcgtcatgggctccacaaccagagcctcagaagatggtacatgccgatgaataaagccacattttcgacatagaggcgtagcgagggctgaaaactctccgggaaagaactctgacaggtgatcagggacagatcgtgaattagcatcagcgtcaccgtcaacagcgtcgtcgcgtgtaaaccgagaaagaacggggccgcggcccgcagcagccaaagtcccagcgccgtagcgcagagcagagacaggaccgacggtagccacagccgccggagagacgcgccaggatcgcaacccaaaagcgaggcccccaggcagctgagatctaccgccagggcgagaagagccgcgccgacaaaggcctgcggcgacggctggcacatcagcaaggtcagaaaggctagcgcgtgcggcaggcagtaagccaacaggagtgggagtttgcggggacaacggtcgatcgacggaccgcgtagcagcaggaacaggcagccgacgggcacgacgaggctgagatgagaaagcggcggtgggtcgtcgtcccgtccccgctcgcatagctcggccaccggtggcggcatgagccaccagctgagcacgctgagggcgacggtggcggtaagctggaaggcgacgaggacggaggcgcgcagccataccgccagcctctctaggtaggggactacctcctcgacggtccattctagcgggacgacatgaagcatggcgacaagcgcggctgctgtgaaaacgggcacggttttataggcattaggacttccccgtcgtactggcggctgtcaaagtcccgttgtccaaaggcgcgccgtccgaaagactaatccaacggggacccgagagcatgagcaacaacgtgagaaagatggccatgctgtccaggtagagacagacggcgtgacggatgcattggttaggtgggcagaaaaagatgaccataagactgtcgtaggccagaatacccaaaaagaagctgatagagaaggcgcacaacgtcaccactatcttctgcagccaatcggcgtcgcttagcagagcgagcgtgaggaacgaaagcagcattaccacgtagacgcagctgatgcatttccagcgacgtcggtcacggccacctagaaacgccagccccgtaaaggagataaacaacgccagggtcatcacgtaggaacctactagtacgcggctttcagagcacatttggaagatggccgccgtcaggctgttggccaacagatagatgaaaagcaccgtggcgttactagggtgttcgttgcccaacgtgtacgtgatgaacatgcagacgatgggcacgagcacggtgagaaagaagctgtagttctcgacgcaaaagttgcggttttgtgggaaccccaaccaaaaaacgcttcccaagccgaagctgaaagccagctgaaagatgaagatggcgtacacgcgcagccatacggtgaactttttgaaccactcgagagcctccatgcgggagagcagcagcgcgttagcctcctgcgcctgcatggtggcgacggtctcggcacaaagccgctgcggcgcacctacccttctcttatacacaagcgagcgagtggggcacggtgacgtggtcacgccgcggacacgtcgattaggagacgaactggggcgacgccgctgctgtggcagcgaccgtcgtctgagcagtgtgggcgctgccgggctcggagggcatgaagtagagcacggagacaaagaggtacatgaggtccatgtacaagcagagcgcgcccgggatataactctcatactcgatgtcgtgcaggatgtcctgcgtatcgcacaccaccgaggtcacgatgacggccaaaccggctatcatcaccaggatctcacttaccgcctcgggaaaaagagaaaatacggcgaacagtaagagaatcagcgtggatgcgcccgtcaatagggaacgctgtaattccacgtcgcgggcaaacagatacgtagcgagcgtgaggaaacaaaatagcgtcactgtggccaccatggcataaatgactgaacgatgactaaagtggaagcctgacgccgtgacagccacgctggtaagcaacgtgtacgtcagtaagatccatacgtttttgggaaagttgggctcggcccaacgcaacagacctaggcacacgatggagatcattaagcaagacagcgtcagacgcacgctggaaaagagctgctccaaccggtgcggcaacaccagccagcaaaaggcgcagacgctcataaggatgaggcattgcacccagataaggatgtagatgcgcagcaggaagaccgaccgggctatctggacctgaccgcggagcgacatggcggcaacgccggcggttatcgccgagattcgtctaaatacacgaagcgaactagaaaacgcacacacgtgatttgcaaaaagaaagcagctgccggcttattattttattaaaaatttatctgtgcagaatcataagtttatgatgaataaaaacggggaaagggaatctgcttttagggacccgggtctggtccgtcgtctcccatctggtcgggttcggggatggggacctgtttcagcgtgtgtccgcgggcgtgcatggcttttgctcgccggccgcgctgtaaccaggcctctttctctgtggtcggcgagtcttccgacgggtagggagcctgggagtccatcgcttcaggcccaccgctcgttccctcgaccgtcgtgtcgtcctcgttttcgctattacacggggtttctggagtatcgcctatacggttggcgattctccgggggcggccgctctcgtcctcgtcgctgctatcgccgcccggtaattcgacgccgcattcgttgtacggaacgcggcacatgggcggcggaaagaacttgggcatgcgaaagcagcgttgtccatccacggtctgcgtggtttcatcgttatcctcccataatcccccctgtagcgccggcagcgtttcgacgctgtgagaggggaaggcccagttctggttgtcttgcagcgcgcccgtgggcagtaggtccgtgcggccccatgcgctgctgttgttgggtaccttgtcagtgccgcgagtaggtcgcagaaaccagtccagagcgctctctagctgcgagcgtgtgatggtgcccagtgcgccgtgccagcgcagcacgtctcttttcagcgtgtggtgacagacgggcagctcctccaaccgacactcgccgcgcaatccgcggtcgaagcggcagagaccacgcagtttaagcagaccgcacttgagaaacatgtgaaaattatcggcaatgcgatataggtccgagtcctcgatcttgtgtaggtagaccacgccaaacttgtcgagcagcaccaggccgctgggcacaaaaggcccgtaggccaggtaatagcccacgaggccgacgacgtaccactcgcagcacaagcgttgacgaataaagttcagaagatcgcgaaagtccgcggccggcatgtggtcaaaaggccggcaggcgcgcaggccctcgatggagcccagcatgagcaacggctccacctcggtgcgacccggcgtgcggatgaccaggttgagaccgctcatttcgcgggccgtcttggccacggccgcagcgtcagtggggtcggtgcagaggaatttttgcacatgatagcgcggttcggtggtggcgaacggcgtttgtgggtgccgatacacatattcgcaccagagtaggccgttcttggaaaaggctttgatatcactggccacctcgtagagcccgtcggtctcccagtcgtagacgtagacggtgccgtaatgacttagcatgagcacgcagggcagttcctgcgcctgcttggtgtttcgtgttagatcgctgtcgggtggacgcacggctagtacaccgacggcttccagggtgtcatcgcagcagagatagtcggcggccagagaacgtgcgtaaatctgcgggatggcggcctgttcgcgcatcactaggaaccagttggcggggttgcgcagtgctacggtggttccttggtggcgttgcacgtaggttctcagcgccggaggatcgtactggcgcagatagaggccttgcagcatcgataacgtcttttgaaagacggtgtttctaaattgaaaaacgccgtagtcgcagcggatagcatcttcgcagcgctcgtcgcgctgtcggagataggtgccccaggcttcggcggcggctttggtgagtagggacatgccggcggagccgtctcgacagcgagtcggataaagcgcgctgcgcgaaagcttaatataggagcagcgtcagacgaatcgcggctggtggcccggggggtgggacgcgccgcctacacaaagtgctcccgaaaatcgaaactcttgacccactccggagacaaatccgtattcagattgatgcgtcgagcttccacttcggcttccgaaacctcggcctccgtccggtaggcgttaacaatacgctgacccaggtgccaacgctctttctctgccaaacgccgttgctcaaaccattcgtctacgtccttgaggtcaaagacagtgtcctcctcaaggtcaaagcctaggtcttcccactcgtcgtcatcgctctcgtggccggcggccatacgcgcggcaaccgcgtcttcccctcctcttctttcaacgttgggtaccacgttgttttcttcgggttccataggttctgcgccgctgtcgtcatcatcctctccctgctcctcatcgtccgccaaggcgtcgtggattacctccaggttctgattgtcgggtacgacgtggttatcttcgtcgtcgtcgcgtggcatgggcggcggccgacggcggacgaccggcatggcgcggccgtcgtttccttcgtcttcctcttcaccgtctcccaaggaacgcggtcgacgacgttccgcgaagtcgccgcggaccacgcgcgcctgccaaatggtaaacgcgtcccaaccgtcccagttattgagcatttcggcgcgaaaacggtcgcctcgacagagccagcgaaactgccgcgcgtagtcgcggtctacgccgctgtcgaacatggtaaagtgcagacgcgccgcctcgcccatgtgtacgcagcctccgttgcgttccagcctggccgcgcgccgtagaccgtgttcgtagcggcgacgcacgtacaccttcatgaggccggcgcgaaaaagttcctctaggctgtcggccagccggtagatttcaccggctagacgctgcaggggcggcgagcggtccagatgcgacttgacaatcaccacgtaaaaacgacagaaacggtcgaagatgatgaggaaggacgtgtcaaaaaaaccaccggcgcggtaagagcccacggcacccagcaggtaccagcggcaacgcagttgcagcgtgacgtacatttcgcactcggccaagcgggcggctggcgctacctcgaagggccagcagtccgtcaagcagccgaaactggtcaggagtttcaacgttttggcatggcgtccaggtgtatgaaagttcacgtcgcgtccgtggtgttcgccaacgcaggcggccaacgcgtcggcgtcatgaccgtgacgcagcagcatcgctaccacgtcgtgcggtacccgcgtagcaaatggcgtctgtggctgacggtatacggcttcggtgtacatcataccgtaacgcgccagctcgtccagatgacgcgcgcacagcagcagaatctcttgcgagggttcgtagatgtagaggcgcgtaccgccacccatgcagagcaccagctccgtctcttcgtagtgatcttccaccatgatcacgcacttgcctagcacgataaggcgttcggggcaacaaatcacgtcgtccagcagctggtcgcgtagctccggcatggtgctgccgggccgtacctgcaggaaccagttgtgcggaatgccgagcgacagcacctggtcgacgtggttacggacccagtcgcgaagcacgtcggcgctgtactggcactcgaagatgccctgaaagtcgcccatgacccgcagaaaagtttcgtagcgcgtgtggcaatagaggaattcatcgtttcgcgtaaacgtgggagctccgtcttcccaacgtgtacgccacatgtcaaaagaggccgccagctagacaccccagaaaagaagcagagaaagagacttctttgtgcgacacgttttattctgcgtcctccgctcgacgttcaaatctggatgtactcgcgcacacccgtcaggctctttaagggaaaagggtccgagtacgtcactaaccgcgactgatgcaccagggcggtaatcacccgctccgcgccctcgcgcgtcgacgaacgcgtcgtcaccaggcaatgcagccgcgggcccgtatcgtcctgatgaccagcggcctcgcgctcggctgcttccacaccgacaatgtcgggatccaacacgtagctctgcgagttggtgtcgtagcggtgtagcaccaacgtgttggggtccagacgctcccacgcgccctcgtgcgggtcaaaacgctccgttaaacagagccagtcatactgctgctgcagaatacgccgctcgcgctcgcgtcgctcatcgggcaacgcggcgtcttcgttgaagagaatgtcccgcttgtggtctacggcacgctcgtggtggtgcgggcacaggtgacggtgttccatacgcgtctgacgttgacgctcgcgctcaaaacgccggtgtcgaaagaccattttcagcaaccccatgcggaaaaactccgtgatggtgttggcaacgcgccgcacatagtggttggggtcgtccatctggatggcgtacacggcaccgaaccagtccagcagtaccagcacttcggccacaaaactgcgtcccggtcgcggacgtcccgtcacgcctagcacataccacggcgtggccagattagcacggacagcccaccaccaacgacggctctccacctcggtgagcgcacaaaagggccaaatgcggtgtaactgctgtaccgttttcatcaaccgcataatcaccgtaccgtaacccggtgtatgcaactttacgtcgcaacccaggattcgttcggccgtggcgtacgagccctcgggcgtggtgtcattgagaaacaaaacatgcatggtacgcgcgcccttaggatatcgtcgcggaacgggtaccgtcattctccgcagagtggtgtgaatcacgtcgcgatacgcaatctccgaacgtgacacaccgtaacgtgccagttcgtccaggttgtgcgataccaacaccatgtacttttcacgagtgtcgtaggcgtagacgcgagaaaagcgacccataaaaaccacgtacggagtagccaccatgccatcatggtgatcgcgacgtggctcgggcaacaaaataacagcgtatcccaacggcgtcaacggctcgcggcaacagatgagctttgacgccgcctgtttggcggcggtaatgatcccgtcctccgtacgtaacatcacatgccagcccttggggggacccaaggacagacagcgtccctcgttacgatgaacgtaacgcgtgatttccattggctccaggcaaaagaacagttccttaaaatcccgcaacacttgtcggtataacgccatgggatcctcggccgccacaggcagcgcggggagctccggcggcataactgcagcgccgtcagggccagaacccgcagccggatccatcattgagcgacactctcagccggacaaccggcgtcactgacagaagccgagccaaatacagagaaagcaacgctacaccgtcaccccgctcccaagcgccgcggaaagtgctccgatttttcaccgtcgttcgcgacgttgatttgcctcggtctgagaaccgacctagcgttcggaccggtgcgcagaaacagccggcggtccgagccactgagcggttcacagccccggccgccgatagttaccggagagacgttcgagctgcaggtacatcagcgcttcccgcttcgccaccccgcgcccgccccagtttatactctccgacgccccgtccaacgcgcctgtggagggccaatcggaccgcgggagctctccaagtggatgacaggcacagccgagtgcccgaccgtgaagagccctcatccacctgaacagaccgctaaccgaaggaccccgagtcgcgtccgtcggtcccgacgtccgtcgccatctggctccctgctgttggctacctctcggatttcaaaaaagagcacgtgccgatgacggtgcacaggaaagagccaaagtgtcacggcgtctttttttatttgtattcctttcctgttttgtactcgtaaactgttgatgttgtttttacatccaaaagggcaagtaagaaacaggatgaggcatggtaggtttgggcgtggggcggccctccagcacggcggcccgggccgcccggcgggtgagcacccggcgttgcgccgtgtctatcttgtgtttcttctgtgtctttttcctatcttgttccgcgacggcctctttcatcacgttcagcatgcgttcctcgacgccctccagggatcctggggaggagggagtcctagtgaggcttccaatgttgttttgtggattttcggtttccttttcttggtcgtcatcgtcggacgtgtcgtcttcctcttgatcctcttcttcgtccgagtagtagacgcatagtccttggttcatcaggctgggattcatcaggttctgacggggaatccgctgttgtagacgtttaaccgcccgttccaggcgagagctcatgccgcaccagacgctgtaacgccgcacgggcccgtagcgggctgtttgttcgcgtacatgatcgttgagctcttgccaatattgtttggcacactccagatcggaggtttgtggatagtcgggtcggatccgcggatcccaactgacatcggcggtgccggagacttcgtccagactgttacgcatagagcaccagtcgggtcggacgataaacctgtccttgcggattaaccatttataacgtagttcgtgatggcgtgtagaggcccgtacacgctccacggtcccaaagcggtcccagaagggaaagttttcgtgggggcagcgacccggcacttccagacgttcggcgtcgtccacggcgtagtgaaaacgccggccggcctggtaaattttgagcagacccactgttaacaacatatccacgctgtcagccaaccgccagatctcgcggcgagacacgtcaaaatagaaaaattcgcaggctcggtcgaccaggatcacgaaatcggcgtgaaagacgccggagggtagcgattcgcccaccacacccattatcatggtttcacagcataagcggtccacaaagaacttcaacaggtcgttgaattgctccgtctccatacagatgaagggccagacgcctttgaggttctcggcctggccgcagagcagtagcggacgtgtcatctcgcccggagtgcgcagaggcacgcattcgccgcgataacgacaggtcacacgctgtagttcgctgatgctgttgtcgtgcaggcgaaggtcgcagataatatgatccggttgcgtggttagcagcggcgtgcgcatttgctcgccgtagatggcctcgcagtgcaacagcccgtgtcgcgcaaaatcgtccaaactgtgcgccaggtagtaaagcaccccgcgatcgcggtctagacaccacacggtttcgtaacgtcctaacaggagcaccagacgggcctggctaggtggctcaatttcctctacatacacgaaaaagtcgtcatcgtccgagtcctcgtcctcagaagaggaccgcggcccgtgtactctgggcaacacggtggtagagaactgcaggacgcccagagactcgagcgattcttcgcagcagatgagctgaccccagggcgtttcgggcccgtcggtgacagccgcgctgccaaagatgtcctcaaactctacaaaatctagacgccatccgggtggcgctgaaatgggaaggctaatgttcatatcagcatagctacgaactaagtggcggatgtcctgccgcaagtcttggcagagaatgagctttcgtaaacccttgagggtcctccgaacaacggccccagacgcgtagcgataggactggcgcatggtgccgcggcgtggagcggcacttggcagcctattttatggagtttcttcagtgacgtggcttgttcacgtcgttcgtgggctgcggttggcagctccggtctgtaaaccacccgaaaagactgacatcgacgtcaaagactcacgtaatttggaacatgtgcgaccgcaaagtgcgtcagaatagcacgtggctttaggacataaaaagtaccgtgaggtctagacgtgggttttgtgattgacacttacaccaggtaagccaagggacggtgaaactgtatgtgaggaatctgggtgcttagacgactaacgtgtaatgctttttacaggactgttcgacaggtgatagtacctgtaaggtgatgaccacctctacaaataatcaaaccttaacgcaggtgagcaacatgacaaaccacaccttaaacagcaccgaaatttatcagttgttcgagtacactcggttgggggtatggttgatgtgcatcgtgggcacgtttctgaacgtgctggtgattaccaccatcctgtactaccgtcgtaagaaaaaatctccgagcgatacctacatctgcaacctggctgtagccgatctgttgattgtcgtcggcctgccgttttttctagaatatgccaagcatcaccctaaactcagccgagaggtggtttgttcgggactcaacgcttgtttctacatctgtctttttgccggcgtttgttttctcatcaacctgtcgatggatcgctactgcgtcatcgtttggggtgtagaattgaaccgcgtgcgaaataacaagcgggccacctgttgggtggtgattttttggatactagccgtgctcatggggatgccacattacctgatgtacagccataccaacaacgagtgtgttggtgaattcgctaacgagacgtcgggttggttccccgtgtttttgaacaccaaagttaacatttgcggctacctggcgcccatcgcgctgatggcgtacacgtacaaccgtatggtgcggtttatcattaactacgttggtaaatggcacatgcagacgctccacgttcttttggttgtggttgtgtcttttgccagcttttggtttcctttcaacctggcgctatttttagaatccatccgtcttctggcgggagtgtacaatgacacacttcaaaacgttattatcttctgtctatacgtcggtcagtttttggcctacgttcgcgcttgtctgaatcctgggatctacatcctagtaggcactcaaatgaggaaggacatgtggacaaccctaagggtattcgcctgttgctgcgtgaagcaggagataccttaccaggacattgatattgagctacaaaaggacatacaaagaagggccaaacacaccaaacgtacccattatgacagaaaaaatgcacctatggagtccggggaggaggaatttctgttgtaattcgatcctctctcacgcgtccgccgcacatctatttttgctaattgcacgtttcttcgtggtcacgtcggctcgaagaggttggtgtgaaaacgtcatctcgccgacgtggtgaaccgctcatatagaccaaaccggacgctgcctcagtctctcggtgcgtggaccagacggcgtccatgcaccgagggcagaactggtgctatcatgacaccgacgacgacgaccgcggaactcacgacggagtttgactacgatgaagacgcgactccttgtgttttcaccgacgtgcttaatcagtcaaagccagttacgttgtttctgtacggcgttgtctttctcttcggttccatcggcaacttcttggtgatcttcaccatcacctggcgacgtcggattcaatgctccggcgatgtttactttatcaacctcgcggccgccgatttgcttttcgtttgtacactacctctgtggatgcaatacctcctagatcacaactccctagccagcgtgccgtgtacgttactcactgcctgtttctacgtggctatgtttgccagtttgtgttttatcacggagattgcactcgatcgctactacgctattgtttacatgagatatcggcctgtaaaacaggcctgccttttcagtattttttggtggatctttgccgtgatcatcgccattccacactttatggtggtgaccaaaaaagacaatcaatgtatgaccgactacgactacttagaggtcagttacccgatcatcctcaacgtagaactcatgcttggtgctttcgtgatcccgctcagtgttatcagctactgctactaccgcatttccagaatcgttgcggtgtctcagtcgcgccacaaaggtcgcattgtacgggtacttatagcggtcgtgcttgtctttatcatcttttggctgccgtaccacctaacgctgtttgtggacacgttaaaactcctcaaatggatctccagcagctgcgagttcgaaagatcgctcaaacgtgcgctcatcttgaccgagtcgctcgccttttgtcactgttgtctcaatccgctgctgtacgtcttcgtgggcaccaagtttcggcaagaactacactgtctgctggccgagtttcgccagcgactcttttcccgcgatgtatcctggtaccacagcatgagcttttcgcgtcggagctcgccgagtcgaagagagacatcttccgacacgctgtccgacgaggtgtgtcgcgtctcacaaattataccgtaatataacttcgtatagcatacattatacgaagttattaaaaaagcgctacctcggccttttcatacaaaccccgtgtccgcccctcttttccccgtgcccgatatacacgatattaaacccacgaccatttccgtgcgattagcgaaccggaaaagtttatggggaaaaagacgtaggaaaggatcatgtagaaaaacatgcggtgtttccgatggtggctctacagtgggtggtggtggctcacgtttggatgtgctcggaccgtgacggtgggtttcgtcgcgcccacggtccgggcacaatcaaccgtggtccgctctgagccggctccgccgtcggaaacccgacgagacaacaatgacacgtcttacttcagcagcacctctttccattcttccgtgtcccctgccacctcagtggaccgtcaatttcgacggaccacgtacgaccgttgggacggtcgacgttggctgcgcacccgctacgggaacgccagcgcctgcgtgacgggcacccaatggagcaccaacttttttttctctcagtgtgagcactaccctagtttcgtgaaactcaacggggtgcagcgctggacacctgttcggagacctatgggcgaggttgcctactacgggggttgttgtatggtgggcgggggtaatcgtgcgtacgtgatactcgtgagcggttacgggaccgccagctacggcaacgctttacgcgtgaattttgggcgcggcaactgcacggcgccgaaacgcacctaccctcggcgcttggaactgcacgatggccgcacagaccctagccgttgcgatccctaccaagtgtatttctacggtctgcagtgtcctgagcaactggttatcaccgcccacggcggcgtgggtatgcgccgctgtcctaccggctctcgtcccaccccgtcccggccccaccggcatgacttggagaacgagctacatggtctgtgtgtggatcttctggtgtgcgtccttttattagctctgctgctgttggagctcgttcccatggaagccgtgcgtcacccgctgcttttctggcgacgcgtggcgttatcgccgtccacttccaaggtggatcgcgccgtcaagctgtgtcttcggcgcatgtttggtctgccgccgccaccgtcagtcgcaccacctggggaaaagaaggagctaccggctcaggcggccttgtcgccgccactgaccacctggtcactaccgccgtttccgtccacgcggatacctgacagtccgccgccaccgtaccagcttcgtcacgccacgtcactagtgacggtacccacgctgctgttatatacgtcatccgacatcggtgacacagcttcagaaacaacgtgtgtggcgcacgctacttatggggaacccccggagcccgctcgatcgacggctacggttcaggaatgtaccgttcttaccgccccgaattgcggcatcgtcaacaacgacggcgcggtctctgaaggccaagaccatggagatgcggttcaccatagcctggatgtggtttcccagtgtgctgctgatactggggttgttgacacctccgagtaacgggtgcaccgtcgatgttggacgaaacgtatccattggagaacagtgccgccttcgaaacggtgcgacgttctccaagggagacatcgaaggtaacttcagtgggcccgtcgtcgtggagttggactacgaagatatcgatattactggcgaacggcagcgacttcggttccatctcagcggactcgggtgtcctacaaaggaaaatataagaaaagacaatgaaagcgacgtcaacggtggaattcgctgggctctatatatacaaaccggcgacgccaagtacggtattcgtaaccagcatttgagtatacggttaatgtatcctggggaaaaaaatacacaacagctgttggattctgatttcagttgcgaacgtcaccggagaccgtccacgccgttgggaaagaacgccgaagtgcctcccgcgacccgcacgtcttctacatacagcgtcctcagcgcttttgtagtgtggatcggatccggcctcaatatcatctggtggaccggcatcgtgcttctggcggtggacgctctcggacttggcgagcgttggctgaggttagcactgtctcaccgggacaaacatcacgcatcgcgaaccgcggcgctccagtgtcaacgcgacatgttacttcggcaacgtcgacgggctcggcggctgcacgccgtttctgaaggcaaactgcaggaagagaagaaacgacagtctgctctggtctggaacgttgaggcgcgaccctttccgtccacacatcagctgattgtgctgccccctcctgtagcgtcagctcctcctgcggttccctcgcagccccccgagtattcgtctgtgtttccgcctgtataaaaataaagagacgggaggctgatcgcggccttcagcgtctcatttgtctttactctcgagtgcggtcggtgtctcgtcggtgagacgaggccgccgcccgacaagttcgatctcatgtcgctcttggagcgcgaagagagttggcgtcgcgtagtcgactactcgcacaacctgtggtgtacgtgcggtaactggcagagccacgttgagattcaggacgaggagccaaactgcgagcagccggagcccgcacactggctggaatacgtggcggtccagtggcaggcccgggttcgcgattctcacgatcgctggtgtctctgcaacgcctggcgtgatcacgccttgcgcggccgttggggtacggcgtattcctcgggttcctcggcctcttcctccggtttcgtcgcggagagcaagttcacctggtggaaacgactgcgccacagtacccggcgctggttgtttcgccgccggcgagctcgatacactccgtctaactgtggggaaagtagcactagcagcggccagagtagcggtgacgagagtaactgcagtctacgcacccacggcgtgtacacacggggtgaacaacactaatcgataagtcgcgtgtaggcgactggctacatcaaccggatatctgcggggatttaaaaagacgacccgttgtcatccggcttagaccaaaccgtccttttatcatcttccgtcgccatggctatgtacacatccgaatccgaacgcgactggcgtcgtgtaatccacgactcgcacggcctgtggtgcgactgcggcgactggcgagagcacctctattgtgtgtacgacagccattttcagcgacgacccacgacccgagccgaacggagggccgccaattggcggcgacagatgcggcggttacaccgtttgtggtgtttttgtcaggactggaagtgtcacgcgttatacgccgagtgggacggcaaagaatccgacgacgagtcgtcggcgtcttcctcgggcgaagcgccagagcaacaggtccccgcttggaagaccgtgcgggccttctcgcgggcctaccaccaccgcattaaccggggtctgcggggcacgcccccaccgcgcaacttgccgggatacgagcacgcctccgagggctggcggttttgcagtcgacgggaacggcgagaggacgatcttcgcacgcgggctgagccggaccgcgtggtgttccagttagggggagtaccccctcgccgtcaccgggaaacttacgtgtaagaacacggcgtgacaataaacaacatagcgtaaatccccgtgtgatgtgtgtgattgacgttcgggaaacatgtccccatcatcagcgtcacaattgacgtgggttggtcactgacgtgcaggatgttacgcgagtcagagaatcgcataagaacggagtggtgagcgggttcccacaggagtctctggcgcaaaagcaccatgagcctcaggttccccgagagggtgggttacgagaaactgggataccgcccgcatgccaaacgcgtgcgggtgcatgactcgttgggattgacgcggtttatcatgaggcaactcatgatgtacccgctggtgttgccgttcacttttccgttttacgtgccgcggtcctagcacgtcagtggtgacgctgataattgcaacatggcccatgacgaacccgcttgggacgaacgtcaataccacgtcaaaccaccgtgacttggctgaacgttgaaacataaagccaaagcgccgtcggcacttggcttcagagcagcgcctcggggcgatgcgacggcgatgaacttagagcaactcatcaacgtccttggtctgctcgtctggattgccgctcgtgctgtcagccgcgttggtccgcatggctccggactcgtttatcgtgagcttcatgatttctacgggtatctgcagctggaccttctgggaccagtggtggcggggaatcgctcagtccggacctggagagagcaggcggaccgagccagagggaccttcgcttggcgttcaggccttaatactagccgcatcttacctgtcggcagcatgtatcggggctccgacgccttacccgccggcctgtatcgtcccgaagaagaggtgttcctcctcttgaatcgctgccatgggccactgtcaacgccgaaaaatgcttgtctggctgaggttggtgtcgctaatgccacttttttgtctcgcttcaatgtcggtgattttcacggagcgtcatgggaaaacggtaccgctcccgatggagagcccggggtatgctgaaattcctcttaaaatttcgtaaacgacgtcgtccagtcgttgtgccgcgattcgtacggttcatcgtctacgtcgttttgttcaccgtcgctgtgcaacgcgtgaaacaagagcgtgatgcgcaccttcggcggtatgaagaacgattacggaaaaaccgcgcacggcgtcggcagtcttttccgtgacttggggcgatgggtccgagctgcggtatgggtcacggcggcgtgtgttttattgacgaagatgccgatgtgtgactaaaaacgtcccagccccagagcgatatgtttcaataaaaaaaatatgtagtatcatattatgcgtgtcctggtttttcatttttggatgtatgtatcgcataaagggtggcgaggtgtgaggatgaaacatatgcagatacgcagtgttgttatccgaacgaaacccgtgtaatgcgtacaacggtacttcagtatgaaagtcccgtgtgtggggggggggggcaaatagttgcgtttgccgttgggcgtacgctacgtttgtatttctggctataatatgtgcggtcatgtgtcgatgttcctattgggaagggtgtgactgtagggtgtataaagtacggtgggacgcagagggacattgatagaaacaggttgagcgctgtacgagtttcacacgctgaatcggcgccaagaataaaacagtggttattcgtaaaagtatgggggggggggggatgttgtcgacggttgttagatgcattgcgtatctgtattagtagttttgcaagccgtggtgcgtgttattgtgacgtagcaattatcgtattgtgcatgtgtcgttcatcacagagtttagtatactaatatgaagcgtcgcgagtattaaagcaattggtgtctctgtgctagtctaacaacacctgtgtaatgcgtacaacgagaaaaaagacgcgaaagcaacgtgtatgggggggggggggaataatattgctaatcatgcgtcttgcagtacagatagccgctgtatcttacgcgtattgtcgcaacagttccacatcggtgtaattggatgtctggtacttatcactggcgtcgttataacattgtaaaacaagttttcgaaacataacgacagctgcaaaagaaaaccagtttattgagcattgtaatggtagtgtgtggctatattagaaaacgtgacgcgtcgcatgtcgcggcacaatctggcagcggggtcggggtagggtacggtgggaggcatgtacacagatggaacaaaagcagaagtaacgtgagaaggagcatacagtccagtatccagcggttcctgagtagcaccacccatcaactgaatgccctcatgagtaaaagtctgcgggcgacagcccttggggaccgttggcatgggacgatcaatctccaaaccacagcgtaacaccgttttcttccaacgtcgttgatagacgtcgtttttacggttactcccaagaacccagaaagtctcgtccaagtcgtaccaggaatcttctccggggagacgcgacggtttccaatcctcgtcgtctcgtctcaaagcacgtcccaaactggcttgaggagtcaacggtggttctgtgggtcgggtgtagcgcgagtgttttcccttcatgagcgattcatcctccttgcctttaggctttttggtctttttgtgtatcatctggccgccggcctccataaccaccgtggccaagtccagtcccagagcttgagcgtcggcgcggcgtcgggcgtcttgcaggtagtcttccacatttgcacagatggccgggtgtttggtggctagggtgaggacctcagcctcgccgcgacccggacgtagcaaaaaagccaactgcccgtgcggctcgcgcgcccacagcgcggcgcgcgggtgcaggtgcagcgcgtcccagcgcggccgctcccactgctcgcggtccagctcgggcagcagccgccgcgcggcctcggcggcgggcgccgactcgcgtcccagcgccagcgcgcccagcacgcccgcgcgcagaaagtgcgacagctccgccgccagcgggtacacgtgcccgtccagcgggcagtacccgaacacggcgcccagctcgtccagcagcaccaccagcatggcgcgcggcacggtccccgacgccgccggacccgccatcgctgtcgaacccaccatcaccgtcggcgccgctgctgctgccgcgtccgccccgaccaccgcgtgcgcgtccgcgttaggcacgcaaatcgcgcccccgccggcggcgccgtacggctgcggaggcacaggtacagcggaccccacggctcccgctatcgcgcacggcgcgtccccgccggcggcctccgtctccgtgccgctcgccgctggcggcgacgtcgtccccgccgccgtccccgtcgccggccccgccgcgcagcccagccaccgcgcgggcagcaccgcgcccagcgccagccagccgcagcacagacgctggttcaggtgccgacgcacggccgtcagcagcgacgcggggtgcggcgccgacgcgaacggctcgtactgcgccagctcctgccacgcgcccagcagtaccatcggctgcagtcgcctgcccggcgtctgcagcgccaccgtcgtgccggcccaccgccggcgcagctcccgtccgagcgccgtcgcctcctcggcgcgcagcaacgtctgtcggagcgccggctgaggcagcagcgtcgcgcgcggggtgcccacgcccagccggttgcagcggtacagccgcaccacctcgcccgcgccgtgccgaaaccactcgtccgcgtcgcgcgccgctaggatcagcgtgttgtttgccaggtcgtacacgaacacgcggaacccggcgcccagcgccaggtacagtccgtcctgcgcgcacagaccctcgggatggccggccttgtcgcccaacgtcgggtcggctgcggggtccacctcgtgcaccacggtagccaccagtacgatccacgcgtcccgcggcgacagttgacgcaggtccgtcgcgcccacgccgttcatctggctgcgcggcgtcacccgcgcgtagaatccgtacggccgtccgagcggcagcagcgtgcccgcgtcgcgctgcgaccacttgcgcatggcgcggcccgtgctgttggccaaaaacgccgcgcgccacacggcgcccatggcctggtattccagctccgtcagcgcctggcgctccaccggaatctgagacagcaacaggcgctccgggccgtgccaaaagttgctattgttgccgctactcggaggggcgcccggcggcccgcggggttctacccggtggacgccgtggcccggcgtcgtcgtagccgcagcactcgcaccagtgcccgctgtggacggcgctcccatcggcacacaagaagaaggaggagaggaaccaacccccgaaggccctccggccccgcggccgcgaccaaggggcggggggcgcggcgacatgccgttgcgctgggccatgggcgccggacacctccgacgtccactatataggaagcaaacccgcgtcagcgagcacgcggtttagacacgcggacgccttcgtcgcccgtgtgccgcgggcgacacgcagctggcttttataggcagcgacgtgcacggcgcgtgctggcgccgccttggcgccacgcagtctggaaggccgtggactgggaaaggcagctacccgaaggaagacgcgcggcaggcgcgtaccactggagcgcacagccgcctcccgggcgcgcacccatctaggtggacgcccgacatccattccgggccgcgtggtgggtcctcgaggggcgggggggtgtttttagcgggggggtgaaacttggagttgcgtgtgtggacggcgactagttgcgtgtggtgcggaggacggcgacggcgaataaaagcgacgtgcggcgcgcacggcgaaaagaagacgcgtgtctgtgtctgtgtgattccccggggaaaagaggaagttcccgggggacggcagcatgggtccctggggacacacgaaaagcaacgcccgggggcgagggacgacggccctggggaccgcgggggaaataacggccgcgaggccacacactcgttcctgcgaagccgcacaccccgaggccgcgcacaccgccgacacaccccgccaccacaccccgccggcacacccgccacacgcccgcgacacacccggcacgacacacccggcacacgcccgcgacacaccctgacacaccctgccaacacacccccgacacacccaacacacgcccgcgacacacccggcacacacccacccggccgcgccccgacacacccaaaacaccgccggtgcggggccgcgtggtgggtcctcgaggg